European Patent Specification EP 3 497 215 B1, published January 10, 2024. Title: CELL-PERMEABLE (CP)-Cas9 RECOMBINANT PROTEIN AND USES THEREOF. Applicant: CELLIVERY THERAPEUTICS INC. The sequence listing filed with the application follows.

SEQUENCE LISTING (1243 sequences)

SEQ ID NO: 1 - protein, 12 aa, Artificial Sequence
  Amino acid Sequence of aMTD1
AAALAPVVLALP

SEQ ID NO: 2 - protein, 12 aa, Artificial Sequence
  Amino acid Sequence of aMTD2
AAAVPLLAVVVP

SEQ ID NO: 3 - protein, 12 aa, Artificial Sequence
  Amino acid Sequence of aMTD3
AALLVPAAVLAP

SEQ ID NO: 4 - protein, 12 aa, Artificial Sequence
  Amino acid Sequence of aMTD4
ALALLPVAALAP

SEQ ID NO: 5 - protein, 12 aa, Artificial Sequence
  Amino acid Sequence of aMTD5
AAALLPVALVAP

SEQ ID NO: 6 - protein, 12 aa, Artificial Sequence
  Amino acid Sequence of aMTD11
VVALAPALAALP

SEQ ID NO: 7 - protein, 12 aa, Artificial Sequence
  Amino acid Sequence of aMTD12
LLAAVPAVLLAP

SEQ ID NO: 8 - protein, 12 aa, Artificial Sequence
  Amino acid Sequence of aMTD13
AAALVPVVALLP

SEQ ID NO: 9 - protein, 12 aa, Artificial Sequence
  Amino acid Sequence of aMTD21
AVALLPALLAVP

SEQ ID NO: 10 - protein, 12 aa, Artificial Sequence
  Amino acid Sequence of aMTD22
AVVLVPVLAAAP

SEQ ID NO: 11 - protein, 12 aa, Artificial Sequence
  Amino acid Sequence of aMTD23
VVLVLPAAAAVP

SEQ ID NO: 12 - protein, 12 aa, Artificial Sequence
  Amino acid Sequence of aMTD24
IALAAPALIVAP

SEQ ID NO: 13 - protein, 12 aa, Artificial Sequence
  Amino acid Sequence of aMTD25
IVAVAPALVALP

SEQ ID NO: 14 - protein, 12 aa, Artificial Sequence
  Amino acid Sequence of aMTD42
VAALPVVAVVAP

SEQ ID NO: 15 - protein, 12 aa, Artificial Sequence
  Amino acid Sequence of aMTD43
LLAAPLVVAAVP

SEQ ID NO: 16 - protein, 12 aa, Artificial Sequence
  Amino acid Sequence of aMTD44
ALAVPVALLVAP

SEQ ID NO: 17 - protein, 12 aa, Artificial Sequence
  Amino acid Sequence of aMTD61
VAALPVLLAALP

SEQ ID NO: 18 - protein, 12 aa, Artificial Sequence
  Amino acid Sequence of aMTD62
VALLAPVALAVP

SEQ ID NO: 19 - protein, 12 aa, Artificial Sequence
  Amino acid Sequence of aMTD63
AALLVPALVAVP

SEQ ID NO: 20 - protein, 12 aa, Artificial Sequence
  Amino acid Sequence of aMTD64
AIVALPVAVLAP

SEQ ID NO: 21 - protein, 12 aa, Artificial Sequence
  Amino acid Sequence of aMTD65
IAIVAPVVALAP

SEQ ID NO: 22 - protein, 12 aa, Artificial Sequence
  Amino acid Sequence of aMTD81
AALLPALAALLP

SEQ ID NO: 23 - protein, 12 aa, Artificial Sequence
  Amino acid Sequence of aMTD82
AVVLAPVAAVLP

SEQ ID NO: 24 - protein, 12 aa, Artificial Sequence
  Amino acid Sequence of aMTD83
LAVAAPLALALP

SEQ ID NO: 25 - protein, 12 aa, Artificial Sequence
  Amino acid Sequence of aMTD84
AAVAAPLLLALP

SEQ ID NO: 26 - protein, 12 aa, Artificial Sequence
  Amino acid Sequence of aMTD85
LLVLPAAALAAP

SEQ ID NO: 27 - protein, 12 aa, Artificial Sequence
  Amino acid Sequence of aMTD101
LVALAPVAAVLP

SEQ ID NO: 28 - protein, 12 aa, Artificial Sequence
  Amino acid Sequence of aMTD102
LALAPAALALLP

SEQ ID NO: 29 - protein, 12 aa, Artificial Sequence
  Amino acid Sequence of aMTD103
ALIAAPILALAP

SEQ ID NO: 30 - protein, 12 aa, Artificial Sequence
  Amino acid Sequence of aMTD104
AVVAAPLVLALP

SEQ ID NO: 31 - protein, 12 aa, Artificial Sequence
  Amino acid Sequence of aMTD105
LLALAPAALLAP

SEQ ID NO: 32 - protein, 12 aa, Artificial Sequence
  Amino acid Sequence of aMTD121
AIVALPALALAP

SEQ ID NO: 33 - protein, 12 aa, Artificial Sequence
  Amino acid Sequence of aMTD123
AAIIVPAALLAP

SEQ ID NO: 34 - protein, 12 aa, Artificial Sequence
  Amino acid Sequence of aMTD124
IAVALPALIAAP

SEQ ID NO: 35 - protein, 12 aa, Artificial Sequence
  Amino acid Sequence of aMTD141
AVIVLPALAVAP

SEQ ID NO: 36 - protein, 12 aa, Artificial Sequence
  Amino acid Sequence of aMTD143
AVLAVPAVLVAP

SEQ ID NO: 37 - protein, 12 aa, Artificial Sequence
  Amino acid Sequence of aMTD144
VLAIVPAVALAP

SEQ ID NO: 38 - protein, 12 aa, Artificial Sequence
  Amino acid Sequence of aMTD145
LLAVVPAVALAP

SEQ ID NO: 39 - protein, 12 aa, Artificial Sequence
  Amino acid Sequence of aMTD161
AVIALPALIAAP

SEQ ID NO: 40 - protein, 12 aa, Artificial Sequence
  Amino acid Sequence of aMTD162
AVVALPAALIVP

SEQ ID NO: 41 - protein, 12 aa, Artificial Sequence
  Amino acid Sequence of aMTD163
LALVLPAALAAP

SEQ ID NO: 42 - protein, 12 aa, Artificial Sequence
  Amino acid Sequence of aMTD164
LAAVLPALLAAP

SEQ ID NO: 43 - protein, 12 aa, Artificial Sequence
  Amino acid Sequence of aMTD165
ALAVPVALAIVP

SEQ ID NO: 44 - protein, 12 aa, Artificial Sequence
  Amino acid Sequence of aMTD182
ALIAPVVALVAP

SEQ ID NO: 45 - protein, 12 aa, Artificial Sequence
  Amino acid Sequence of aMTD183
LLAAPVVIALAP

SEQ ID NO: 46 - protein, 12 aa, Artificial Sequence
  Amino acid Sequence of aMTD184
LAAIVPAIIAVP

SEQ ID NO: 47 - protein, 12 aa, Artificial Sequence
  Amino acid Sequence of aMTD185
AALVLPLIIAAP

SEQ ID NO: 48 - protein, 12 aa, Artificial Sequence
  Amino acid Sequence of aMTD201
LALAVPALAALP

SEQ ID NO: 49 - protein, 12 aa, Artificial Sequence
  Amino acid Sequence of aMTD204
LIAALPAVAALP

SEQ ID NO: 50 - protein, 12 aa, Artificial Sequence
  Amino acid Sequence of aMTD205
ALALVPAIAALP

SEQ ID NO: 51 - protein, 12 aa, Artificial Sequence
  Amino acid Sequence of aMTD221
AAILAPIVALAP

SEQ ID NO: 52 - protein, 12 aa, Artificial Sequence
  Amino acid Sequence of aMTD222
ALLIAPAAVIAP

SEQ ID NO: 53 - protein, 12 aa, Artificial Sequence
  Amino acid Sequence of aMTD223
AILAVPIAVVAP

SEQ ID NO: 54 - protein, 12 aa, Artificial Sequence
  Amino acid Sequence of aMTD224
ILAAVPIALAAP

SEQ ID NO: 55 - protein, 12 aa, Artificial Sequence
  Amino acid Sequence of aMTD225
VAALLPAAAVLP

SEQ ID NO: 56 - protein, 12 aa, Artificial Sequence
  Amino acid Sequence of aMTD241
AAAVVPVLLVAP

SEQ ID NO: 57 - protein, 12 aa, Artificial Sequence
  Amino acid Sequence of aMTD242
AALLVPALVAAP

SEQ ID NO: 58 - protein, 12 aa, Artificial Sequence
  Amino acid Sequence of aMTD243
AAVLLPVALAAP

SEQ ID NO: 59 - protein, 12 aa, Artificial Sequence
  Amino acid Sequence of aMTD245
AAALAPVLALVP

SEQ ID NO: 60 - protein, 12 aa, Artificial Sequence
  Amino acid Sequence of aMTD261
LVLVPLLAAAAP

SEQ ID NO: 61 - protein, 12 aa, Artificial Sequence
  Amino acid Sequence of aMTD262
ALIAVPAIIVAP

SEQ ID NO: 62 - protein, 12 aa, Artificial Sequence
  Amino acid Sequence of aMTD263
ALAVIPAAAILP

SEQ ID NO: 63 - protein, 12 aa, Artificial Sequence
  Amino acid Sequence of aMTD264
LAAAPVVIVIAP

SEQ ID NO: 64 - protein, 12 aa, Artificial Sequence
  Amino acid Sequence of aMTD265
VLAIAPLLAAVP

SEQ ID NO: 65 - protein, 12 aa, Artificial Sequence
  Amino acid Sequence of aMTD281
ALIVLPAAVAVP

SEQ ID NO: 66 - protein, 12 aa, Artificial Sequence
  Amino acid Sequence of aMTD282
VLAVAPALIVAP

SEQ ID NO: 67 - protein, 12 aa, Artificial Sequence
  Amino acid Sequence of aMTD283
AALLAPALIVAP

SEQ ID NO: 68 - protein, 12 aa, Artificial Sequence
  Amino acid Sequence of aMTD284
ALIAPAVALIVP

SEQ ID NO: 69 - protein, 12 aa, Artificial Sequence
  Amino acid Sequence of aMTD285
AIVLLPAAVVAP

SEQ ID NO: 70 - protein, 12 aa, Artificial Sequence
  Amino acid Sequence of aMTD301
VIAAPVLAVLAP

SEQ ID NO: 71 - protein, 12 aa, Artificial Sequence
  Amino acid Sequence of aMTD302
LALAPALALLAP

SEQ ID NO: 72 - protein, 12 aa, Artificial Sequence
  Amino acid Sequence of aMTD304
AIILAPIAAIAP

SEQ ID NO: 73 - protein, 12 aa, Artificial Sequence
  Amino acid Sequence of aMTD305
IALAAPILLAAP

SEQ ID NO: 74 - protein, 12 aa, Artificial Sequence
  Amino acid Sequence of aMTD321
IVAVALPALAVP

SEQ ID NO: 75 - protein, 12 aa, Artificial Sequence
  Amino acid Sequence of aMTD322
VVAIVLPALAAP

SEQ ID NO: 76 - protein, 12 aa, Artificial Sequence
  Amino acid Sequence of aMTD323
IVAVALPVALAP

SEQ ID NO: 77 - protein, 12 aa, Artificial Sequence
  Amino acid Sequence of aMTD324
IVAVALPAALVP

SEQ ID NO: 78 - protein, 12 aa, Artificial Sequence
  Amino acid Sequence of aMTD325
IVAVALPAVALP

SEQ ID NO: 79 - protein, 12 aa, Artificial Sequence
  Amino acid Sequence of aMTD341
IVAVALPAVLAP

SEQ ID NO: 80 - protein, 12 aa, Artificial Sequence
  Amino acid Sequence of aMTD342
VIVALAPAVLAP

SEQ ID NO: 81 - protein, 12 aa, Artificial Sequence
  Amino acid Sequence of aMTD343
IVAVALPALVAP

SEQ ID NO: 82 - protein, 12 aa, Artificial Sequence
  Amino acid Sequence of aMTD345
ALLIVAPVAVAP

SEQ ID NO: 83 - protein, 12 aa, Artificial Sequence
  Amino acid Sequence of aMTD361
AVVIVAPAVIAP

SEQ ID NO: 84 - protein, 12 aa, Artificial Sequence
  Amino acid Sequence of aMTD363
AVLAVAPALIVP

SEQ ID NO: 85 - protein, 12 aa, Artificial Sequence
  Amino acid Sequence of aMTD364
LVAAVAPALIVP

SEQ ID NO: 86 - protein, 12 aa, Artificial Sequence
  Amino acid Sequence of aMTD365
AVIVVAPALLAP

SEQ ID NO: 87 - protein, 12 aa, Artificial Sequence
  Amino acid Sequence of aMTD381
VVAIVLPAVAAP

SEQ ID NO: 88 - protein, 12 aa, Artificial Sequence
  Amino acid Sequence of aMTD382
AAALVIPAILAP

SEQ ID NO: 89 - protein, 12 aa, Artificial Sequence
  Amino acid Sequence of aMTD383
VIVALAPALLAP

SEQ ID NO: 90 - protein, 12 aa, Artificial Sequence
  Amino acid Sequence of aMTD384
VIVAIAPALLAP

SEQ ID NO: 91 - protein, 12 aa, Artificial Sequence
  Amino acid Sequence of aMTD385
IVAIAVPALVAP

SEQ ID NO: 92 - protein, 12 aa, Artificial Sequence
  Amino acid Sequence of aMTD401
AALAVIPAAILP

SEQ ID NO: 93 - protein, 12 aa, Artificial Sequence
  Amino acid Sequence of aMTD402
ALAAVIPAAILP

SEQ ID NO: 94 - protein, 12 aa, Artificial Sequence
  Amino acid Sequence of aMTD403
AAALVIPAAILP

SEQ ID NO: 95 - protein, 12 aa, Artificial Sequence
  Amino acid Sequence of aMTD404
LAAAVIPAAILP

SEQ ID NO: 96 - protein, 12 aa, Artificial Sequence
  Amino acid Sequence of aMTD405
LAAAVIPVAILP

SEQ ID NO: 97 - protein, 12 aa, Artificial Sequence
  Amino acid Sequence of aMTD421
AAILAAPLIAVP

SEQ ID NO: 98 - protein, 12 aa, Artificial Sequence
  Amino acid Sequence of aMTD422
VVAILAPLLAAP

SEQ ID NO: 99 - protein, 12 aa, Artificial Sequence
  Amino acid Sequence of aMTD424
AVVVAAPVLALP

SEQ ID NO: 100 - protein, 12 aa, Artificial Sequence
  Amino acid Sequence of aMTD425
AVVAIAPVLALP

SEQ ID NO: 101 - protein, 12 aa, Artificial Sequence
  Amino acid Sequence of aMTD442
ALAALVPAVLVP

SEQ ID NO: 102 - protein, 12 aa, Artificial Sequence
  Amino acid Sequence of aMTD443
ALAALVPVALVP

SEQ ID NO: 103 - protein, 12 aa, Artificial Sequence
  Amino acid Sequence of aMTD444
LAAALVPVALVP

SEQ ID NO: 104 - protein, 12 aa, Artificial Sequence
  Amino acid Sequence of aMTD445
ALAALVPALVVP

SEQ ID NO: 105 - protein, 12 aa, Artificial Sequence
  Amino acid Sequence of aMTD461
IAAVIVPAVALP

SEQ ID NO: 106 - protein, 12 aa, Artificial Sequence
  Amino acid Sequence of aMTD462
IAAVLVPAVALP

SEQ ID NO: 107 - protein, 12 aa, Artificial Sequence
  Amino acid Sequence of aMTD463
AVAILVPLLAAP

SEQ ID NO: 108 - protein, 12 aa, Artificial Sequence
  Amino acid Sequence of aMTD464
AVVILVPLAAAP

SEQ ID NO: 109 - protein, 12 aa, Artificial Sequence
  Amino acid Sequence of aMTD465
IAAVIVPVAALP

SEQ ID NO: 110 - protein, 12 aa, Artificial Sequence
  Amino acid Sequence of aMTD481
AIAIAIVPVALP

SEQ ID NO: 111 - protein, 12 aa, Artificial Sequence
  Amino acid Sequence of aMTD482
ILAVAAIPVAVP

SEQ ID NO: 112 - protein, 12 aa, Artificial Sequence
  Amino acid Sequence of aMTD483
ILAAAIIPAALP

SEQ ID NO: 113 - protein, 12 aa, Artificial Sequence
  Amino acid Sequence of aMTD484
LAVVLAAPAIVP

SEQ ID NO: 114 - protein, 12 aa, Artificial Sequence
  Amino acid Sequence of aMTD485
AILAAIVPLAVP

SEQ ID NO: 115 - protein, 12 aa, Artificial Sequence
  Amino acid Sequence of aMTD501
VIVALAVPALAP

SEQ ID NO: 116 - protein, 12 aa, Artificial Sequence
  Amino acid Sequence of aMTD502
AIVALAVPVLAP

SEQ ID NO: 117 - protein, 12 aa, Artificial Sequence
  Amino acid Sequence of aMTD503
AAIIIVLPAALP

SEQ ID NO: 118 - protein, 12 aa, Artificial Sequence
  Amino acid Sequence of aMTD504
LIVALAVPALAP

SEQ ID NO: 119 - protein, 12 aa, Artificial Sequence
  Amino acid Sequence of aMTD505
AIIIVIAPAAAP

SEQ ID NO: 120 - protein, 12 aa, Artificial Sequence
  Amino acid Sequence of aMTD521
LAALIVVPAVAP

SEQ ID NO: 121 - protein, 12 aa, Artificial Sequence
  Amino acid Sequence of aMTD522
ALLVIAVPAVAP

SEQ ID NO: 122 - protein, 12 aa, Artificial Sequence
  Amino acid Sequence of aMTD524
AVALIVVPALAP

SEQ ID NO: 123 - protein, 12 aa, Artificial Sequence
  Amino acid Sequence of aMTD525
ALAIVVAPVAVP

SEQ ID NO: 124 - protein, 12 aa, Artificial Sequence
  Amino acid Sequence of aMTD541
LLALIIAPAAAP

SEQ ID NO: 125 - protein, 12 aa, Artificial Sequence
  Amino acid Sequence of aMTD542
ALALIIVPAVAP

SEQ ID NO: 126 - protein, 12 aa, Artificial Sequence
  Amino acid Sequence of aMTD543
LLAALIAPAALP

SEQ ID NO: 127 - protein, 12 aa, Artificial Sequence
  Amino acid Sequence of aMTD544
IVALIVAPAAVP

SEQ ID NO: 128 - protein, 12 aa, Artificial Sequence
  Amino acid Sequence of aMTD545
VVLVLAAPAAVP

SEQ ID NO: 129 - protein, 12 aa, Artificial Sequence
  Amino acid Sequence of aMTD561
AAVAIVLPAVVP

SEQ ID NO: 130 - protein, 12 aa, Artificial Sequence
  Amino acid Sequence of aMTD562
ALIAAIVPALVP

SEQ ID NO: 131 - protein, 12 aa, Artificial Sequence
  Amino acid Sequence of aMTD563
ALAVIVVPALAP

SEQ ID NO: 132 - protein, 12 aa, Artificial Sequence
  Amino acid Sequence of aMTD564
VAIALIVPALAP

SEQ ID NO: 133 - protein, 12 aa, Artificial Sequence
  Amino acid Sequence of aMTD565
VAIVLVAPAVAP

SEQ ID NO: 134 - protein, 12 aa, Artificial Sequence
  Amino acid Sequence of aMTD582
VAVALIVPALAP

SEQ ID NO: 135 - protein, 12 aa, Artificial Sequence
  Amino acid Sequence of aMTD583
AVILALAPIVAP

SEQ ID NO: 136 - protein, 12 aa, Artificial Sequence
  Amino acid Sequence of aMTD585
ALIVAIAPALVP

SEQ ID NO: 137 - protein, 12 aa, Artificial Sequence
  Amino acid Sequence of aMTD601
AAILIAVPIAAP

SEQ ID NO: 138 - protein, 12 aa, Artificial Sequence
  Amino acid Sequence of aMTD602
VIVALAAPVLAP

SEQ ID NO: 139 - protein, 12 aa, Artificial Sequence
  Amino acid Sequence of aMTD603
VLVALAAPVIAP

SEQ ID NO: 140 - protein, 12 aa, Artificial Sequence
  Amino acid Sequence of aMTD604
VALIAVAPAVVP

SEQ ID NO: 141 - protein, 12 aa, Artificial Sequence
  Amino acid Sequence of aMTD605
VIAAVLAPVAVP

SEQ ID NO: 142 - protein, 12 aa, Artificial Sequence
  Amino acid Sequence of aMTD622
ALIVLAAPVAVP

SEQ ID NO: 143 - protein, 12 aa, Artificial Sequence
  Amino acid Sequence of aMTD623
VAAAIALPAIVP

SEQ ID NO: 144 - protein, 12 aa, Artificial Sequence
  Amino acid Sequence of aMTD625
ILAAAAAPLIVP

SEQ ID NO: 145 - protein, 12 aa, Artificial Sequence
  Amino acid Sequence of aMTD643
LALVLAAPAIVP

SEQ ID NO: 146 - protein, 12 aa, Artificial Sequence
  Amino acid Sequence of aMTD645
ALAVVALPAIVP

SEQ ID NO: 147 - protein, 12 aa, Artificial Sequence
  Amino acid Sequence of aMTD661
AAILAPIVAALP

SEQ ID NO: 148 - protein, 12 aa, Artificial Sequence
  Amino acid Sequence of aMTD664
ILIAIAIPAAAP

SEQ ID NO: 149 - protein, 12 aa, Artificial Sequence
  Amino acid Sequence of aMTD665
LAIVLAAPVAVP

SEQ ID NO: 150 - protein, 12 aa, Artificial Sequence
  Amino acid Sequence of aMTD666
AAIAIIAPAIVP

SEQ ID NO: 151 - protein, 12 aa, Artificial Sequence
  Amino acid Sequence of aMTD667
LAVAIVAPALVP

SEQ ID NO: 152 - protein, 12 aa, Artificial Sequence
  Amino acid Sequence of aMTD683
LAIVLAAPAVLP

SEQ ID NO: 153 - protein, 12 aa, Artificial Sequence
  Amino acid Sequence of aMTD684
AAIVLALPAVLP

SEQ ID NO: 154 - protein, 12 aa, Artificial Sequence
  Amino acid Sequence of aMTD685
ALLVAVLPAALP

SEQ ID NO: 155 - protein, 12 aa, Artificial Sequence
  Amino acid Sequence of aMTD686
AALVAVLPVALP

SEQ ID NO: 156 - protein, 12 aa, Artificial Sequence
  Amino acid Sequence of aMTD687
AILAVALPLLAP

SEQ ID NO: 157 - protein, 12 aa, Artificial Sequence
  Amino acid Sequence of aMTD703
IVAVALVPALAP

SEQ ID NO: 158 - protein, 12 aa, Artificial Sequence
  Amino acid Sequence of aMTD705
IVAVALLPALAP

SEQ ID NO: 159 - protein, 12 aa, Artificial Sequence
  Amino acid Sequence of aMTD706
IVAVALLPAVAP

SEQ ID NO: 160 - protein, 12 aa, Artificial Sequence
  Amino acid Sequence of aMTD707
IVALAVLPAVAP

SEQ ID NO: 161 - protein, 12 aa, Artificial Sequence
  Amino acid Sequence of aMTD724
VAVLAVLPALAP

SEQ ID NO: 162 - protein, 12 aa, Artificial Sequence
  Amino acid Sequence of aMTD725
IAVLAVAPAVLP

SEQ ID NO: 163 - protein, 12 aa, Artificial Sequence
  Amino acid Sequence of aMTD726
LAVAIIAPAVAP

SEQ ID NO: 164 - protein, 12 aa, Artificial Sequence
  Amino acid Sequence of aMTD727
VALAIALPAVLP

SEQ ID NO: 165 - protein, 12 aa, Artificial Sequence
  Amino acid Sequence of aMTD743
AIAIALVPVALP

SEQ ID NO: 166 - protein, 12 aa, Artificial Sequence
  Amino acid Sequence of aMTD744
AAVVIVAPVALP

SEQ ID NO: 167 - protein, 12 aa, Artificial Sequence
  Amino acid Sequence of aMTD746
VAIIVVAPALAP

SEQ ID NO: 168 - protein, 12 aa, Artificial Sequence
  Amino acid Sequence of aMTD747
VALLAIAPALAP

SEQ ID NO: 169 - protein, 12 aa, Artificial Sequence
  Amino acid Sequence of aMTD763
VAVLIAVPALAP

SEQ ID NO: 170 - protein, 12 aa, Artificial Sequence
  Amino acid Sequence of aMTD764
AVALAVLPAVVP

SEQ ID NO: 171 - protein, 12 aa, Artificial Sequence
  Amino acid Sequence of aMTD765
AVALAVVPAVLP

SEQ ID NO: 172 - protein, 12 aa, Artificial Sequence
  Amino acid Sequence of aMTD766
IVVIAVAPAVAP

SEQ ID NO: 173 - protein, 12 aa, Artificial Sequence
  Amino acid Sequence of aMTD767
IVVAAVVPALAP

SEQ ID NO: 174 - protein, 12 aa, Artificial Sequence
  Amino acid Sequence of aMTD783
IVALVPAVAIAP

SEQ ID NO: 175 - protein, 12 aa, Artificial Sequence
  Amino acid Sequence of aMTD784
VAALPAVALVVP

SEQ ID NO: 176 - protein, 12 aa, Artificial Sequence
  Amino acid Sequence of aMTD786
LVAIAPLAVLAP

SEQ ID NO: 177 - protein, 12 aa, Artificial Sequence
  Amino acid Sequence of aMTD787
AVALVPVIVAAP

SEQ ID NO: 178 - protein, 12 aa, Artificial Sequence
  Amino acid Sequence of aMTD788
AIAVAIAPVALP

SEQ ID NO: 179 - protein, 12 aa, Artificial Sequence
  Amino acid Sequence of aMTD803
AIALAVPVLALP

SEQ ID NO: 180 - protein, 12 aa, Artificial Sequence
  Amino acid Sequence of aMTD805
LVLIAAAPIALP

SEQ ID NO: 181 - protein, 12 aa, Artificial Sequence
  Amino acid Sequence of aMTD806
LVALAVPAAVLP

SEQ ID NO: 182 - protein, 12 aa, Artificial Sequence
  Amino acid Sequence of aMTD807
AVALAVPALVLP

SEQ ID NO: 183 - protein, 12 aa, Artificial Sequence
  Amino acid Sequence of aMTD808
LVVLAAAPLAVP

SEQ ID NO: 184 - protein, 12 aa, Artificial Sequence
  Amino acid Sequence of aMTD809
LIVLAAPALAAP

SEQ ID NO: 185 - protein, 12 aa, Artificial Sequence
  Amino acid Sequence of aMTD810
VIVLAAPALAAP

SEQ ID NO: 186 - protein, 12 aa, Artificial Sequence
  Amino acid Sequence of aMTD811
AVVLAVPALAVP

SEQ ID NO: 187 - protein, 12 aa, Artificial Sequence
  Amino acid Sequence of aMTD824
LIIVAAAPAVAP

SEQ ID NO: 188 - protein, 12 aa, Artificial Sequence
  Amino acid Sequence of aMTD825
IVAVIVAPAVAP

SEQ ID NO: 189 - protein, 12 aa, Artificial Sequence
  Amino acid Sequence of aMTD826
LVALAAPIIAVP

SEQ ID NO: 190 - protein, 12 aa, Artificial Sequence
  Amino acid Sequence of aMTD827
IAAVLAAPALVP

SEQ ID NO: 191 - protein, 12 aa, Artificial Sequence
  Amino acid Sequence of aMTD828
IALLAAPIIAVP

SEQ ID NO: 192 - protein, 12 aa, Artificial Sequence
  Amino acid Sequence of aMTD829
AALALVAPVIVP

SEQ ID NO: 193 - protein, 12 aa, Artificial Sequence
  Amino acid Sequence of aMTD830
IALVAAPVALVP

SEQ ID NO: 194 - protein, 12 aa, Artificial Sequence
  Amino acid Sequence of aMTD831
IIVAVAPAAIVP

SEQ ID NO: 195 - protein, 12 aa, Artificial Sequence
  Amino acid Sequence of aMTD832
AVAAIVPVIVAP

SEQ ID NO: 196 - protein, 12 aa, Artificial Sequence
  Amino acid Sequence of aMTD843
AVLVLVAPAAAP

SEQ ID NO: 197 - protein, 12 aa, Artificial Sequence
  Amino acid Sequence of aMTD844
VVALLAPLIAAP

SEQ ID NO: 198 - protein, 12 aa, Artificial Sequence
  Amino acid Sequence of aMTD845
AAVVIAPLLAVP

SEQ ID NO: 199 - protein, 12 aa, Artificial Sequence
  Amino acid Sequence of aMTD846
IAVAVAAPLLVP

SEQ ID NO: 200 - protein, 12 aa, Artificial Sequence
  Amino acid Sequence of aMTD847
LVAIVVLPAVAP

SEQ ID NO: 201 - protein, 12 aa, Artificial Sequence
  Amino acid Sequence of aMTD848
AVAIVVLPAVAP

SEQ ID NO: 202 - protein, 12 aa, Artificial Sequence
  Amino acid Sequence of aMTD849
AVILLAPLIAAP

SEQ ID NO: 203 - protein, 12 aa, Artificial Sequence
  Amino acid Sequence of aMTD850
LVIALAAPVALP

SEQ ID NO: 204 - protein, 12 aa, Artificial Sequence
  Amino acid Sequence of aMTD851
VLAVVLPAVALP

SEQ ID NO: 205 - protein, 12 aa, Artificial Sequence
  Amino acid Sequence of aMTD852
VLAVAAPAVLLP

SEQ ID NO: 206 - protein, 12 aa, Artificial Sequence
  Amino acid Sequence of aMTD863
AAVVLLPIIAAP

SEQ ID NO: 207 - protein, 12 aa, Artificial Sequence
  Amino acid Sequence of aMTD864
ALLVIAPAIAVP

SEQ ID NO: 208 - protein, 12 aa, Artificial Sequence
  Amino acid Sequence of aMTD865
AVLVIAVPAIAP

SEQ ID NO: 209 - protein, 12 aa, Artificial Sequence
  Amino acid Sequence of aMTD867
ALLVVIAPLAAP

SEQ ID NO: 210 - protein, 12 aa, Artificial Sequence
  Amino acid Sequence of aMTD868
VLVAAILPAAIP

SEQ ID NO: 211 - protein, 12 aa, Artificial Sequence
  Amino acid Sequence of aMTD870
VLVAAVLPIAAP

SEQ ID NO: 212 - protein, 12 aa, Artificial Sequence
  Amino acid Sequence of aMTD872
VLAAAVLPLVVP

SEQ ID NO: 213 - protein, 12 aa, Artificial Sequence
  Amino acid Sequence of aMTD875
AIAIVVPAVAVP

SEQ ID NO: 214 - protein, 12 aa, Artificial Sequence
  Amino acid Sequence of aMTD877
VAIIAVPAVVAP

SEQ ID NO: 215 - protein, 12 aa, Artificial Sequence
  Amino acid Sequence of aMTD878
IVALVAPAAVVP

SEQ ID NO: 216 - protein, 12 aa, Artificial Sequence
  Amino acid Sequence of aMTD879
AAIVLLPAVVVP

SEQ ID NO: 217 - protein, 12 aa, Artificial Sequence
  Amino acid Sequence of aMTD881
AALIVVPAVAVP

SEQ ID NO: 218 - protein, 12 aa, Artificial Sequence
  Amino acid Sequence of aMTD882
AIALVVPAVAVP

SEQ ID NO: 219 - protein, 12 aa, Artificial Sequence
  Amino acid Sequence of aMTD883
LAIVPAAIAALP

SEQ ID NO: 220 - protein, 12 aa, Artificial Sequence
  Amino acid Sequence of aMTD885
LVAIAPAVAVLP

SEQ ID NO: 221 - protein, 12 aa, Artificial Sequence
  Amino acid Sequence of aMTD887
VLAVAPAVAVLP

SEQ ID NO: 222 - protein, 12 aa, Artificial Sequence
  Amino acid Sequence of aMTD888
ILAVVAIPAAAP

SEQ ID NO: 223 - protein, 12 aa, Artificial Sequence
  Amino acid Sequence of aMTD889
ILVAAAPIAALP

SEQ ID NO: 224 - protein, 12 aa, Artificial Sequence
  Amino acid Sequence of aMTD891
ILAVAAIPAALP

SEQ ID NO: 225 - protein, 12 aa, Artificial Sequence
  Amino acid Sequence of aMTD893
VIAIPAILAAAP

SEQ ID NO: 226 - protein, 12 aa, Artificial Sequence
  Amino acid Sequence of aMTD895
AIIIVVPAIAAP

SEQ ID NO: 227 - protein, 12 aa, Artificial Sequence
  Amino acid Sequence of aMTD896
AILIVVAPIAAP

SEQ ID NO: 228 - protein, 12 aa, Artificial Sequence
  Amino acid Sequence of aMTD897
AVIVPVAIIAAP

SEQ ID NO: 229 - protein, 12 aa, Artificial Sequence
  Amino acid Sequence of aMTD899
AVVIALPAVVAP

SEQ ID NO: 230 - protein, 12 aa, Artificial Sequence
  Amino acid Sequence of aMTD900
ALVAVIAPVVAP

SEQ ID NO: 231 - protein, 12 aa, Artificial Sequence
  Amino acid Sequence of aMTD901
ALVAVLPAVAVP

SEQ ID NO: 232 - protein, 12 aa, Artificial Sequence
  Amino acid Sequence of aMTD902
ALVAPLLAVAVP

SEQ ID NO: 233 - protein, 12 aa, Artificial Sequence
  Amino acid Sequence of aMTD904
AVLAVVAPVVAP

SEQ ID NO: 234 - protein, 12 aa, Artificial Sequence
  Amino acid Sequence of aMTD905
AVIAVAPLVVAP

SEQ ID NO: 235 - protein, 12 aa, Artificial Sequence
  Amino acid Sequence of aMTD906
AVIALAPVVVAP

SEQ ID NO: 236 - protein, 12 aa, Artificial Sequence
  Amino acid Sequence of aMTD907
VAIALAPVVVAP

SEQ ID NO: 237 - protein, 12 aa, Artificial Sequence
  Amino acid Sequence of aMTD908
VALALAPVVVAP

SEQ ID NO: 238 - protein, 12 aa, Artificial Sequence
  Amino acid Sequence of aMTD910
VAALLPAVVVAP

SEQ ID NO: 239 - protein, 12 aa, Artificial Sequence
  Amino acid Sequence of aMTD911
VALALPAVVVAP

SEQ ID NO: 240 - protein, 12 aa, Artificial Sequence
  Amino acid Sequence of aMTD912
VALLAPAVVVAP

SEQ ID NO: 241 - DNA, 36 bp, Artificial Sequence
  Polynucleotide Sequence of aMTD1
gcggcggcgctggcgccggtggtgctggcgctgccg

SEQ ID NO: 242 - DNA, 36 bp, Artificial Sequence
  Polynucleotide Sequence of aMTD2
gcggcggcggtgccgctgctggcggtggtggtgccg

SEQ ID NO: 243 - DNA, 36 bp, Artificial Sequence
  Polynucleotide Sequence of aMTD3
gcggcgctgctggtgccggcggcggtgctggcgccg

SEQ ID NO: 244 - DNA, 36 bp, Artificial Sequence
  Polynucleotide Sequence of aMTD4
gcgctggcgctgctgccggtggcggcgctggcgccg

SEQ ID NO: 245 - DNA, 36 bp, Artificial Sequence
  Polynucleotide Sequence of aMTD5
gcggcggcgctgctgccggtggcgctggtggcgccg

SEQ ID NO: 246 - DNA, 36 bp, Artificial Sequence
  Polynucleotide Sequence of aMTD11
gtggtggcgctggcgccggcgctggcggcgctgccg

SEQ ID NO: 247 - DNA, 36 bp, Artificial Sequence
  Polynucleotide Sequence of aMTD12
ctgctggcggcggtgccggcggtgctgctggcgccg

SEQ ID NO: 248 - DNA, 36 bp, Artificial Sequence
  Polynucleotide Sequence of aMTD13
gcggcggcgctggtgccggtggtggcgctgctgccg

SEQ ID NO: 249 - DNA, 36 bp, Artificial Sequence
  Polynucleotide Sequence of aMTD21
gcggtggcgctgctgccggcgctgctggcggtgccg

SEQ ID NO: 250 - DNA, 36 bp, Artificial Sequence
  Polynucleotide Sequence of aMTD22
gcggtggtgctggtgccggtgctggcggcggcgccg

SEQ ID NO: 251 - DNA, 36 bp, Artificial Sequence
  Polynucleotide Sequence of aMTD23
gtggtgctggtgctgccggcggcggcggcggtgccg

SEQ ID NO: 252 - DNA, 36 bp, Artificial Sequence
  Polynucleotide Sequence of aMTD24
attgcgctggcggcgccggcgctgattgtggcgccg

SEQ ID NO: 253 - DNA, 36 bp, Artificial Sequence
  Polynucleotide Sequence of aMTD25
attgtggcggtggcgccggcgctggtggcgctgccg

SEQ ID NO: 254 - DNA, 36 bp, Artificial Sequence
  Polynucleotide Sequence of aMTD42
gtggcggcgctgccggtggtggcggtggtggcgccg

SEQ ID NO: 255 - DNA, 36 bp, Artificial Sequence
  Polynucleotide Sequence of aMTD43
ctgctggcggcgccgctggtggtggcggcggtgccg

SEQ ID NO: 256 - DNA, 36 bp, Artificial Sequence
  Polynucleotide Sequence of aMTD44
gcgctggcggtgccggtggcgctgctggtggcgccg

SEQ ID NO: 257 - DNA, 36 bp, Artificial Sequence
  Polynucleotide Sequence of aMTD61
gtggcggcgctgccggtgctgctggcggcgctgccg

SEQ ID NO: 258 - DNA, 36 bp, Artificial Sequence
  Polynucleotide Sequence of aMTD62
gtggcgctgctggcgccggtggcgctggcggtgccg

SEQ ID NO: 259 - DNA, 36 bp, Artificial Sequence
  Polynucleotide Sequence of aMTD63
gcggcgctgctggtgccggcgctggtggcggtgccg

SEQ ID NO: 260 - DNA, 36 bp, Artificial Sequence
  Polynucleotide Sequence of aMTD64
gcgattgtggcgctgccggtggcggtgctggcgccg

SEQ ID NO: 261 - DNA, 36 bp, Artificial Sequence
  Polynucleotide Sequence of aMTD65
attgcgattgtggcgccggtggtggcgctggcgccg

SEQ ID NO: 262 - DNA, 36 bp, Artificial Sequence
  Polynucleotide Sequence of aMTD81
gcggcgctgctgccggcgctggcggcgctgctgccg

SEQ ID NO: 263 - DNA, 36 bp, Artificial Sequence
  Polynucleotide Sequence of aMTD82
gcggtggtgctggcgccggtggcggcggtgctgccg

SEQ ID NO: 264 - DNA, 36 bp, Artificial Sequence
  Polynucleotide Sequence of aMTD83
ctggcggtggcggcgccgctggcgctggcgctgccg

SEQ ID NO: 265 - DNA, 36 bp, Artificial Sequence
  Polynucleotide Sequence of aMTD84
gcggcggtggcggcgccgctgctgctggcgctgccg

SEQ ID NO: 266 - DNA, 36 bp, Artificial Sequence
  Polynucleotide Sequence of aMTD85
ctgctggtgctgccggcggcggcgctggcggcgccg

SEQ ID NO: 267 - DNA, 36 bp, Artificial Sequence
  Polynucleotide Sequence of aMTD101
ctggtggcggtggcgccggtggcggcggtgctgccg

SEQ ID NO: 268 - DNA, 36 bp, Artificial Sequence
  Polynucleotide Sequence of aMTD102
ctggcgctggcgccggcggcgctggcgctgctgccg

SEQ ID NO: 269 - DNA, 36 bp, Artificial Sequence
  Polynucleotide Sequence of aMTD103
gcgctgattgcggcgccgattctggcgctggcgccg

SEQ ID NO: 270 - DNA, 36 bp, Artificial Sequence
  Polynucleotide Sequence of aMTD104
gcggtggtggcggcgccgctggtgctggcgctgccg

SEQ ID NO: 271 - DNA, 36 bp, Artificial Sequence
  Polynucleotide Sequence of aMTD105
ctgctggcgctggcgccggcggcgctgctggcgccg

SEQ ID NO: 272 - DNA, 36 bp, Artificial Sequence
  Polynucleotide Sequence of aMTD121
gcgattgtggcgctgccggcgctggcgctggcgccg

SEQ ID NO: 273 - DNA, 36 bp, Artificial Sequence
  Polynucleotide Sequence of aMTD123
gcggcgattattgtgccggcggcgctgctggcgccg

SEQ ID NO: 274 - DNA, 36 bp, Artificial Sequence
  Polynucleotide Sequence of aMTD124
attgcggtggcgctgccggcgctgattgcggcgccg

SEQ ID NO: 275 - DNA, 36 bp, Artificial Sequence
  Polynucleotide Sequence of aMTD141
gcggtgattgtgctgccggcgctggcggtggcgccg

SEQ ID NO: 276 - DNA, 36 bp, Artificial Sequence
  Polynucleotide Sequence of aMTD143
gcggtgctggcggtgccggcggtgctggtggcgccg

SEQ ID NO: 277 - DNA, 36 bp, Artificial Sequence
  Polynucleotide Sequence of aMTD144
gtgctggcgattgtgccggcggtggcgctggcgccg

SEQ ID NO: 278 - DNA, 36 bp, Artificial Sequence
  Polynucleotide Sequence of aMTD145
ctgctggcggtggtgccggcggtggcgctggcgccg

SEQ ID NO: 279 - DNA, 36 bp, Artificial Sequence
  Polynucleotide Sequence of aMTD161
gcggtgattgcgctgccggcgctgattgcggcgccg

SEQ ID NO: 280 - DNA, 36 bp, Artificial Sequence
  Polynucleotide Sequence of aMTD162
gcggtggtggcgctgccggcggcgctgattgtgccg

SEQ ID NO: 281 - DNA, 36 bp, Artificial Sequence
  Polynucleotide Sequence of aMTD163
ctggcgctggtgctgccggcggcgctggcggcgccg

SEQ ID NO: 282 - DNA, 36 bp, Artificial Sequence
  Polynucleotide Sequence of aMTD164
ctggcggcggtgctgccggcgctgctggcggcgccg

SEQ ID NO: 283 - DNA, 36 bp, Artificial Sequence
  Polynucleotide Sequence of aMTD165
gcgctggcggtgccggtggcgctggcgattgtgccg

SEQ ID NO: 284 - DNA, 36 bp, Artificial Sequence
  Polynucleotide Sequence of aMTD182
gcgctgattgcgccggtggtggcgctggtggcgccg

SEQ ID NO: 285 - DNA, 36 bp, Artificial Sequence
  Polynucleotide Sequence of aMTD183
ctgctggcggcgccggtggtgattgcgctggcgccg

SEQ ID NO: 286 - DNA, 36 bp, Artificial Sequence
  Polynucleotide Sequence of aMTD184
ctggcggcgattgtgccggcgattattgcggtgccg

SEQ ID NO: 287 - DNA, 36 bp, Artificial Sequence
  Polynucleotide Sequence of aMTD185
gcggcgctggtgctgccgctgattattgcggcgccg

SEQ ID NO: 288 - DNA, 36 bp, Artificial Sequence
  Polynucleotide Sequence of aMTD201
ctggcgctggcggtgccggcgctggcggcgctgccg

SEQ ID NO: 289 - DNA, 36 bp, Artificial Sequence
  Polynucleotide Sequence of aMTD204
ctgattgcggcgctgccggcggtggcggcgctgccg

SEQ ID NO: 290 - DNA, 36 bp, Artificial Sequence
  Polynucleotide Sequence of aMTD205
gcgctggcgctggtgccggcgattgcggcgctgccg

SEQ ID NO: 291 - DNA, 36 bp, Artificial Sequence
  Polynucleotide Sequence of aMTD221
gcggcgattctggcgccgattgtggcgctggcgccg

SEQ ID NO: 292 - DNA, 36 bp, Artificial Sequence
  Polynucleotide Sequence of aMTD222
gcgctgctgattgcgccggcggcggtgattgcgccg

SEQ ID NO: 293 - DNA, 36 bp, Artificial Sequence
  Polynucleotide Sequence of aMTD223
gcgattctggcggtgccgattgcggtggtggcgccg

SEQ ID NO: 294 - DNA, 36 bp, Artificial Sequence
  Polynucleotide Sequence of aMTD224
attctggcggcggtgccgattgcgctggcggcgccg

SEQ ID NO: 295 - DNA, 36 bp, Artificial Sequence
  Polynucleotide Sequence of aMTD225
gtggcggcgctgctgccggcggcggcggtgctgccg

SEQ ID NO: 296 - DNA, 36 bp, Artificial Sequence
  Polynucleotide Sequence of aMTD241
gcggcggcggtggtgccggtgctgctggtggcgccg

SEQ ID NO: 297 - DNA, 36 bp, Artificial Sequence
  Polynucleotide Sequence of aMTD242
gcggcgctgctggtgccggcgctggtggcggcgccg

SEQ ID NO: 298 - DNA, 36 bp, Artificial Sequence
  Polynucleotide Sequence of aMTD243
gcggcggtgctgctgccggtggcgctggcggcgccg

SEQ ID NO: 299 - DNA, 36 bp, Artificial Sequence
  Polynucleotide Sequence of aMTD245
gcggcggcgctggcgccggtgctggcgctggtgccg

SEQ ID NO: 300 - DNA, 36 bp, Artificial Sequence
  Polynucleotide Sequence of aMTD261
ctggtgctggtgccgctgctggcggcggcggcgccg

SEQ ID NO: 301 - DNA, 36 bp, Artificial Sequence
  Polynucleotide Sequence of aMTD262
gcgctgattgcggtgccggcgattattgtggcgccg

SEQ ID NO: 302 - DNA, 36 bp, Artificial Sequence
  Polynucleotide Sequence of aMTD263
gcgctggcggtgattccggcggcggcgattctgccg

SEQ ID NO: 303 - DNA, 36 bp, Artificial Sequence
  Polynucleotide Sequence of aMTD264
ctggcggcggcgccggtggtgattgtgattgcgccg

SEQ ID NO: 304 - DNA, 36 bp, Artificial Sequence
  Polynucleotide Sequence of aMTD265
gtgctggcgattgcgccgctgctggcggcggtgccg

SEQ ID NO: 305 - DNA, 36 bp, Artificial Sequence
  Polynucleotide Sequence of aMTD281
gcgctgattgtgctgccggcggcggtggcggtgccg

SEQ ID NO: 306 - DNA, 36 bp, Artificial Sequence
  Polynucleotide Sequence of aMTD282
gtgctggcggtggcgccggcgctgattgtggcgccg

SEQ ID NO: 307 - DNA, 36 bp, Artificial Sequence
  Polynucleotide Sequence of aMTD283
gcggcgctgctggcgccggcgctgattgtggcgccg

SEQ ID NO: 308 - DNA, 36 bp, Artificial Sequence
  Polynucleotide Sequence of aMTD284
gcgctgattgcgccggcggtggcgctgattgtgccg

SEQ ID NO: 309 - DNA, 36 bp, Artificial Sequence
  Polynucleotide Sequence of aMTD285
gcgattgtgctgctgccggcggcggtggtggcgccg

SEQ ID NO: 310 - DNA, 36 bp, Artificial Sequence
  Polynucleotide Sequence of aMTD301
gtgattgcggcgccggtgctggcggtgctggcgccg

SEQ ID NO: 311 - DNA, 36 bp, Artificial Sequence
  Polynucleotide Sequence of aMTD302
ctggcgctggcgccggcgctggcgctgctggcgccg

SEQ ID NO: 312 - DNA, 36 bp, Artificial Sequence
  Polynucleotide Sequence of aMTD304
gcgattattctggcgccgattgcggcgattgcgccg

SEQ ID NO: 313 - DNA, 36 bp, Artificial Sequence
  Polynucleotide Sequence of aMTD305
attgcgctggcggcgccgattctgctggcggcgccg

SEQ ID NO: 314 - DNA, 36 bp, Artificial Sequence
  Polynucleotide Sequence of aMTD321
attgtggcggtggcgctgccggcgctggcggtgccg

SEQ ID NO: 315 - DNA, 36 bp, Artificial Sequence
  Polynucleotide Sequence of aMTD322
gtggtggcgattgtgctgccggcgctggcggcgccg

SEQ ID NO: 316 - DNA, 36 bp, Artificial Sequence
  Polynucleotide Sequence of aMTD323
attgtggcggtggcgctgccggtggcgctggcgccg

SEQ ID NO: 317 - DNA, 36 bp, Artificial Sequence
  Polynucleotide Sequence of aMTD324
attgtggcggtggcgctgccggcggcgctggtgccg

SEQ ID NO: 318 - DNA, 36 bp, Artificial Sequence
  Polynucleotide Sequence of aMTD325
attgtggcggtggcgctgccggcggtggcgctgccg

SEQ ID NO: 319 - DNA, 36 bp, Artificial Sequence
  Polynucleotide Sequence of aMTD341
attgtggcggtggcgctgccggcggtgctggcgccg

SEQ ID NO: 320 - DNA, 36 bp, Artificial Sequence
  Polynucleotide Sequence of aMTD342
gtgattgtggcgctggcgccggcggtgctggcgccg

SEQ ID NO: 321 - DNA, 36 bp, Artificial Sequence
  Polynucleotide Sequence of aMTD343
attgtggcggtggcgctgccggcgctggtggcgccg

SEQ ID NO: 322 - DNA, 36 bp, Artificial Sequence
  Polynucleotide Sequence of aMTD345
gcgctgctgattgtggcgccggtggcggtggcgccg

SEQ ID NO: 323 - DNA, 36 bp, Artificial Sequence
  Polynucleotide Sequence of aMTD361
gcggtggtgattgtggcgccggcggtgattgcgccg

SEQ ID NO: 324 - DNA, 36 bp, Artificial Sequence
  Polynucleotide Sequence of aMTD363
gcggtgctggcggtggcgccggcgctgattgtgccg

SEQ ID NO: 325 - DNA, 36 bp, Artificial Sequence
  Polynucleotide Sequence of aMTD364
ctggtggcggcggtggcgccggcgctgattgtgccg

SEQ ID NO: 326 - DNA, 36 bp, Artificial Sequence
  Polynucleotide Sequence of aMTD365
gcggtgattgtggtggcgccggcgctgctggcgccg

SEQ ID NO: 327 - DNA, 36 bp, Artificial Sequence
  Polynucleotide Sequence of aMTD381
gtggtggcgattgtgctgccggcggtggcggcgccg

SEQ ID NO: 328 - DNA, 36 bp, Artificial Sequence
  Polynucleotide Sequence of aMTD382
gcggcggcgctggtgattccggcgattctggcgccg

SEQ ID NO: 329 - DNA, 36 bp, Artificial Sequence
  Polynucleotide Sequence of aMTD383
gtgattgtggcgctggcgccggcgctgctggcgccg

SEQ ID NO: 330 - DNA, 36 bp, Artificial Sequence
  Polynucleotide Sequence of aMTD384
gtgattgtggcgattgcgccggcgctgctggcgccg

SEQ ID NO: 331 - DNA, 36 bp, Artificial Sequence
  Polynucleotide Sequence of aMTD385
attgtggcgattgcggtgccggcgctggtggcgccg

SEQ ID NO: 332 - DNA, 36 bp, Artificial Sequence
  Polynucleotide Sequence of aMTD401
gcggcgctggcggtgattccggcggcgattctgccg

SEQ ID NO: 333 - DNA, 36 bp, Artificial Sequence
  Polynucleotide Sequence of aMTD402
gcgctggcggcggtgattccggcggcgattctgccg

SEQ ID NO: 334 - DNA, 36 bp, Artificial Sequence
  Polynucleotide Sequence of aMTD403
gcggcggcgctggtgattccggcggcgattctgccg

SEQ ID NO: 335 - DNA, 36 bp, Artificial Sequence
  Polynucleotide Sequence of aMTD404
ctggcggcggcggtgattccggcggcgattctgccg

SEQ ID NO: 336 - DNA, 36 bp, Artificial Sequence
  Polynucleotide Sequence of aMTD405
ctggcggcggcggtgattccggtggcgattctgccg

SEQ ID NO: 337 - DNA, 36 bp, Artificial Sequence
  Polynucleotide Sequence of aMTD421
gcggcgattctggcggcgccgctgattgcggtgccg

SEQ ID NO: 338 - DNA, 36 bp, Artificial Sequence
  Polynucleotide Sequence of aMTD422
gtggtggcgattctggcgccgctgctggcggcgccg

SEQ ID NO: 339 - DNA, 36 bp, Artificial Sequence
  Polynucleotide Sequence of aMTD424
gcggtggtggtggcggcgccggtgctggcgctgccg

SEQ ID NO: 340 - DNA, 36 bp, Artificial Sequence
  Polynucleotide Sequence of aMTD425
gcggtggtggcgattgcgccggtgctggcgctgccg

SEQ ID NO: 341 - DNA, 36 bp, Artificial Sequence
  Polynucleotide Sequence of aMTD442
gcgctggcggcgctggtgccggcggtgctggtgccg

SEQ ID NO: 342 - DNA, 36 bp, Artificial Sequence
  Polynucleotide Sequence of aMTD443
gcgctggcggcgctggtgccggtggcgctggtgccg

SEQ ID NO: 343 - DNA, 36 bp, Artificial Sequence
  Polynucleotide Sequence of aMTD444
ctggcggcggcgctggtgccggtggcgctggtgccg

SEQ ID NO: 344 - DNA, 36 bp, Artificial Sequence
  Polynucleotide Sequence of aMTD445
gcgctggcggcgctggtgccggcgctggtggtgccg

SEQ ID NO: 345 - DNA, 36 bp, Artificial Sequence
  Polynucleotide Sequence of aMTD461
attgcggcggtgattgtgccggcggtggcgctgccg

SEQ ID NO: 346 - DNA, 36 bp, Artificial Sequence
  Polynucleotide Sequence of aMTD462
attgcggcggtgctggtgccggcggtggcgctgccg

SEQ ID NO: 347 - DNA, 36 bp, Artificial Sequence
  Polynucleotide Sequence of aMTD463
gcggtggcgattctggtgccgctgctggcggcgccg

SEQ ID NO: 348 - DNA, 36 bp, Artificial Sequence
  Polynucleotide Sequence of aMTD464
gcggtggtgattctggtgccgctggcggcggcgccg

SEQ ID NO: 349 - DNA, 36 bp, Artificial Sequence
  Polynucleotide Sequence of aMTD465
attgcggcggtgattgtgccggtggcggcgctgccg

SEQ ID NO: 350 - DNA, 36 bp, Artificial Sequence
  Polynucleotide Sequence of aMTD481
gcgattgcgattgcgattgtgccggtggcgctgccg

SEQ ID NO: 351 - DNA, 36 bp, Artificial Sequence
  Polynucleotide Sequence of aMTD482
attctggcggtggcggcgattccggtggcggtgccg

SEQ ID NO: 352 - DNA, 36 bp, Artificial Sequence
  Polynucleotide Sequence of aMTD483
attctggcggcggcgattattccggcggcgctgccg

SEQ ID NO: 353 - DNA, 36 bp, Artificial Sequence
  Polynucleotide Sequence of aMTD484
ctggcggtggtgctggcggcgccggcgattgtgccg

SEQ ID NO: 354 - DNA, 36 bp, Artificial Sequence
  Polynucleotide Sequence of aMTD485
gcgattctggcggcgattgtgccgctggcggtgccg

SEQ ID NO: 355 - DNA, 36 bp, Artificial Sequence
  Polynucleotide Sequence of aMTD501
gtgattgtggcgctggcggtgccggcgctggcgccg

SEQ ID NO: 356 - DNA, 36 bp, Artificial Sequence
  Polynucleotide Sequence of aMTD502
gcgattgtggcgctggcggtgccggtgctggcgccg

SEQ ID NO: 357 - DNA, 36 bp, Artificial Sequence
  Polynucleotide Sequence of aMTD503
gcggcgattattattgtgctgccggcggcgctgccg

SEQ ID NO: 358 - DNA, 36 bp, Artificial Sequence
  Polynucleotide Sequence of aMTD504
ctgattgtggcgctggcggtgccggcgctggcgccg

SEQ ID NO: 359 - DNA, 36 bp, Artificial Sequence
  Polynucleotide Sequence of aMTD505
gcgattattattgtgattgcgccggcggcggcgccg

SEQ ID NO: 360 - DNA, 36 bp, Artificial Sequence
  Polynucleotide Sequence of aMTD521
ctggcggcgctgattgtggtgccggcggtggcgccg

SEQ ID NO: 361 - DNA, 36 bp, Artificial Sequence
  Polynucleotide Sequence of aMTD522
gcgctgctggtgattgcggtgccggcggtggcgccg

SEQ ID NO: 362 - DNA, 36 bp, Artificial Sequence
  Polynucleotide Sequence of aMTD524
gcggtggcgctgattgtggtgccggcgctggcgccg

SEQ ID NO: 363 - DNA, 36 bp, Artificial Sequence
  Polynucleotide Sequence of aMTD525
gcgctggcgattgtggtggcgccggtggcggtgccg

SEQ ID NO: 364 - DNA, 36 bp, Artificial Sequence
  Polynucleotide Sequence of aMTD541
ctgctggcgctgattattgcgccggcggcggcgccg

SEQ ID NO: 365 - DNA, 36 bp, Artificial Sequence
  Polynucleotide Sequence of aMTD542
gcgctggcgctgattattgtgccggcggtggcgccg

SEQ ID NO: 366 - DNA, 36 bp, Artificial Sequence
  Polynucleotide Sequence of aMTD543
ctgctggcggcgctgattgcgccggcggcgctgccg

SEQ ID NO: 367 - DNA, 36 bp, Artificial Sequence
  Polynucleotide Sequence of aMTD544
attgtggcgctgattgtggcgccggcggcggtgccg

SEQ ID NO: 368 - DNA, 36 bp, Artificial Sequence
  Polynucleotide Sequence of aMTD545
gtggtgctggtgctggcggcgccggcggcggtgccg

SEQ ID NO: 369 - DNA, 36 bp, Artificial Sequence
  Polynucleotide Sequence of aMTD561
gcggcggtggcgattgtgctgccggcggtggtgccg

SEQ ID NO: 370 - DNA, 36 bp, Artificial Sequence
  Polynucleotide Sequence of aMTD562
gcgctgattgcggcgattgtgccggcgctggtgccg

SEQ ID NO: 371 - DNA, 36 bp, Artificial Sequence
  Polynucleotide Sequence of aMTD563
gcgctggcggtgattgtggtgccggcgctggcgccg

SEQ ID NO: 372 - DNA, 36 bp, Artificial Sequence
  Polynucleotide Sequence of aMTD564
gtggcgattgcgctgattgtgccggcgctggcgccg

SEQ ID NO: 373 - DNA, 36 bp, Artificial Sequence
  Polynucleotide Sequence of aMTD565
gtggcgattgtgctggtggcgccggcggtggcgccg

SEQ ID NO: 374 - DNA, 36 bp, Artificial Sequence
  Polynucleotide Sequence of aMTD582
gtggcggtggcgctgattgtgccggcgctggcgccg

SEQ ID NO: 375 - DNA, 36 bp, Artificial Sequence
  Polynucleotide Sequence of aMTD583
gcggtgattctggcgctggcgccgattgtggcgccg

SEQ ID NO: 376 - DNA, 36 bp, Artificial Sequence
  Polynucleotide Sequence of aMTD585
gcgctgattgtggcgattgcgccggcgctggtgccg

SEQ ID NO: 377 - DNA, 36 bp, Artificial Sequence
  Polynucleotide Sequence of aMTD601
gcggcgattctgattgcggtgccgattgcggcgccg

SEQ ID NO: 378 - DNA, 36 bp, Artificial Sequence
  Polynucleotide Sequence of aMTD602
gtgattgtggcgctggcggcgccggtgctggcgccg

SEQ ID NO: 379 - DNA, 36 bp, Artificial Sequence
  Polynucleotide Sequence of aMTD603
gtgctggtggcgctggcggcgccggtgattgcgccg

SEQ ID NO: 380 - DNA, 36 bp, Artificial Sequence
  Polynucleotide Sequence of aMTD604
gtggcgctgattgcggtggcgccggcggtggtgccg

SEQ ID NO: 381 - DNA, 36 bp, Artificial Sequence
  Polynucleotide Sequence of aMTD605
gtgattgcggcggtgctggcgccggtggcggtgccg

SEQ ID NO: 382 - DNA, 36 bp, Artificial Sequence
  Polynucleotide Sequence of aMTD622
gcgctgattgtgctggcggcgccggtggcggtgccg

SEQ ID NO: 383 - DNA, 36 bp, Artificial Sequence
  Polynucleotide Sequence of aMTD623
gtggcggcggcgattgcgctgccggcgattgtgccg

SEQ ID NO: 384 - DNA, 36 bp, Artificial Sequence
  Polynucleotide Sequence of aMTD625
attctggcggcggcggcggcgccgctgattgtgccg

SEQ ID NO: 385 - DNA, 36 bp, Artificial Sequence
  Polynucleotide Sequence of aMTD643
ctggcgctggtgctggcggcgccggcgattgtgccg

SEQ ID NO: 386 - DNA, 36 bp, Artificial Sequence
  Polynucleotide Sequence of aMTD645
gcgctggcggtggtggcgctgccggcgattgtgccg

SEQ ID NO: 387 - DNA, 36 bp, Artificial Sequence
  Polynucleotide Sequence of aMTD661
gcggcgattctggcgccgattgtggcggcgctgccg

SEQ ID NO: 388 - DNA, 36 bp, Artificial Sequence
  Polynucleotide Sequence of aMTD664
attctgattgcgattgcgattccggcggcggcgccg

SEQ ID NO: 389 - DNA, 36 bp, Artificial Sequence
  Polynucleotide Sequence of aMTD665
ctggcgattgtgctggcggcgccggtggcggtgccg

SEQ ID NO: 390 - DNA, 36 bp, Artificial Sequence
  Polynucleotide Sequence of aMTD666
gcggcgattgcgattattgcgccggcgattgtgccg

SEQ ID NO: 391 - DNA, 36 bp, Artificial Sequence
  Polynucleotide Sequence of aMTD667
ctggcggtggcgattgtggcgccggcgctggtgccg

SEQ ID NO: 392 - DNA, 36 bp, Artificial Sequence
  Polynucleotide Sequence of aMTD683
ctggcgattgtgctggcggcgccggcggtgctgccg

SEQ ID NO: 393 - DNA, 36 bp, Artificial Sequence
  Polynucleotide Sequence of aMTD684
gcggcgattgtgctggcgctgccggcggtgctgccg

SEQ ID NO: 394 - DNA, 36 bp, Artificial Sequence
  Polynucleotide Sequence of aMTD685
gcgctgctggtggcggtgctgccggcggcgctgccg

SEQ ID NO: 395 - DNA, 36 bp, Artificial Sequence
  Polynucleotide Sequence of aMTD686
gcggcgctggtggcggtgctgccggtggcgctgccg

SEQ ID NO: 396 - DNA, 36 bp, Artificial Sequence
  Polynucleotide Sequence of aMTD687
attgtggcggtggcgctggtgccggcgctggcgccg

SEQ ID NO: 397 - DNA, 36 bp, Artificial Sequence; identical to SEQ ID NO: 396
  Polynucleotide Sequence of aMTD703

SEQ ID NO: 398 - DNA, 36 bp, Artificial Sequence
  Polynucleotide Sequence of aMTD705
attgtggcggtggcgctgctgccggcgctggcgccg

SEQ ID NO: 399 - DNA, 36 bp, Artificial Sequence
  Polynucleotide Sequence of aMTD706
attgtggcggtggcgctgctgccggcggtggcgccg

SEQ ID NO: 400 - DNA, 36 bp, Artificial Sequence
  Polynucleotide Sequence of aMTD707
attgtggcgctggcggtgctgccggcggtggcgccg

SEQ ID NO: 401 - DNA, 36 bp, Artificial Sequence
  Polynucleotide Sequence of aMTD724
gtggcggtgctggcggtgctgccggcgctggcgccg

SEQ ID NO: 402 - DNA, 36 bp, Artificial Sequence
  Polynucleotide Sequence of aMTD725
attgcggtgctggcggtggcgccggcggtgctgccg

SEQ ID NO: 403 - DNA, 36 bp, Artificial Sequence
  Polynucleotide Sequence of aMTD726
ctggcggtggcgattattgcgccggcggtggcgccg

SEQ ID NO: 404 - DNA, 36 bp, Artificial Sequence
  Polynucleotide Sequence of aMTD727
gtggcgctggcgattgcgctgccggcggtgctgccg

SEQ ID NO: 405 - DNA, 36 bp, Artificial Sequence
  Polynucleotide Sequence of aMTD743
gcgattgcgattgcgctggtgccggtggcgctgccg

SEQ ID NO: 406 - DNA, 36 bp, Artificial Sequence
  Polynucleotide Sequence of aMTD744
gcggcggtggtgattgtggcgccggtggcgctgccg

SEQ ID NO: 407 - DNA, 36 bp, Artificial Sequence
  Polynucleotide Sequence of aMTD746
gcggcgattctggcgattgtggcgccgctggcgccg

SEQ ID NO: 408 - DNA, 36 bp, Artificial Sequence
  Polynucleotide Sequence of aMTD747
gtggcgctgctggcgattgcgccggcgctggcgccg

SEQ ID NO: 409 - DNA, 36 bp, Artificial Sequence
  Polynucleotide Sequence of aMTD763
gtggcggtgctgattgcggtgccggcgctggcgccg

SEQ ID NO: 410 - DNA, 36 bp, Artificial Sequence
  Polynucleotide Sequence of aMTD764
gcggtggcgctggcggtgctgccggcggtggtgccg

SEQ ID NO: 411 - DNA, 36 bp, Artificial Sequence
  Polynucleotide Sequence of aMTD765
gcggtggcgctggcggtggtgccggcggtgctgccg

SEQ ID NO: 412 - DNA, 36 bp, Artificial Sequence
  Polynucleotide Sequence of aMTD766
attgtggtgattgcggtggcgccggcggtggcgccg

SEQ ID NO: 413 - DNA, 36 bp, Artificial Sequence
  Polynucleotide Sequence of aMTD767
attgtggtggcggcggtggtgccggcgctggcgccg

SEQ ID NO: 414 - DNA, 36 bp, Artificial Sequence
  Polynucleotide Sequence of aMTD783
attgtggcgctggtgccggcggtggcgattgcgccg

SEQ ID NO: 415 - DNA, 36 bp, Artificial Sequence
  Polynucleotide Sequence of aMTD784
gtggcggcgctgccggcggtggcgctggtggtgccg

SEQ ID NO: 416 - DNA, 36 bp, Artificial Sequence
  Polynucleotide Sequence of aMTD786
ctggtggcgattgcgccgctggcggtgctggcgccg

SEQ ID NO: 417 - DNA, 36 bp, Artificial Sequence
  Polynucleotide Sequence of aMTD787
gcggtggcgctggtgccggtgattgtggcggcgccg

SEQ ID NO: 418 - DNA, 36 bp, Artificial Sequence
  Polynucleotide Sequence of aMTD788
gcgattgcggtggcgattgcgccggtggcgctgccg

SEQ ID NO: 419 - DNA, 36 bp, Artificial Sequence
  Polynucleotide Sequence of aMTD803
gcgattgcgctggcggtgccggtgctggcgctgccg

SEQ ID NO: 420 - DNA, 36 bp, Artificial Sequence
  Polynucleotide Sequence of aMTD805
ctggtgctgattgcggcggcgccgattgcgctgccg

SEQ ID NO: 421 - DNA, 36 bp, Artificial Sequence
  Polynucleotide Sequence of aMTD806
ctggtggcgctggcggtgccggcggcggtgctgccg

SEQ ID NO: 422 - DNA, 36 bp, Artificial Sequence
  Polynucleotide Sequence of aMTD807
gcggtggcgctggcggtgccggcgctggtgctgccg

SEQ ID NO: 423 - DNA, 36 bp, Artificial Sequence
  Polynucleotide Sequence of aMTD808
ctggtggtgctggcggcggcgccgctggcggtgccg

SEQ ID NO: 424 - DNA, 36 bp, Artificial Sequence
  Polynucleotide Sequence of aMTD809
ctgattgtgctggcggcgccggcgctggcggcgccg

SEQ ID NO: 425 - DNA, 36 bp, Artificial Sequence
  Polynucleotide Sequence of aMTD810
gtgattgtgctggcggcgccggcgctggcggcgccg

SEQ ID NO: 426 - DNA, 36 bp, Artificial Sequence
  Polynucleotide Sequence of aMTD811
gcggtggtgctggcggtgccggcgctggcggtgccg

SEQ ID NO: 427 - DNA, 36 bp, Artificial Sequence
  Polynucleotide Sequence of aMTD824
ctgattattgtggcggcggcgccggcggtggcgccg

SEQ ID NO: 428 - DNA, 36 bp, Artificial Sequence
  Polynucleotide Sequence of aMTD825
attgtggcggtgattgtggcgccggcggtggcgccg

SEQ ID NO: 429 - DNA, 36 bp, Artificial Sequence
  Polynucleotide Sequence of aMTD826
ctggtggcgctggcggcgccgattattgcggtgccg

SEQ ID NO: 430 - DNA, 36 bp, Artificial Sequence
  Polynucleotide Sequence of aMTD827
attgcggcggtgctggcggcgccggcgctggtgccg

SEQ ID NO: 431 - DNA, 36 bp, Artificial Sequence
  Polynucleotide Sequence of aMTD828
attgcgctgctggcggcgccgattattgcggtgccg

SEQ ID NO: 432 - DNA, 36 bp, Artificial Sequence
  Polynucleotide Sequence of aMTD829
gcggcgctggcgctggtggcgccggtgattgtgccg

SEQ ID NO: 433 - DNA, 36 bp, Artificial Sequence
  Polynucleotide Sequence of aMTD830
attgcgctggtggcggcgccggtggcgctggtgccg

SEQ ID NO: 434 - DNA, 36 bp, Artificial Sequence
  Polynucleotide Sequence of aMTD831
attattgtggcggtggcgccggcggcgattgtgccg

SEQ ID NO: 435 - DNA, 36 bp, Artificial Sequence
  Polynucleotide Sequence of aMTD832
gcggtggcggcgattgtgccggtgattgtggcgccg

SEQ ID NO: 436 - DNA, 36 bp, Artificial Sequence
  Polynucleotide Sequence of aMTD843
gcggtgctggtgctggtggcgccggcggcggcgccg

SEQ ID NO: 437 - DNA, 36 bp, Artificial Sequence
  Polynucleotide Sequence of aMTD844
gtggtggcgctgctggcgccgctgattgcggcgccg

SEQ ID NO: 438 - DNA, 36 bp, Artificial Sequence
  Polynucleotide Sequence of aMTD845
gcggcggtggtgattgcgccgctgctggcggtgccg

SEQ ID NO: 439 - DNA, 36 bp, Artificial Sequence
  Polynucleotide Sequence of aMTD846
attgcggtggcggtggcggcgccgctgctggtgccg

SEQ ID NO: 440 - DNA, 36 bp, Artificial Sequence
  Polynucleotide Sequence of aMTD847
ctggtggcgattgtggtgctgccggcggtggcgccg

SEQ ID NO: 441 - DNA, 36 bp, Artificial Sequence
  Polynucleotide Sequence of aMTD848
gcggtggcgattgtggtgctgccggcggtggcgccg

SEQ ID NO: 442 - DNA, 36 bp, Artificial Sequence
  Polynucleotide Sequence of aMTD849
gcggtgattctgctggcgccgctgattgcggcgccg

SEQ ID NO: 443 - DNA, 36 bp, Artificial Sequence
  Polynucleotide Sequence of aMTD850
ctggtgattgcgctggcggcgccggtggcgctgccg

SEQ ID NO: 444 - DNA, 36 bp, Artificial Sequence
  Polynucleotide Sequence of aMTD851
gtgctggcggtggtgctgccggcggtggcgctgccg

SEQ ID NO: 445 - DNA, 36 bp, Artificial Sequence
  Polynucleotide Sequence of aMTD852
gtgctggcggtggcggcgccggcggtgctgctgccg

SEQ ID NO: 446 - DNA, 36 bp, Artificial Sequence
  Polynucleotide Sequence of aMTD863
gcggcggtggtgctgctgccgattattgcggcgccg

SEQ ID NO: 447 - DNA, 36 bp, Artificial Sequence
  Polynucleotide Sequence of aMTD864
gcgctgctggtgattgcgccggcgattgcggtgccg

SEQ ID NO: 448 - DNA, 36 bp, Artificial Sequence
  Polynucleotide Sequence of aMTD865
gcggtgctggtgattgcggtgccggcgattgcgccg

SEQ ID NO: 449 - DNA, 36 bp, Artificial Sequence
  Polynucleotide Sequence of aMTD867
gcgctgctggtggtgattgcgccgctggcggcgccg

SEQ ID NO: 450 - DNA, 36 bp, Artificial Sequence
  Polynucleotide Sequence of aMTD868
gtgctggtggcggcgattctgccggcggcgattccg

SEQ ID NO: 451 - DNA, 36 bp, Artificial Sequence
  Polynucleotide Sequence of aMTD870
gtgctggtggcggcggtgctgccgattgcggcgccg

SEQ ID NO: 452 - DNA, 36 bp, Artificial Sequence
  Polynucleotide Sequence of aMTD872
gtgctggcggcggcggtgctgccgctggtggtgccg

SEQ ID NO: 453 - DNA, 36 bp, Artificial Sequence
  Polynucleotide Sequence of aMTD875
gcgattgcgattgtggtgccggcggtggcggtgccg

SEQ ID NO: 454 - DNA, 36 bp, Artificial Sequence
  Polynucleotide Sequence of aMTD877
gtggcgattattgcggtgccggcggtggtggcgccg

SEQ ID NO: 455 - DNA, 36 bp, Artificial Sequence
  Polynucleotide Sequence of aMTD878
attgtggcgctggtggcgccggcggcggtggtgccg

SEQ ID NO: 456 - DNA, 36 bp, Artificial Sequence
  Polynucleotide Sequence of aMTD879
gcggcgattgtgctgctgccggcggtggtggtgccg

SEQ ID NO: 457 - DNA, 36 bp, Artificial Sequence
  Polynucleotide Sequence of aMTD881
gcggcgctgattgtggtgccggcggtggcggtgccg

SEQ ID NO: 458 - DNA, 36 bp, Artificial Sequence
  Polynucleotide Sequence of aMTD882
gcgattgcgctggtggtgccggcggtggcggtgccg

SEQ ID NO: 459 - DNA, 36 bp, Artificial Sequence
  Polynucleotide Sequence of aMTD883
ctggcgattgtgccggcggcgattgcggcgctgccg

SEQ ID NO: 460 - DNA, 36 bp, Artificial Sequence
  Polynucleotide Sequence of aMTD885
ctggtggcgattgcgccggcggtggcggtgctgccg

SEQ ID NO: 461 - DNA, 36 bp, Artificial Sequence
  Polynucleotide Sequence of aMTD887
gtgctggcggtggcgccggcggtggcggtgctgccg

SEQ ID NO: 462 - DNA, 36 bp, Artificial Sequence
  Polynucleotide Sequence of aMTD888
attctggcggtggtggcgattccggcggcggcgccg

SEQ ID NO: 463 - DNA, 36 bp, Artificial Sequence
  Polynucleotide Sequence of aMTD889
attctggtggcggcggcgccgattgcggcgctgccg

SEQ ID NO: 464 - DNA, 36 bp, Artificial Sequence
  Polynucleotide Sequence of aMTD891
attctggcggtggcggcgattccggcggcgctgccg

SEQ ID NO: 465 - DNA, 36 bp, Artificial Sequence
  Polynucleotide Sequence of aMTD893
gtgattgcgattccggcgattctggcggcggcgccg

SEQ ID NO: 466 - DNA, 36 bp, Artificial Sequence
  Polynucleotide Sequence of aMTD895
gcgattattattgtggtgccggcgattgcggcgccg

SEQ ID NO: 467 - DNA, 36 bp, Artificial Sequence
  Polynucleotide Sequence of aMTD896
gcgattctgattgtggtggcgccgattgcggcgccg

SEQ ID NO: 468 - DNA, 36 bp, Artificial Sequence
  Polynucleotide Sequence of aMTD897
gcggtgattgtgccggtggcgattattgcggcgccg

SEQ ID NO: 469 - DNA, 36 bp, Artificial Sequence
  Polynucleotide Sequence of aMTD899
gcggtggtgattgcgctgccggcggtggtggcgccg

SEQ ID NO: 470 - DNA, 36 bp, Artificial Sequence
  Polynucleotide Sequence of aMTD900
gcgctggtggcggtgattgcgccggtggtggcgccg

SEQ ID NO: 471 - DNA, 36 bp, Artificial Sequence
  Polynucleotide Sequence of aMTD901
gcgctggtggcggtgctgccggcggtggcggtgccg

SEQ ID NO: 472 - DNA, 36 bp, Artificial Sequence
  Polynucleotide Sequence of aMTD902
gcgctggtggcgccgctgctggcggtggcggtgccg

SEQ ID NO: 473 - DNA, 36 bp, Artificial Sequence
  Polynucleotide Sequence of aMTD904
gcggtgctggcggtggtggcgccggtggtggcgccg

SEQ ID NO: 474 - DNA, 36 bp, Artificial Sequence
  Polynucleotide Sequence of aMTD905
gcggtgattgcggtggcgccgctggtggtggcgccg

SEQ ID NO: 475 - DNA, 36 bp, Artificial Sequence
  Polynucleotide Sequence of aMTD906
gcggtgattgcgctggcgccggtggtggtggcgccg

SEQ ID NO: 476 - DNA, 36 bp, Artificial Sequence
  Polynucleotide Sequence of aMTD907
gtggcgattgcgctggcgccggtggtggtggcgccg

SEQ ID NO: 477 - DNA, 36 bp, Artificial Sequence
  Polynucleotide Sequence of aMTD908
gtggcgctggcgctggcgccggtggtggtggcgccg

SEQ ID NO: 478 - DNA, 36 bp, Artificial Sequence
  Polynucleotide Sequence of aMTD910
gtggcggcgctgctgccggcggtggtggtggcgccg

SEQ ID NO: 479 - DNA, 36 bp, Artificial Sequence
  Polynucleotide Sequence of aMTD911
gtggcgctggcgctgccggcggtggtggtggcgccg

SEQ ID NO: 480 - DNA, 36 bp, Artificial Sequence
  Polynucleotide Sequence of aMTD912
gtggcgctgctggcgccggcggtggtggtggcgccg

SEQ ID NO: 481 - DNA, 69 bp, Artificial Sequence
  Polynucleotide Sequence of aMTD1 5'-primer
gggtttcatatggcggcggcgctggcgccggtggtgctggcgctgccggcaaatattaccgttttctat

SEQ ID NO: 482 - DNA, 69 bp, Artificial Sequence
  Polynucleotide Sequence of aMTD2 5'-primer
gggtttcatatggcggcggcggtgccgctgctggcggtggtggtgccggcaaatattaccgttttctat

SEQ ID NO: 483 - DNA, 69 bp, Artificial Sequence
  Polynucleotide Sequence of aMTD3 5'-primer
gggtttcatatggcggcgctgctggtgccggcggcggtgctggcgccggcaaatattaccgttttctat

SEQ ID NO: 484 - DNA, 69 bp, Artificial Sequence
  Polynucleotide Sequence of aMTD4 5'-primer
gggtttcatatggcgctggcgctgctgccggtggcggcgctggcgccggcaaatattaccgttttctat

SEQ ID NO: 485 - DNA, 69 bp, Artificial Sequence
  Polynucleotide Sequence of aMTD5 5'-primer
gggtttcatatggcggcggcgctgctgccggtggcgctggtggcgccggcaaatattaccgttttctat

SEQ ID NO: 486 - DNA, 69 bp, Artificial Sequence
  Polynucleotide Sequence of aMTD6 5'-primer
gggtttcatatggtgattgcgatgattccggcggcgttttgggtggcggcaaatattaccgttttctat

SEQ ID NO: 487 - DNA, 69 bp, Artificial Sequence
  Polynucleotide Sequence of aMTD9 5'-primer
gggtttcatatggtggcgctggtgccggcggcgctgattctgccgccggcaaatattaccgttttctat

SEQ ID NO: 488 - DNA, 69 bp, Artificial Sequence
  Polynucleotide Sequence of aMTD11 5'-primer
gggtttcatatggtggtggcgctggcgccggcgctggcggcgctgccggcaaatattaccgttttctat

SEQ ID NO: 489 - DNA, 69 bp, Artificial Sequence
  Polynucleotide Sequence of aMTD12 5'-primer
gggtttcatatgctgctggcggcggtgccggcggtgctgctggcgccggcaaatattaccgttttctat

SEQ ID NO: 490 - DNA, 69 bp, Artificial Sequence
  Polynucleotide Sequence of aMTD13 5'-primer
gggtttcatatggcggcggcgctggtgccggtggtggcgctgctgccggcaaatattaccgttttctat

SEQ ID NO: 491 - DNA, 69 bp, Artificial Sequence
  Polynucleotide Sequence of aMTD16 5'-primer
gggtttcatatgaacaacagctgcaccacctataccaacggcagccaggcaaatattaccgttttctat

SEQ ID NO: 492 - DNA, 69 bp, Artificial Sequence
  Polynucleotide Sequence of aMTD17 5'-primer
gggtttcatatgggcggctgcagcgcgccgcagaccacctgcagcaacgcaaatattaccgttttctat

SEQ ID NO: 493 - DNA, 69 bp, Artificial Sequence
  Polynucleotide Sequence of aMTD18 5'-primer
gggtttcatatgaactattgctgcaccccgaccaccaacggccagagcgcaaatattaccgttttctat

SEQ ID NO: 494 - DNA, 69 bp, Artificial Sequence
  Polynucleotide Sequence of aMTD19 5'-primer
gggtttcatatgtatgtgagctgctgcacctataccaacggcagccaggcaaatattaccgttttctat

SEQ ID NO: 495 - DNA, 69 bp, Artificial Sequence
  Polynucleotide Sequence of aMTD20 5'-primer
gggtttcatatgaactattgcaacacctgcccgacctatggccagagcgcaaatattaccgttttctat

SEQ ID NO: 496 - DNA, 69 bp, Artificial Sequence
  Polynucleotide Sequence of aMTD21 5'-primer
gggtttcatatggcggtggcgctgctgccggcgctgctggcggtgccggcaaatattaccgttttctat

SEQ ID NO: 497 - DNA, 69 bp, Artificial Sequence
  Polynucleotide Sequence of aMTD22 5'-primer
gggtttcatatggcggtggtgctggtgccggtgctggcggcggcgccggcaaatattaccgttttctat

SEQ ID NO: 498 - DNA, 69 bp, Artificial Sequence
  Polynucleotide Sequence of aMTD23 5'-primer
gggtttcatatggtggtgctggtgctgccggcggcggcggcggtgccggcaaatattaccgttttctat

SEQ ID NO: 499 - DNA, 69 bp, Artificial Sequence
  Polynucleotide Sequence of aMTD24 5'-primer
gggtttcatatgattgcgctggcggcgccggcgctgattgtggcgccggcaaatattaccgttttctat

SEQ ID NO: 500 - DNA, 69 bp, Artificial Sequence
  Polynucleotide Sequence of aMTD25 5'-primer
gggtttcatatgattgtggcggtggcgccggcgctggtggcgctgccggcaaatattaccgttttctat

SEQ ID NO: 501 - DNA, 69 bp, Artificial Sequence
  Polynucleotide Sequence of aMTD26 5'-primer
gggtttcatatggcggcgattgcgctggcggcgccgctggcgattgtggcaaatattaccgttttctat

SEQ ID NO: 502 - DNA, 69 bp, Artificial Sequence
  Polynucleotide Sequence of aMTD27 5'-primer
gggtttcatatgctggcgattgtggcggcggcggcggcgctggtggcggcaaatattaccgttttctat

SEQ ID NO: 503 - DNA, 69 bp, Artificial Sequence
  Polynucleotide Sequence of aMTD28 5'-primer
gggtttcatatggcggtgccgctgctgccgctggtgccggcggtgccggcaaatattaccgttttctat

SEQ ID NO: 504 - DNA, 69 bp, Artificial Sequence
  Polynucleotide Sequence of aMTD29 5'-primer
gggtttcatatggtgctgccgccgctgccggtgctgccggtgctgccggcaaatattaccgttttctat

SEQ ID NO: 505 - DNA, 69 bp, Artificial Sequence
  Polynucleotide Sequence of aMTD30 5'-primer
gggtttcatatggcgatggcgctgctgccggcggcggtggcggtggcggcaaatattaccgttttctat

SEQ ID NO: 506 - DNA, 69 bp, Artificial Sequence
  Polynucleotide Sequence of aMTD33 5'-primer
gggtttcatatggcggcggcgattctggcgccggcgtttctggcggtggcaaatattaccgttttctat

SEQ ID NO: 507 - DNA, 69 bp, Artificial Sequence
  Polynucleotide Sequence of aMTD37 5'-primer
gggtttcatatgtattataaccagagcacctgcggcggccagtgctatgcaaatattaccgttttctat

SEQ ID NO: 508 - DNA, 69 bp, Artificial Sequence
  Polynucleotide Sequence of aMTD38 5'-primer
gggtttcatatgaccacctgcagccagcagcagtattgcaccaacggcgcaaatattaccgttttctat

SEQ ID NO: 509 - DNA, 69 bp, Artificial Sequence
  Polynucleotide Sequence of aMTD39 5'-primer
gggtttcatatgtgctataacaccagcccgtgcaccggctgctgctatgcaaatattaccgttttctat

SEQ ID NO: 510 - DNA, 69 bp, Artificial Sequence
  Polynucleotide Sequence of aMTD40 5'-primer
gggtttcatatgacctataacaccagctgcaccccgggcacctgctatgcaaatattaccgttttctat

SEQ ID NO: 511 - DNA, 69 bp, Artificial Sequence
  Polynucleotide Sequence of aMTD42 5'-primer
gggtttcatatggtggcggcgctgccggtggtggcggtggtggcgccggcaaatattaccgttttctat

SEQ ID NO: 512 - DNA, 69 bp, Artificial Sequence
  Polynucleotide Sequence of aMTD43 5'-primer
gggtttcatatgctgctggcggcgccgctggtggtggcggcggtgccggcaaatattaccgttttctat

SEQ ID NO: 513 - DNA, 69 bp, Artificial Sequence
  Polynucleotide Sequence of aMTD44 5'-primer
gggtttcatatggcgctggcggtgccggtggcgctgctggtggcgccggcaaatattaccgttttctat

SEQ ID NO: 514 - DNA, 69 bp, Artificial Sequence
  Polynucleotide Sequence of aMTD49 5'-primer
gggtttcatatggtggtgccggcggcgccggcggtgccggtggtgccggcaaatattaccgttttctat

SEQ ID NO: 515 - DNA, 69 bp, Artificial Sequence
  Polynucleotide Sequence of aMTD54 5'-primer
gggtttcatatgctggcggtggcggcgccgccggtggtggcgctgctggcaaatattaccgttttctat

SEQ ID NO: 516 - DNA, 69 bp, Artificial Sequence
  Polynucleotide Sequence of aMTD57 5'-primer
gggtttcatatgcagaacaactgcaacaccagcagccagggcggcggcgcaaatattaccgttttctat

SEQ ID NO: 517 - DNA, 69 bp, Artificial Sequence
  Polynucleotide Sequence of aMTD59 5'-primer
gggtttcatatggcggtgctggcggcgccggtggtggcggcgctggcggcaaatattaccgttttctat

SEQ ID NO: 518 - DNA, 69 bp, Artificial Sequence
  Polynucleotide Sequence of aMTD61 5'-primer
gggtttcatatggtggcggcgctgccggtgctgctggcggcgctgccggcaaatattaccgttttctat

SEQ ID NO: 519 - DNA, 69 bp, Artificial Sequence
  Polynucleotide Sequence of aMTD62 5'-primer
gggtttcatatggtggcgctgctggcgccggtggcgctggcggtgccggcaaatattaccgttttctat

SEQ ID NO: 520 - DNA, 69 bp, Artificial Sequence
  Polynucleotide Sequence of aMTD63 5'-primer
gggtttcatatggcggcgctgctggtgccggcgctggtggcggtgccggcaaatattaccgttttctat

SEQ ID NO: 521 - DNA, 69 bp, Artificial Sequence
  Polynucleotide Sequence of aMTD64 5'-primer
gggtttcatatggcgattgtggcgctgccggtggcggtgctggcgccggcaaatattaccgttttctat

SEQ ID NO: 522 - DNA, 69 bp, Artificial Sequence
  Polynucleotide Sequence of aMTD65 5'-primer
gggtttcatatgattgcgattgtggcgccggtggtggcgctggcgccggcaaatattaccgttttctat

SEQ ID NO: 523 - DNA, 69 bp, Artificial Sequence
  Polynucleotide Sequence of aMTD66 5'-primer
gggtttcatatggcgggcgtgctgggcggcccgattatgggcgtgccggcaaatattaccgttttctat

SEQ ID NO: 524 - DNA, 69 bp, Artificial Sequence
  Polynucleotide Sequence of aMTD67 5'-primer
gggtttcatatgctggatgcggaagtgccgctggcggatgatgtgccggcaaatattaccgttttctat

SEQ ID NO: 525 - DNA, 69 bp, Artificial Sequence
  Polynucleotide Sequence of aMTD68 5'-primer
gggtttcatatggtggcgccggtgctgccggcggcgccgctggtgccggcaaatattaccgttttctat

SEQ ID NO: 526 - DNA, 69 bp, Artificial Sequence
  Polynucleotide Sequence of aMTD69 5'-primer
gggtttcatatgccggtggcggtgctgccgccggcggcgctggtgccggcaaatattaccgttttctat

SEQ ID NO: 527 - DNA, 69 bp, Artificial Sequence
  Polynucleotide Sequence of aMTD71 5'-primer
gggtttcatatgtttatgtggatgtggtttccgtttatgtggtatccggcaaatattaccgttttctat

SEQ ID NO: 528 - DNA, 69 bp, Artificial Sequence
  Polynucleotide Sequence of aMTD77 5'-primer
gggtttcatatggcgatgctgctgatgccgattgtgctgattgcgccggcaaatattaccgttttctat

SEQ ID NO: 529 - DNA, 69 bp, Artificial Sequence
  Polynucleotide Sequence of aMTD81 5'-primer
gggtttcatatggcggcgctgctgccggcgctggcggcgctgctgccggcaaatattaccgttttctat

SEQ ID NO: 530 - DNA, 69 bp, Artificial Sequence
  Polynucleotide Sequence of aMTD82 5'-primer
gggtttcatatggcggtggtgctggcgccggtggcggcggtgctgccggcaaatattaccgttttctat

SEQ ID NO: 531 - DNA, 69 bp, Artificial Sequence
  Polynucleotide Sequence of aMTD83 5'-primer
gggtttcatatgctggcggtggcggcgccgctggcgctggcgctgccggcaaatattaccgttttctat

SEQ ID NO: 532 - DNA, 69 bp, Artificial Sequence
  Polynucleotide Sequence of aMTD84 5'-primer
gggtttcatatggcggcggtggcggcgccgctgctgctggcgctgccggcaaatattaccgttttctat

SEQ ID NO: 533 - DNA, 69 bp, Artificial Sequence
  Polynucleotide Sequence of aMTD85 5'-primer
gggtttcatatgctgctggtgctgccggcggcggcgctggcggcgccggcaaatattaccgttttctat

SEQ ID NO: 534 - DNA, 69 bp, Artificial Sequence
  Polynucleotide Sequence of aMTD97 5'-primer
gggtttcatatggcgctgctggcggcgccgccggcgctgctggcgctggcaaatattaccgttttctat

SEQ ID NO: 535 - DNA, 69 bp, Artificial Sequence
  Polynucleotide Sequence of aMTD101 5'-primer
gggtttcatatgctggtggcggtggcgccggtggcggcggtgctgccggcaaatattaccgttttctat

SEQ ID NO: 536 - DNA, 69 bp, Artificial Sequence
  Polynucleotide Sequence of aMTD102 5'-primer
gggtttcatatgctggcgctggcgccggcggcgctggcgctgctgccggcaaatattaccgttttctat

SEQ ID NO: 537 - DNA, 69 bp, Artificial Sequence
  Polynucleotide Sequence of aMTD103 5'-primer
gggtttcatatggcgctgattgcggcgccgattctggcgctggcgccggcaaatattaccgttttctat

SEQ ID NO: 538 - DNA, 69 bp, Artificial Sequence
  Polynucleotide Sequence of aMTD104 5'-primer
gggtttcatatggcggtggtggcggcgccgctggtgctggcgctgccggcaaatattaccgttttctat

SEQ ID NO: 539 - DNA, 69 bp, Artificial Sequence
  Polynucleotide Sequence of aMTD105 5'-primer
gggtttcatatgctgctggcgctggcgccggcggcgctgctggcgccggcaaatattaccgttttctat

SEQ ID NO: 540 - DNA, 69 bp, Artificial Sequence
  Polynucleotide Sequence of aMTD113 5'-primer
gggtttcatatgccggtggcggtggcgctgctgattgcggtgccgccggcaaatattaccgttttctat

SEQ ID NO: 541 - DNA, 69 bp, Artificial Sequence
  Polynucleotide Sequence of aMTD121 5'-primer
gggtttcatatggcgattgtggcgctgccggcgctggcgctggcgccggcaaatattaccgttttctat

SEQ ID NO: 542 - DNA, 69 bp, Artificial Sequence
  Polynucleotide Sequence of aMTD123 5'-primer
gggtttcatatggcggcgattattgtgccggcggcgctgctggcgccggcaaatattaccgttttctat

SEQ ID NO: 543 - DNA, 69 bp, Artificial Sequence
  Polynucleotide Sequence of aMTD124 5'-primer
gggtttcatatgattgcggtggcgctgccggcgctgattgcggcgccggcaaatattaccgttttctat

SEQ ID NO: 544 - DNA, 69 bp, Artificial Sequence
  Polynucleotide Sequence of aMTD131 5'-primer
gggtttcatatgtggattattgcgccggtgtggctggcgtggattgcggcaaatattaccgttttctat

SEQ ID NO: 545 - DNA, 69 bp, Artificial Sequence
  Polynucleotide Sequence of aMTD138 5'-primer
gggtttcatatgccgccggcggcgctgctggcgattctggcggtggcggcaaatattaccgttttctat

SEQ ID NO: 546 - DNA, 69 bp, Artificial Sequence
  Polynucleotide Sequence of aMTD139 5'-primer
gggtttcatatgaccggcagcaccaacagcccgacctgcaccagcaccgcaaatattaccgttttctat

SEQ ID NO: 547 - DNA, 69 bp, Artificial Sequence
  Polynucleotide Sequence of aMTD141 5'-primer
gggtttcatatggcggtgattgtgctgccggcgctggcggtggcgccggcaaatattaccgttttctat

SEQ ID NO: 548 - DNA, 69 bp, Artificial Sequence
  Polynucleotide Sequence of aMTD142 5'-primer
gggtttcatatgctgctggcggcggtgccggtggcgctggtggcgccggcaaatattaccgttttctat

SEQ ID NO: 549 - DNA, 69 bp, Artificial Sequence
  Polynucleotide Sequence of aMTD143 5'-primer
gggtttcatatggcggtgctggcggtgccggcggtgctggtggcgccggcaaatattaccgttttctat

SEQ ID NO: 550 - DNA, 69 bp, Artificial Sequence; identical to SEQ ID NO: 549
  Polynucleotide Sequence of aMTD144 5'-primer

SEQ ID NO: 551 - DNA, 69 bp, Artificial Sequence
  Polynucleotide Sequence of aMTD145 5'-primer
gggtttcatatgctgctggcggtggtgccggcggtggcgctggcgccggcaaatattaccgttttctat

SEQ ID NO: 552 - DNA, 69 bp, Artificial Sequence
  Polynucleotide Sequence of aMTD152 5'-primer
gggtttcatatgctggcggcggcggtggcggcggtggcggcgctgctggcaaatattaccgttttctat

SEQ ID NO: 553 - DNA, 69 bp, Artificial Sequence
  Polynucleotide Sequence of aMTD159 5'-primer
gggtttcatatgtgctatagcggcagcaccagccagaaccagccgccggcaaatattaccgttttctat

SEQ ID NO: 554 - DNA, 69 bp, Artificial Sequence
  Polynucleotide Sequence of aMTD161 5'-primer
gggtttcatatggcggtgattgcgctgccggcgctgattgcggcgccggcaaatattaccgttttctat

SEQ ID NO: 555 - DNA, 69 bp, Artificial Sequence
  Polynucleotide Sequence of aMTD162 5'-primer
gggtttcatatggcggtggtggcgctgccggcggcgctgattgtgccggcaaatattaccgttttctat

SEQ ID NO: 556 - DNA, 69 bp, Artificial Sequence
  Polynucleotide Sequence of aMTD163 5'-primer
gggtttcatatgctggcgctggtgctgccggcggcgctggcggcgccggcaaatattaccgttttctat

SEQ ID NO: 557 - DNA, 69 bp, Artificial Sequence
  Polynucleotide Sequence of aMTD164 5'-primer
gggtttcatatgctggcggcggtgctgccggcgctgctggcggcgccggcaaatattaccgttttctat

SEQ ID NO: 558 - DNA, 69 bp, Artificial Sequence
  Polynucleotide Sequence of aMTD165 5'-primer
gggtttcatatggcgctggcggtgccggtggcgctggcgattgtgccggcaaatattaccgttttctat

SEQ ID NO: 559 - DNA, 69 bp, Artificial Sequence
  Polynucleotide Sequence of aMTD167 5'-primer
gggtttcatatggtggcgattgcgattccggcggcgctggcgattccggcaaatattaccgttttctat

SEQ ID NO: 560 - DNA, 69 bp, Artificial Sequence
  Polynucleotide Sequence of aMTD169 5'-primer
gggtttcatatggtggcgctggtggcgccggcgctgattctggcgccggcaaatattaccgttttctat

SEQ ID NO: 561 - DNA, 69 bp, Artificial Sequence
  Polynucleotide Sequence of aMTD182 5'-primer
gggtttcatatggcgctgattgcgccggtggtggcgctggtggcgccggcaaatattaccgttttctat

SEQ ID NO: 562 - DNA, 69 bp, Artificial Sequence
  Polynucleotide Sequence of aMTD183 5'-primer
gggtttcatatgctgctggcggcgccggtggtgattgcgctggcgccggcaaatattaccgttttctat

SEQ ID NO: 563 - DNA, 69 bp, Artificial Sequence
  Polynucleotide Sequence of aMTD184 5'-primer
gggtttcatatgctggcggcgattgtgccggcgattattgcggtgccggcaaatattaccgttttctat

SEQ ID NO: 564 - DNA, 69 bp, Artificial Sequence
  Polynucleotide Sequence of aMTD185 5'-primer
gggtttcatatggcggcgctggtgctgccgctgattattgcggcgccggcaaatattaccgttttctat

SEQ ID NO: 565 - DNA, 69 bp, Artificial Sequence
  Polynucleotide Sequence of aMTD189 5'-primer
gggtttcatatggtgattctggtggcgccggcggtgattgcgccgccggcaaatattaccgttttctat

SEQ ID NO: 566 - DNA, 69 bp, Artificial Sequence
  Polynucleotide Sequence of aMTD190 5'-primer
gggtttcatatggcggcgattctggcgccggcggtgattgcgccgccggcaaatattaccgttttctat

SEQ ID NO: 567 - DNA, 69 bp, Artificial Sequence
  Polynucleotide Sequence of aMTD201 5'-primer
gggtttcatatgctggcgctggcggtgccggcgctggcggcgctgccggcaaatattaccgttttctat

SEQ ID NO: 568 - DNA, 69 bp, Artificial Sequence
  Polynucleotide Sequence of aMTD204 5'-primer
gggtttcatatgctgattgcggcgctgccggcggtggcggcgctgccggcaaatattaccgttttctat

SEQ ID NO: 569 - DNA, 69 bp, Artificial Sequence
  Polynucleotide Sequence of aMTD205 5'-primer
gggtttcatatggcgctggcgctggtgccggcgattgcggcgctgccggcaaatattaccgttttctat

SEQ ID NO: 570 - DNA, 69 bp, Artificial Sequence
  Polynucleotide Sequence of aMTD210 5'-primer
gggtttcatatggcgctgattgcgctgccggcgctgccggcgctgccggcaaatattaccgttttctat

SEQ ID NO: 571 - DNA, 69 bp, Artificial Sequence
  Polynucleotide Sequence of aMTD214 5'-primer
gggtttcatatggcgctgattgtggcgccggcgctgatggcgctgccggcaaatattaccgttttctat

SEQ ID NO: 572 - DNA, 69 bp, Artificial Sequence
  Polynucleotide Sequence of aMTD221 5'-primer
gggtttcatatggcggcgattctggcgccgattgtggcgctggcgccggcaaatattaccgttttctat

SEQ ID NO: 573 - DNA, 69 bp, Artificial Sequence
  Polynucleotide Sequence of aMTD222 5'-primer
gggtttcatatggcgctgctgattgcgccggcggcggtgattgcgccggcaaatattaccgttttctat

SEQ ID NO: 574 - DNA, 69 bp, Artificial Sequence
  Polynucleotide Sequence of aMTD223 5'-primer
gggtttcatatggcgattctggcggtgccgattgcggtggtggcgccggcaaatattaccgttttctat

SEQ ID NO: 575 - DNA, 69 bp, Artificial Sequence
  Polynucleotide Sequence of aMTD224 5'-primer
gggtttcatatgattctggcggcggtgccgattgcgctggcggcgccggcaaatattaccgttttctat

SEQ ID NO: 576 - DNA, 69 bp, Artificial Sequence
  Polynucleotide Sequence of aMTD225 5'-primer
gggtttcatatggtggcggcgctgctgccggcggcggcggtgctgccggcaaatattaccgttttctat

SEQ ID NO: 577 - DNA, 69 bp, Artificial Sequence
  Polynucleotide Sequence of aMTD226 5'-primer
gggtttcatatggcgctggtggcggcgattccggcgctggcgattccggcaaatattaccgttttctat

SEQ ID NO: 578 - DNA, 69 bp, Artificial Sequence
  Polynucleotide Sequence of aMTD227 5'-primer
gggtttcatatgctggcggcgattgtgccgattgcggcggcggtgccggcaaatattaccgttttctat

SEQ ID NO: 579 - DNA, 69 bp, Artificial Sequence
  Polynucleotide Sequence of aMTD241 5'-primer
gggtttcatatggcggcggcggtggtgccggtgctgctggtggcgccggcaaatattaccgttttctat

SEQ ID NO: 580 - DNA, 69 bp, Artificial Sequence
  Polynucleotide Sequence of aMTD242 5'-primer
gggtttcatatggcggcgctgctggtgccggcgctggtggcggcgccggcaaatattaccgttttctat

SEQ ID NO: 581 - DNA, 69 bp, Artificial Sequence
  Polynucleotide Sequence of aMTD243 5'-primer
gggtttcatatggcggcggtgctgctgccggtggcgctggcggcgccggcaaatattaccgttttctat

SEQ ID NO: 582 - DNA, 69 bp, Artificial Sequence
  Polynucleotide Sequence of aMTD245 5'-primer
gggtttcatatggcggcggcgctggcgccggtgctggcgctggtgccggcaaatattaccgttttctat

SEQ ID NO: 583 - DNA, 69 bp, Artificial Sequence
  Polynucleotide Sequence of aMTD246 5'-primer
gggtttcatatggtggtggcggtgccgctgctggtggcgtttgcggcggcaaatattaccgttttctat

SEQ ID NO: 584 - DNA, 69 bp, Artificial Sequence
  Polynucleotide Sequence of aMTD248 5'-primer
gggtttcatatggtggcggcgattgtgccgattgcggcgctggtgccggcaaatattaccgttttctat

SEQ ID NO: 585 - DNA, 69 bp, Artificial Sequence
  Polynucleotide Sequence of aMTD261 5'-primer
gggtttcatatgctggtgctggtgccgctgctggcggcggcggcgccggcaaatattaccgttttctat

SEQ ID NO: 586 - DNA, 69 bp, Artificial Sequence
  Polynucleotide Sequence of aMTD262 5'-primer
gggtttcatatggcgctgattgcggtgccggcgattattgtggcgccggcaaatattaccgttttctat

SEQ ID NO: 587 - DNA, 69 bp, Artificial Sequence
  Polynucleotide Sequence of aMTD263 5'-primer
gggtttcatatggcgctggcggtgattccggcggcggcgattctgccggcaaatattaccgttttctat

SEQ ID NO: 588 - DNA, 69 bp, Artificial Sequence
  Polynucleotide Sequence of aMTD264 5'-primer
gggtttcatatgctggcggcggcgccggtggtgattgtgattgcgccggcaaatattaccgttttctat

SEQ ID NO: 589 - DNA, 69 bp, Artificial Sequence
  Polynucleotide Sequence of aMTD265 5'-primer
gggtttcatatggtgctggcgattgcgccgctgctggcggcggtgccggcaaatattaccgttttctat

SEQ ID NO: 590 - DNA, 69 bp, Artificial Sequence
  Polynucleotide Sequence of aMTD281 5'-primer
gggtttcatatggcgctgattgtgctgccggcggcggtggcggtgccggcaaatattaccgttttctat

SEQ ID NO: 591 - DNA, 69 bp, Artificial Sequence
  Polynucleotide Sequence of aMTD282 5'-primer
gggtttcatatggtgctggcggtggcgccggcgctgattgtggcgccggcaaatattaccgttttctat

SEQ ID NO: 592 - DNA, 69 bp, Artificial Sequence
  Polynucleotide Sequence of aMTD283 5'-primer
gggtttcatatggcggcgctgctggcgccggcgctgattgtggcgccggcaaatattaccgttttctat

SEQ ID NO: 593 - DNA, 69 bp, Artificial Sequence
  Polynucleotide Sequence of aMTD284 5'-primer
gggtttcatatggcgctgattgcgccggcggtggcgctgattgtgccggcaaatattaccgttttctat

SEQ ID NO: 594 - DNA, 69 bp, Artificial Sequence
  Polynucleotide Sequence of aMTD285 5'-primer
gggtttcatatggcgattgtgctgctgccggcggcggtggtggcgccggcaaatattaccgttttctat

SEQ ID NO: 595 - DNA, 69 bp, Artificial Sequence
  Polynucleotide Sequence of aMTD301 5'-primer
gggtttcatatggtgattgcggcgccggtgctggcggtgctggcgccggcaaatattaccgttttctat

SEQ ID NO: 596 - DNA, 69 bp, Artificial Sequence
  Polynucleotide Sequence of aMTD302 5'-primer
gggtttcatatgctggcgctggcgccggcgctggcgctgctggcgccggcaaatattaccgttttctat

SEQ ID NO: 597 - DNA, 69 bp, Artificial Sequence
  Polynucleotide Sequence of aMTD304 5'-primer
gggtttcatatggcgattattctggcgccgattgcggcgattgcgccggcaaatattaccgttttctat

SEQ ID NO: 598 - DNA, 69 bp, Artificial Sequence
  Polynucleotide Sequence of aMTD305 5'-primer
gggtttcatatgattgcgctggcggcgccgattctgctggcggcgccggcaaatattaccgttttctat

SEQ ID NO: 599 - DNA, 69 bp, Artificial Sequence
  Polynucleotide Sequence of aMTD321 5'-primer
gggtttcatatgattgtggcggtggcgctgccggcgctggcggtgccggcaaatattaccgttttctat

SEQ ID NO: 600 - DNA, 69 bp, Artificial Sequence
  Polynucleotide Sequence of aMTD322 5'-primer
gggtttcatatggtggtggcgattgtgctgccggcgctggcggcgccggcaaatattaccgttttctat

SEQ ID NO: 601 - DNA, 69 bp, Artificial Sequence
  Polynucleotide Sequence of aMTD323 5'-primer
gggtttcatatgattgtggcggtggcgctgccggtggcgctggcgccggcaaatattaccgttttctat

SEQ ID NO: 602 - DNA, 69 bp, Artificial Sequence
  Polynucleotide Sequence of aMTD324 5'-primer
gggtttcatatgattgtggcggtggcgctgccggcggcgctggtgccggcaaatattaccgttttctat

SEQ ID NO: 603 - DNA, 69 bp, Artificial Sequence
  Polynucleotide Sequence of aMTD325 5'-primer
gggtttcatatgattgtggcggtggcgctgccggcggtggcgctgccggcaaatattaccgttttctat

SEQ ID NO: 604 - DNA, 69 bp, Artificial Sequence
  Polynucleotide Sequence of aMTD329 5'-primer
gggtttcatatgctgccggtgctggtgccggtggtgccggtggtgccggcaaatattaccgttttctat

SEQ ID NO: 605 - DNA, 69 bp, Artificial Sequence
  Polynucleotide Sequence of aMTD331 5'-primer
gggtttcatatggtgccggtgctggtgccgctggtgccggtggtgccggcaaatattaccgttttctat

SEQ ID NO: 606 - DNA, 69 bp, Artificial Sequence
  Polynucleotide Sequence of aMTD341 5'-primer
gggtttcatatgattgtggcggtggcgctgccggcggtgctggcgccggcaaatattaccgttttctat

SEQ ID NO: 607 - DNA, 69 bp, Artificial Sequence
  Polynucleotide Sequence of aMTD342 5'-primer
gggtttcatatggtgattgtggcgctggcgccggcggtgctggcgccggcaaatattaccgttttctat

SEQ ID NO: 608 - DNA, 69 bp, Artificial Sequence
  Polynucleotide Sequence of aMTD343 5'-primer
gggtttcatatgattgtggcggtggcgctgccggcgctggtggcgccggcaaatattaccgttttctat

SEQ ID NO: 609 - DNA, 69 bp, Artificial Sequence
  Polynucleotide Sequence of aMTD345 5'-primer
gggtttcatatggcgctgctgattgtggcgccggtggcggtggcgccggcaaatattaccgttttctat

SEQ ID NO: 610 - DNA, 69 bp, Artificial Sequence
  Polynucleotide Sequence of aMTD349 5'-primer
gggtttcatatggtgccggtgctggtgccggtggtgccggtggtgccggcaaatattaccgttttctat

SEQ ID NO: 611 - DNA, 69 bp, Artificial Sequence
  Polynucleotide Sequence of aMTD350 5'-primer
gggtttcatatggtgccgattctggtgccggtggtgccggtggtgccggcaaatattaccgttttctat

SEQ ID NO: 612 - DNA, 69 bp, Artificial Sequence
  Polynucleotide Sequence of aMTD361 5'-primer
gggtttcatatggcggtggtgattgtggcgccggcggtgattgcgccggcaaatattaccgttttctat

SEQ ID NO: 613 - DNA, 69 bp, Artificial Sequence
  Polynucleotide Sequence of aMTD363 5'-primer
gggtttcatatggcggtgctggcggtggcgccggcgctgattgtgccggcaaatattaccgttttctat

SEQ ID NO: 614 - DNA, 69 bp, Artificial Sequence
  Polynucleotide Sequence of aMTD364 5'-primer
gggtttcatatgctggtggcggcggtggcgccggcgctgattgtgccggcaaatattaccgttttctat

SEQ ID NO: 615 - DNA, 69 bp, Artificial Sequence
  Polynucleotide Sequence of aMTD365 5'-primer
gggtttcatatggcggtgattgtggtggcgccggcgctgctggcgccggcaaatattaccgttttctat

SEQ ID NO: 616 - DNA, 69 bp, Artificial Sequence
  Polynucleotide Sequence of aMTD381 5'-primer
gggtttcatatggtggtggcgattgtgctgccggcggtggcggcgccggcaaatattaccgttttctat

SEQ ID NO: 617 - DNA, 69 bp, Artificial Sequence
  Polynucleotide Sequence of aMTD382 5'-primer
gggtttcatatggcggcggcgctggtgattccggcgattctggcgccggcaaatattaccgttttctat

SEQ ID NO: 618 - DNA, 69 bp, Artificial Sequence
  Polynucleotide Sequence of aMTD383 5'-primer
gggtttcatatggtgattgtggcgctggcgccggcgctgctggcgccggcaaatattaccgttttctat

SEQ ID NO: 619 - DNA, 69 bp, Artificial Sequence
  Polynucleotide Sequence of aMTD384 5'-primer
gggtttcatatggtgattgtggcgattgcgccggcgctgctggcgccggcaaatattaccgttttctat

SEQ ID NO: 620 - DNA, 69 bp, Artificial Sequence
  Polynucleotide Sequence of aMTD385 5'-primer
gggtttcatatgattgtggcgattgcggtgccggcgctggtggcgccggcaaatattaccgttttctat

SEQ ID NO: 621 - DNA, 69 bp, Artificial Sequence
  Polynucleotide Sequence of aMTD390 5'-primer
gggtttcatatggtgccgctgctggtgccggtggtgccggtggtgccggcaaatattaccgttttctat

SEQ ID NO: 622 - DNA, 69 bp, Artificial Sequence
  Polynucleotide Sequence of aMTD401 5'-primer
gggtttcatatggcggcgctggcggtgattccggcggcgattctgccggcaaatattaccgttttctat

SEQ ID NO: 623 - DNA, 69 bp, Artificial Sequence
  Polynucleotide Sequence of aMTD402 5'-primer
gggtttcatatggcgctggcggcggtgattccggcggcgattctgccggcaaatattaccgttttctat

SEQ ID NO: 624 - DNA, 69 bp, Artificial Sequence
  Polynucleotide Sequence of aMTD403 5'-primer
gggtttcatatggcggcggcgctggtgattccggcggcgattctgccggcaaatattaccgttttctat

SEQ ID NO: 625 - DNA, 69 bp, Artificial Sequence
  Polynucleotide Sequence of aMTD404 5'-primer
gggtttcatatgctggcggcggcggtgattccggcggcgattctgccggcaaatattaccgttttctat

SEQ ID NO: 626 - DNA, 69 bp, Artificial Sequence
  Polynucleotide Sequence of aMTD405 5'-primer
gggtttcatatgctggcggcggcggtgattccggtggcgattctgccggcaaatattaccgttttctat

SEQ ID NO: 627 - DNA, 69 bp, Artificial Sequence
  Polynucleotide Sequence of aMTD421 5'-primer
gggtttcatatggcggcgattctggcggcgccgctgattgcggtgccggcaaatattaccgttttctat

SEQ ID NO: 628 - DNA, 69 bp, Artificial Sequence
  Polynucleotide Sequence of aMTD422 5'-primer
gggtttcatatggtggtggcgattctggcgccgctgctggcggcgccggcaaatattaccgttttctat

SEQ ID NO: 629 - DNA, 69 bp, Artificial Sequence
  Polynucleotide Sequence of aMTD424 5'-primer
gggtttcatatggcggtggtggtggcggcgccggtgctggcgctgccggcaaatattaccgttttctat

SEQ ID NO: 630 - DNA, 69 bp, Artificial Sequence
  Polynucleotide Sequence of aMTD425 5'-primer
gggtttcatatggcggtggtggcgattgcgccggtgctggcgctgccggcaaatattaccgttttctat

SEQ ID NO: 631 - DNA, 69 bp, Artificial Sequence
  Polynucleotide Sequence of aMTD426 5'-primer
gggtttcatatggcggcggcgctggcgattccgctggcgattattccggcaaatattaccgttttctat

SEQ ID NO: 632 - DNA, 69 bp, Artificial Sequence
  Polynucleotide Sequence of aMTD436 5'-primer
gggtttcatatggcggtggtgctggtgattatgccggcggcgattccggcaaatattaccgttttctat

SEQ ID NO: 633 - DNA, 69 bp, Artificial Sequence
  Polynucleotide Sequence of aMTD442 5'-primer
gggtttcatatggcgctggcggcgctggtgccggcggtgctggtgccggcaaatattaccgttttctat

SEQ ID NO: 634 - DNA, 69 bp, Artificial Sequence
  Polynucleotide Sequence of aMTD443 5'-primer
gggtttcatatggcgctggcggcgctggtgccggtggcgctggtgccggcaaatattaccgttttctat

SEQ ID NO: 635 - DNA, 69 bp, Artificial Sequence
  Polynucleotide Sequence of aMTD444 5'-primer
gggtttcatatgctggcggcggcgctggtgccggtggcgctggtgccggcaaatattaccgttttctat

SEQ ID NO: 636 - DNA, 69 bp, Artificial Sequence
  Polynucleotide Sequence of aMTD445 5'-primer
gggtttcatatggcgctggcggcgctggtgccggcgctggtggtgccggcaaatattaccgttttctat

SEQ ID NO: 637 - DNA, 69 bp, Artificial Sequence
  Polynucleotide Sequence of aMTD461 5'-primer
gggtttcatatgattgcggcggtgattgtgccggcggtggcgctgccggcaaatattaccgttttctat

SEQ ID NO: 638 - DNA, 69 bp, Artificial Sequence
  Polynucleotide Sequence of aMTD462 5'-primer
gggtttcatatgattgcggcggtgctggtgccggcggtggcgctgccggcaaatattaccgttttctat

SEQ ID NO: 639 - DNA, 69 bp, Artificial Sequence
  Polynucleotide Sequence of aMTD463 5'-primer
gggtttcatatggcggtggcgattctggtgccgctgctggcggcgccggcaaatattaccgttttctat

SEQ ID NO: 640 - DNA, 69 bp, Artificial Sequence
  Polynucleotide Sequence of aMTD464 5'-primer
gggtttcatatggcggtggtgattctggtgccgctggcggcggcgccggcaaatattaccgttttctat

SEQ ID NO: 641 - DNA, 69 bp, Artificial Sequence
  Polynucleotide Sequence of aMTD465 5'-primer
gggtttcatatgattgcggcggtgattgtgccggtggcggcgctgccggcaaatattaccgttttctat

SEQ ID NO: 642 - DNA, 69 bp, Artificial Sequence
  Polynucleotide Sequence of aMTD466 5'-primer
gggtttcatatgattattgcggcggcggcgccgctggcgattattccggcaaatattaccgttttctat

SEQ ID NO: 643 - DNA, 69 bp, Artificial Sequence
  Polynucleotide Sequence of aMTD481 5'-primer
gggtttcatatggcgattgcgattgcgattgtgccggtggcgctgccggcaaatattaccgttttctat

SEQ ID NO: 644 - DNA, 69 bp, Artificial Sequence
  Polynucleotide Sequence of aMTD482 5'-primer
gggtttcatatgattctggcggtggcggcgattccggtggcggtgccggcaaatattaccgttttctat

SEQ ID NO: 645 - DNA, 69 bp, Artificial Sequence
  Polynucleotide Sequence of aMTD483 5'-primer
gggtttcatatgattctggcggcggcgattattccggcggcgctgccggcaaatattaccgttttctat

SEQ ID NO: 646 - DNA, 69 bp, Artificial Sequence
  Polynucleotide Sequence of aMTD484 5'-primer
gggtttcatatgctggcggtggtgctggcggcgccggcgattgtgccggcaaatattaccgttttctat

SEQ ID NO: 647 - DNA, 69 bp, Artificial Sequence
  Polynucleotide Sequence of aMTD485 5'-primer
gggtttcatatggcgattctggcggcgattgtgccgctggcggtgccggcaaatattaccgttttctat

SEQ ID NO: 648 - DNA, 69 bp, Artificial Sequence
  Polynucleotide Sequence of aMTD501 5'-primer
gggtttcatatggtgattgtggcgctggcggtgccggcgctggcgccggcaaatattaccgttttctat

SEQ ID NO: 649 - DNA, 69 bp, Artificial Sequence
  Polynucleotide Sequence of aMTD502 5'-primer
gggtttcatatggcgattgtggcgctggcggtgccggtgctggcgccggcaaatattaccgttttctat

SEQ ID NO: 650 - DNA, 69 bp, Artificial Sequence
  Polynucleotide Sequence of aMTD503 5'-primer
gggtttcatatggcggcgattattattgtgctgccggcggcgctgccggcaaatattaccgttttctat

SEQ ID NO: 651 - DNA, 69 bp, Artificial Sequence
  Polynucleotide Sequence of aMTD504 5'-primer
gggtttcatatgctgattgtggcgctggcggtgccggcgctggcgccggcaaatattaccgttttctat

SEQ ID NO: 652 - DNA, 69 bp, Artificial Sequence
  Polynucleotide Sequence of aMTD505 5'-primer
gggtttcatatggcgattattattgtgattgcgccggcggcggcgccggcaaatattaccgttttctat

SEQ ID NO: 653 - DNA, 69 bp, Artificial Sequence
  Polynucleotide Sequence of aMTD521 5'-primer
gggtttcatatgctggcggcgctgattgtggtgccggcggtggcgccggcaaatattaccgttttctat

SEQ ID NO: 654 - DNA, 69 bp, Artificial Sequence
  Polynucleotide Sequence of aMTD522 5'-primer
gggtttcatatggcgctgctggtgattgcggtgccggcggtggcgccggcaaatattaccgttttctat

SEQ ID NO: 655 - DNA, 69 bp, Artificial Sequence
  Polynucleotide Sequence of aMTD524 5'-primer
gggtttcatatggcggtggcgctgattgtggtgccggcgctggcgccggcaaatattaccgttttctat

SEQ ID NO: 656 - DNA, 69 bp, Artificial Sequence
  Polynucleotide Sequence of aMTD525 5'-primer
gggtttcatatggcgctggcgattgtggtggcgccggtggcggtgccggcaaatattaccgttttctat

SEQ ID NO: 657 - DNA, 69 bp, Artificial Sequence
  Polynucleotide Sequence of aMTD527 5'-primer
gggtttcatatgctggtgctggcggcggtggcgccgattgcgattccggcaaatattaccgttttctat

SEQ ID NO: 658 - DNA, 69 bp, Artificial Sequence
  Polynucleotide Sequence of aMTD541 5'-primer
gggtttcatatgctgctggcgctgattattgcgccggcggcggcgccggcaaatattaccgttttctat

SEQ ID NO: 659 - DNA, 69 bp, Artificial Sequence
  Polynucleotide Sequence of aMTD542 5'-primer
gggtttcatatggcgctggcgctgattattgtgccggcggtggcgccggcaaatattaccgttttctat

SEQ ID NO: 660 - DNA, 69 bp, Artificial Sequence
  Polynucleotide Sequence of aMTD543 5'-primer
gggtttcatatgctgctggcggcgctgattgcgccggcggcgctgccggcaaatattaccgttttctat

SEQ ID NO: 661 - DNA, 69 bp, Artificial Sequence
  Polynucleotide Sequence of aMTD544 5'-primer
gggtttcatatgattgtggcgctgattgtggcgccggcggcggtgccggcaaatattaccgttttctat

SEQ ID NO: 662 - DNA, 69 bp, Artificial Sequence
  Polynucleotide Sequence of aMTD545 5'-primer
gggtttcatatggtggtgctggtgctggcggcgccggcggcggtgccggcaaatattaccgttttctat

SEQ ID NO: 663 - DNA, 69 bp, Artificial Sequence
  Polynucleotide Sequence of aMTD561 5'-primer
gggtttcatatggcggcggtggcgattgtgctgccggcggtggtgccggcaaatattaccgttttctat

SEQ ID NO: 664 - DNA, 69 bp, Artificial Sequence
  Polynucleotide Sequence of aMTD562 5'-primer
gggtttcatatggcgctgattgcggcgattgtgccggcgctggtgccggcaaatattaccgttttctat

SEQ ID NO: 665 - DNA, 69 bp, Artificial Sequence
  Polynucleotide Sequence of aMTD563 5'-primer
gggtttcatatggcgctggcggtgattgtggtgccggcgctggcgccggcaaatattaccgttttctat

SEQ ID NO: 666 - DNA, 69 bp, Artificial Sequence
  Polynucleotide Sequence of aMTD564 5'-primer
gggtttcatatggtggcgattgcgctgattgtgccggcgctggcgccggcaaatattaccgttttctat

SEQ ID NO: 667 - DNA, 69 bp, Artificial Sequence
  Polynucleotide Sequence of aMTD565 5'-primer
gggtttcatatggtggcgattgtgctggtggcgccggcggtggcgccggcaaatattaccgttttctat

SEQ ID NO: 668 - DNA, 69 bp, Artificial Sequence
  Polynucleotide Sequence of aMTD577 5'-primer
gggtttcatatggcggcggtgctgattgtgccgattatggtgatgccggcaaatattaccgttttctat

SEQ ID NO: 669 - DNA, 69 bp, Artificial Sequence
  Polynucleotide Sequence of aMTD582 5'-primer
gggtttcatatggtggcggtggcgctgattgtgccggcgctggcgccggcaaatattaccgttttctat

SEQ ID NO: 670 - DNA, 69 bp, Artificial Sequence
  Polynucleotide Sequence of aMTD583 5'-primer
gggtttcatatggcggtgattctggcgctggcgccgattgtggcgccggcaaatattaccgttttctat

SEQ ID NO: 671 - DNA, 69 bp, Artificial Sequence
  Polynucleotide Sequence of aMTD585 5'-primer
gggtttcatatggcgctgattgtggcgattgcgccggcgctggtgccggcaaatattaccgttttctat

SEQ ID NO: 672 - DNA, 69 bp, Artificial Sequence
  Polynucleotide Sequence of aMTD601 5'-primer
gggtttcatatggcggcgattctgattgcggtgccgattgcggcgccggcaaatattaccgttttctat

SEQ ID NO: 673 - DNA, 69 bp, Artificial Sequence
  Polynucleotide Sequence of aMTD602 5'-primer
gggtttcatatggtgattgtggcgctggcggcgccggtgctggcgccggcaaatattaccgttttctat

SEQ ID NO: 674 - DNA, 69 bp, Artificial Sequence
  Polynucleotide Sequence of aMTD603 5'-primer
gggtttcatatggtgctggtggcgctggcggcgccggtgattgcgccggcaaatattaccgttttctat

SEQ ID NO: 675 - DNA, 69 bp, Artificial Sequence
  Polynucleotide Sequence of aMTD604 5'-primer
gggtttcatatggtggcgctgattgcggtggcgccggcggtggtgccggcaaatattaccgttttctat

SEQ ID NO: 676 - DNA, 69 bp, Artificial Sequence
  Polynucleotide Sequence of aMTD605 5'-primer
gggtttcatatggtgattgcggcggtgctggcgccggtggcggtgccggcaaatattaccgttttctat

SEQ ID NO: 677 - DNA, 69 bp, Artificial Sequence
  Polynucleotide Sequence of aMTD606 5'-primer
gggtttcatatggcggcggcgattgcggcgattccgattattattccggcaaatattaccgttttctat

SEQ ID NO: 678 - DNA, 69 bp, Artificial Sequence; identical to SEQ ID NO: 677
  Polynucleotide Sequence of aMTD622 5'-primer

SEQ ID NO: 679 - DNA, 69 bp, Artificial Sequence
  Polynucleotide Sequence of aMTD623 5'-primer
gggtttcatatggtggcggcggcgattgcgctgccggcgattgtgccggcaaatattaccgttttctat

SEQ ID NO: 680 - DNA, 69 bp, Artificial Sequence
  Polynucleotide Sequence of aMTD625 5'-primer
gggtttcatatgattctggcggcggcggcggcgccgctgattgtgccggcaaatattaccgttttctat

SEQ ID NO: 681 - DNA, 69 bp, Artificial Sequence
  Polynucleotide Sequence of aMTD635 5'-primer
gggtttcatatgggcagcaccggcggcagccagcagaacaaccagtatgcaaatattaccgttttctat

SEQ ID NO: 682 - DNA, 69 bp, Artificial Sequence
  Polynucleotide Sequence of aMTD643 5'-primer
gggtttcatatgctggcgctggtgctggcggcgccggcgattgtgccggcaaatattaccgttttctat

SEQ ID NO: 683 - DNA, 69 bp, Artificial Sequence
  Polynucleotide Sequence of aMTD645 5'-primer
gggtttcatatggcgctggcggtggtggcgctgccggcgattgtgccggcaaatattaccgttttctat

SEQ ID NO: 684 - DNA, 69 bp, Artificial Sequence
  Polynucleotide Sequence of aMTD661 5'-primer
gggtttcatatggcggcgattctggcgccgattgtggcggcgctgccggcaaatattaccgttttctat

SEQ ID NO: 685 - DNA, 69 bp, Artificial Sequence
  Polynucleotide Sequence of aMTD664 5'-primer
gggtttcatatgattctgattgcgattgcgattccggcggcggcgccggcaaatattaccgttttctat

SEQ ID NO: 686 - DNA, 69 bp, Artificial Sequence
  Polynucleotide Sequence of aMTD665 5'-primer
gggtttcatatgctggcgattgtgctggcggcgccggtggcggtgccggcaaatattaccgttttctat

SEQ ID NO: 687 - DNA, 69 bp, Artificial Sequence
  Polynucleotide Sequence of aMTD666 5'-primer
gggtttcatatggcggcgattgcgattattgcgccggcgattgtgccggcaaatattaccgttttctat

SEQ ID NO: 688 - DNA, 69 bp, Artificial Sequence
  Polynucleotide Sequence of aMTD667 5'-primer
gggtttcatatgctggcggtggcgattgtggcgccggcgctggtgccggcaaatattaccgttttctat

SEQ ID NO: 689 - DNA, 69 bp, Artificial Sequence
  Polynucleotide Sequence of aMTD676 5'-primer
gggtttcatatggtgccgctgctggtgccggtgccggtggtggtgccggcaaatattaccgttttctat

SEQ ID NO: 690 - DNA, 69 bp, Artificial Sequence
  Polynucleotide Sequence of aMTD683 5'-primer
gggtttcatatgctggcgattgtgctggcggcgccggcggtgctgccggcaaatattaccgttttctat

SEQ ID NO: 691 - DNA, 69 bp, Artificial Sequence
  Polynucleotide Sequence of aMTD684 5'-primer
gggtttcatatggcggcgattgtgctggcgctgccggcggtgctgccggcaaatattaccgttttctat

SEQ ID NO: 692 - DNA, 69 bp, Artificial Sequence
  Polynucleotide Sequence of aMTD685 5'-primer
gggtttcatatggcgctgctggtggcggtgctgccggcggcgctgccggcaaatattaccgttttctat

SEQ ID NO: 693 - DNA, 69 bp, Artificial Sequence
  Polynucleotide Sequence of aMTD686 5'-primer
gggtttcatatggcggcgctggtggcggtgctgccggtggcgctgccggcaaatattaccgttttctat

SEQ ID NO: 694 - DNA, 69 bp, Artificial Sequence
  Polynucleotide Sequence of aMTD687 5'-primer
gggtttcatatggcgattctggcggtggcgctgccgctgctggcgccggcaaatattaccgttttctat

SEQ ID NO: 695 - DNA, 69 bp, Artificial Sequence
  Polynucleotide Sequence of aMTD692 5'-primer
gggtttcatatgccggcgccgctgccgccggtggtgattctggcggtggcaaatattaccgttttctat

SEQ ID NO: 696 - DNA, 69 bp, Artificial Sequence
  Polynucleotide Sequence of aMTD693 5'-primer
gggtttcatatggcggcgccggtgctgccggtggcggtgccgattgtggcaaatattaccgttttctat

SEQ ID NO: 697 - DNA, 69 bp, Artificial Sequence
  Polynucleotide Sequence of aMTD700 5'-primer
gggtttcatatgggcaccagcaacacctgccagagcaaccagaacagcgcaaatattaccgttttctat

SEQ ID NO: 698 - DNA, 69 bp, Artificial Sequence
  Polynucleotide Sequence of aMTD703 5'-primer
gggtttcatatgattgtggcggtggcgctggtgccggcgctggcgccggcaaatattaccgttttctat

SEQ ID NO: 699 - DNA, 68 bp, Artificial Sequence
  Polynucleotide Sequence of aMTD705 5'-primer
gggtttcatatattgtggcggtggcgctgctgccggcgctggcgccggcaaatattaccgttttctat

SEQ ID NO: 700 - DNA, 69 bp, Artificial Sequence
  Polynucleotide Sequence of aMTD706 5'-primer
gggtttcatatgattgtggcggtggcgctgctgccggcggtggcgccggcaaatattaccgttttctat

SEQ ID NO: 701 - DNA, 69 bp, Artificial Sequence
  Polynucleotide Sequence of aMTD707 5'-primer
gggtttcatatgattgtggcgctggcggtgctgccggcggtggcgccggcaaatattaccgttttctat

SEQ ID NO: 702 - DNA, 69 bp, Artificial Sequence
  Polynucleotide Sequence of aMTD724 5'-primer
gggtttcatatggtggcggtgctggcggtgctgccggcgctggcgccggcaaatattaccgttttctat

SEQ ID NO: 703 - DNA, 69 bp, Artificial Sequence
  Polynucleotide Sequence of aMTD725 5'-primer
gggtttcatatgattgcggtgctggcggtggcgccggcggtgctgccggcaaatattaccgttttctat

SEQ ID NO: 704 - DNA, 69 bp, Artificial Sequence
  Polynucleotide Sequence of aMTD726 5'-primer
gggtttcatatgctggcggtggcgattattgcgccggcggtggcgccggcaaatattaccgttttctat

SEQ ID NO: 705 - DNA, 69 bp, Artificial Sequence
  Polynucleotide Sequence of aMTD727 5'-primer
gggtttcatatggtggcgctggcgattgcgctgccggcggtgctgccggcaaatattaccgttttctat

SEQ ID NO: 706 - DNA, 69 bp, Artificial Sequence
  Polynucleotide Sequence of aMTD743 5'-primer
gggtttcatatggcgattgcgattgcgctggtgccggtggcgctgccggcaaatattaccgttttctat

SEQ ID NO: 707 - DNA, 69 bp, Artificial Sequence
  Polynucleotide Sequence of aMTD744 5'-primer
gggtttcatatggcggcggtggtgattgtggcgccggtggcgctgccggcaaatattaccgttttctat

SEQ ID NO: 708 - DNA, 69 bp, Artificial Sequence
  Polynucleotide Sequence of aMTD745 5'-primer
gggtttcatatggcggcgattctggcgattgtggcgccgctggcgccggcaaatattaccgttttctat

SEQ ID NO: 709 - DNA, 69 bp, Artificial Sequence
  Polynucleotide Sequence of aMTD746 5'-primer
gggtttcatatggtggcgattattgtggtggcgccggcgctggcgccggcaaatattaccgttttctat

SEQ ID NO: 710 - DNA, 69 bp, Artificial Sequence
  Polynucleotide Sequence of aMTD747 5'-primer
gggtttcatatggtggcgctgctggcgattgcgccggcgctggcgccggcaaatattaccgttttctat

SEQ ID NO: 711 - DNA, 69 bp, Artificial Sequence
  Polynucleotide Sequence of aMTD750 5'-primer
gggtttcatatgctggcgattgcggcgattgcgccgctggcgattccggcaaatattaccgttttctat

SEQ ID NO: 712 - DNA, 69 bp, Artificial Sequence
  Polynucleotide Sequence of aMTD763 5'-primer
gggtttcatatggtggcggtgctgattgcggtgccggcgctggcgccggcaaatattaccgttttctat

SEQ ID NO: 713 - DNA, 69 bp, Artificial Sequence
  Polynucleotide Sequence of aMTD764 5'-primer
gggtttcatatggcggtggcgctggcggtgctgccggcggtggtgccggcaaatattaccgttttctat

SEQ ID NO: 714 - DNA, 69 bp, Artificial Sequence
  Polynucleotide Sequence of aMTD765 5'-primer
gggtttcatatggcggtggcgctggcggtggtgccggcggtgctgccggcaaatattaccgttttctat

SEQ ID NO: 715 - DNA, 69 bp, Artificial Sequence
  Polynucleotide Sequence of aMTD766 5'-primer
gggtttcatatgattgtggtgattgcggtggcgccggcggtggcgccggcaaatattaccgttttctat

SEQ ID NO: 716 - DNA, 69 bp, Artificial Sequence
  Polynucleotide Sequence of aMTD767 5'-primer
gggtttcatatgattgtggtggcggcggtggtgccggcgctggcgccggcaaatattaccgttttctat

SEQ ID NO: 717 - DNA, 69 bp, Artificial Sequence
  Polynucleotide Sequence of aMTD772 5'-primer
gggtttcatatgctgccggtggcgccggtgattccgattattgtgccggcaaatattaccgttttctat

SEQ ID NO: 718 - DNA, 69 bp, Artificial Sequence
  Polynucleotide Sequence of aMTD783 5'-primer
gggtttcatatgattgtggcgctggtgccggcggtggcgattgcgccggcaaatattaccgttttctat

SEQ ID NO: 719 - DNA, 69 bp, Artificial Sequence
  Polynucleotide Sequence of aMTD784 5'-primer
gggtttcatatggtggcggcgctgccggcggtggcgctggtggtgccggcaaatattaccgttttctat

SEQ ID NO: 720 - DNA, 69 bp, Artificial Sequence
  Polynucleotide Sequence of aMTD786 5'-primer
gggtttcatatgctggtggcgattgcgccgctggcggtgctggcgccggcaaatattaccgttttctat

SEQ ID NO: 721 - DNA, 69 bp, Artificial Sequence
  Polynucleotide Sequence of aMTD787 5'-primer
gggtttcatatggcggtggcgctggtgccggtgattgtggcggcgccggcaaatattaccgttttctat

SEQ ID NO: 722 - DNA, 69 bp, Artificial Sequence
  Polynucleotide Sequence of aMTD788 5'-primer
gggtttcatatggcgattgcggtggcgattgcgccggtggcgctgccggcaaatattaccgttttctat

SEQ ID NO: 723 - DNA, 69 bp, Artificial Sequence
  Polynucleotide Sequence of aMTD803 5'-primer
gggtttcatatggcgattgcgctggcggtgccggtgctggcgctgccggcaaatattaccgttttctat

SEQ ID NO: 724 - DNA, 69 bp, Artificial Sequence
  Polynucleotide Sequence of aMTD805 5'-primer
gggtttcatatgctggtgctgattgcggcggcgccgattgcgctgccggcaaatattaccgttttctat

SEQ ID NO: 725 - DNA, 69 bp, Artificial Sequence
  Polynucleotide Sequence of aMTD806 5'-primer
gggtttcatatgctggtggcgctggcggtgccggcggcggtgctgccggcaaatattaccgttttctat

SEQ ID NO: 726 - DNA, 69 bp, Artificial Sequence
  Polynucleotide Sequence of aMTD807 5'-primer
gggtttcatatggcggtggcgctggcggtgccggcgctggtgctgccggcaaatattaccgttttctat

SEQ ID NO: 727 - DNA, 69 bp, Artificial Sequence
  Polynucleotide Sequence of aMTD808 5'-primer
gggtttcatatgctggtggtgctggcggcggcgccgctggcggtgccggcaaatattaccgttttctat

SEQ ID NO: 728 - DNA, 69 bp, Artificial Sequence
  Polynucleotide Sequence of aMTD809 5'-primer
gggtttcatatgctgattgtgctggcggcgccggcgctggcggcgccggcaaatattaccgttttctat

SEQ ID NO: 729 - DNA, 69 bp, Artificial Sequence
  Polynucleotide Sequence of aMTD810 5'-primer
gggtttcatatggtgattgtgctggcggcgccggcgctggcggcgccggcaaatattaccgttttctat

SEQ ID NO: 730 - DNA, 69 bp, Artificial Sequence
  Polynucleotide Sequence of aMTD811 5'-primer
gggtttcatatggcggtggtgctggcggtgccggcgctggcggtgccggcaaatattaccgttttctat

SEQ ID NO: 731 - DNA, 69 bp, Artificial Sequence
  Polynucleotide Sequence of aMTD824 5'-primer
gggtttcatatgctgattattgtggcggcggcgccggcggtggcgccggcaaatattaccgttttctat

SEQ ID NO: 732 - DNA, 69 bp, Artificial Sequence
  Polynucleotide Sequence of aMTD825 5'-primer
gggtttcatatgattgtggcggtgattgtggcgccggcggtggcgccggcaaatattaccgttttctat

SEQ ID NO: 733 - DNA, 69 bp, Artificial Sequence
  Polynucleotide Sequence of aMTD826 5'-primer
gggtttcatatgctggtggcgctggcggcgccgattattgcggtgccggcaaatattaccgttttctat

SEQ ID NO: 734 - DNA, 69 bp, Artificial Sequence
  Polynucleotide Sequence of aMTD827 5'-primer
gggtttcatatgattgcggcggtgctggcggcgccggcgctggtgccggcaaatattaccgttttctat

SEQ ID NO: 735 - DNA, 69 bp, Artificial Sequence
  Polynucleotide Sequence of aMTD828 5'-primer
gggtttcatatgattgcgctgctggcggcgccgattattgcggtgccggcaaatattaccgttttctat

SEQ ID NO: 736 - DNA, 69 bp, Artificial Sequence
  Polynucleotide Sequence of aMTD829 5'-primer
gggtttcatatggcggcgctggcgctggtggcgccggtgattgtgccggcaaatattaccgttttctat

SEQ ID NO: 737 - DNA, 69 bp, Artificial Sequence
  Polynucleotide Sequence of aMTD830 5'-primer
gggtttcatatgattgcgctggtggcggcgccggtggcgctggtgccggcaaatattaccgttttctat

SEQ ID NO: 738 - DNA, 69 bp, Artificial Sequence
  Polynucleotide Sequence of aMTD831 5'-primer
gggtttcatatgattattgtggcggtggcgccggcggcgattgtgccggcaaatattaccgttttctat

SEQ ID NO: 739 - DNA, 69 bp, Artificial Sequence
  Polynucleotide Sequence of aMTD832 5'-primer
gggtttcatatggcggtggcggcgattgtgccggtgattgtggcgccggcaaatattaccgttttctat

SEQ ID NO: 740 - DNA, 69 bp, Artificial Sequence
  Polynucleotide Sequence of aMTD843 5'-primer
gggtttcatatggcggtgctggtgctggtggcgccggcggcggcgccggcaaatattaccgttttctat

SEQ ID NO: 741 - DNA, 69 bp, Artificial Sequence
  Polynucleotide Sequence of aMTD844 5'-primer
gggtttcatatggtggtggcgctgctggcgccgctgattgcggcgccggcaaatattaccgttttctat

SEQ ID NO: 742 - DNA, 69 bp, Artificial Sequence
  Polynucleotide Sequence of aMTD845 5'-primer
gggtttcatatggcggcggtggtgattgcgccgctgctggcggtgccggcaaatattaccgttttctat

SEQ ID NO: 743 - DNA, 69 bp, Artificial Sequence
  Polynucleotide Sequence of aMTD846 5'-primer
gggtttcatatgattgcggtggcggtggcggcgccgctgctggtgccggcaaatattaccgttttctat

SEQ ID NO: 744 - DNA, 69 bp, Artificial Sequence
  Polynucleotide Sequence of aMTD847 5'-primer
gggtttcatatgctggtggcgattgtggtgctgccggcggtggcgccggcaaatattaccgttttctat

SEQ ID NO: 745 - DNA, 69 bp, Artificial Sequence
  Polynucleotide Sequence of aMTD848 5'-primer
gggtttcatatggcggtggcgattgtggtgctgccggcggtggcgccggcaaatattaccgttttctat

SEQ ID NO: 746 - DNA, 69 bp, Artificial Sequence
  Polynucleotide Sequence of aMTD849 5'-primer
gggtttcatatggcggtgattctgctggcgccgctgattgcggcgccggcaaatattaccgttttctat

SEQ ID NO: 747 - DNA, 69 bp, Artificial Sequence
  Polynucleotide Sequence of aMTD850 5'-primer
gggtttcatatgctggtgattgcgctggcggcgccggtggcgctgccggcaaatattaccgttttctat

SEQ ID NO: 748 - DNA, 69 bp, Artificial Sequence
  Polynucleotide Sequence of aMTD851 5'-primer
gggtttcatatggtgctggcggtggtgctgccggcggtggcgctgccggcaaatattaccgttttctat

SEQ ID NO: 749 - DNA, 69 bp, Artificial Sequence
  Polynucleotide Sequence of aMTD852 5'-primer
gggtttcatatggtgctggcggtggcggcgccggcggtgctgctgccggcaaatattaccgttttctat

SEQ ID NO: 750 - DNA, 69 bp, Artificial Sequence
  Polynucleotide Sequence of aMTD863 5'-primer
gggtttcatatggcggcggtggtgctgctgccgattattgcggcgccggcaaatattaccgttttctat

SEQ ID NO: 751 - DNA, 69 bp, Artificial Sequence
  Polynucleotide Sequence of aMTD864 5'-primer
gggtttcatatggcgctgctggtgattgcgccggcgattgcggtgccggcaaatattaccgttttctat

SEQ ID NO: 752 - DNA, 69 bp, Artificial Sequence
  Polynucleotide Sequence of aMTD865 5'-primer
gggtttcatatggcggtgctggtgattgcggtgccggcgattgcgccggcaaatattaccgttttctat

SEQ ID NO: 753 - DNA, 69 bp, Artificial Sequence
  Polynucleotide Sequence of aMTD867 5'-primer
gggtttcatatggcgctgctggtggtgattgcgccgctggcggcgccggcaaatattaccgttttctat

SEQ ID NO: 754 - DNA, 69 bp, Artificial Sequence
  Polynucleotide Sequence of aMTD868 5'-primer
gggtttcatatggtgctggtggcggcgattctgccggcggcgattccggcaaatattaccgttttctat

SEQ ID NO: 755 - DNA, 69 bp, Artificial Sequence
  Polynucleotide Sequence of aMTD870 5'-primer
gggtttcatatggtgctggtggcggcggtgctgccgattgcggcgccggcaaatattaccgttttctat

SEQ ID NO: 756 - DNA, 69 bp, Artificial Sequence
  Polynucleotide Sequence of aMTD872 5'-primer
gggtttcatatggtgctggcggcggcggtgctgccgctggtggtgccggcaaatattaccgttttctat

SEQ ID NO: 757 - DNA, 69 bp, Artificial Sequence
  Polynucleotide Sequence of aMTD875 5'-primer
gggtttcatatggcgattgcgattgtggtgccggcggtggcggtgccggcaaatattaccgttttctat

SEQ ID NO: 758 - DNA, 69 bp, Artificial Sequence
  Polynucleotide Sequence of aMTD877 5'-primer
gggtttcatatggtggcgattattgcggtgccggcggtggtggcgccggcaaatattaccgttttctat

SEQ ID NO: 759 - DNA, 69 bp, Artificial Sequence
  Polynucleotide Sequence of aMTD878 5'-primer
gggtttcatatgattgtggcgctggtggcgccggcggcggtggtgccggcaaatattaccgttttctat

SEQ ID NO: 760 - DNA, 69 bp, Artificial Sequence
  Polynucleotide Sequence of aMTD879 5'-primer
gggtttcatatggcggcgattgtgctgctgccggcggtggtggtgccggcaaatattaccgttttctat

SEQ ID NO: 761 - DNA, 69 bp, Artificial Sequence
  Polynucleotide Sequence of aMTD881 5'-primer
gggtttcatatggcggcgctgattgtggtgccggcggtggcggtgccggcaaatattaccgttttctat

SEQ ID NO: 762 - DNA, 69 bp, Artificial Sequence
  Polynucleotide Sequence of aMTD882 5'-primer
gggtttcatatggcgattgcgctggtggtgccggcggtggcggtgccggcaaatattaccgttttctat

SEQ ID NO: 763 - DNA, 69 bp, Artificial Sequence
  Polynucleotide Sequence of aMTD883 5'-primer
gggtttcatatgctggcgattgtgccggcggcgattgcggcgctgccggcaaatattaccgttttctat

SEQ ID NO: 764 - DNA, 69 bp, Artificial Sequence
  Polynucleotide Sequence of aMTD884 5'-primer
gggtttcatatggtgctgattgtgccggcggcgattgcggcgctgccggcaaatattaccgttttctat

SEQ ID NO: 765 - DNA, 69 bp, Artificial Sequence
  Polynucleotide Sequence of aMTD885 5'-primer
gggtttcatatgctggtggcgattgcgccggcggtggcggtgctgccggcaaatattaccgttttctat

SEQ ID NO: 766 - DNA, 69 bp, Artificial Sequence
  Polynucleotide Sequence of aMTD886 5'-primer
gggtttcatatggtgctggcggtgccggcggcgattgcggcgctgccggcaaatattaccgttttctat

SEQ ID NO: 767 - DNA, 69 bp, Artificial Sequence
  Polynucleotide Sequence of aMTD887 5'-primer
gggtttcatatggtgctggcggtggcgccggcggtggcggtgctgccggcaaatattaccgttttctat

SEQ ID NO: 768 - DNA, 69 bp, Artificial Sequence
  Polynucleotide Sequence of aMTD888 5'-primer
gggtttcatatgattctggcggtggtggcgattccggcggcggcgccggcaaatattaccgttttctat

SEQ ID NO: 769 - DNA, 69 bp, Artificial Sequence
  Polynucleotide Sequence of aMTD889 5'-primer
gggtttcatatgattctggtggcggcggcgccgattgcggcgctgccggcaaatattaccgttttctat

SEQ ID NO: 770 - DNA, 69 bp, Artificial Sequence
  Polynucleotide Sequence of aMTD891 5'-primer
gggtttcatatgattctggcggtggcggcgattccggcggcgctgccggcaaatattaccgttttctat

SEQ ID NO: 771 - DNA, 69 bp, Artificial Sequence
  Polynucleotide Sequence of aMTD893 5'-primer
gggtttcatatggtgattgcgattccggcgattctggcggcggcgccggcaaatattaccgttttctat

SEQ ID NO: 772 - DNA, 69 bp, Artificial Sequence
  Polynucleotide Sequence of aMTD895 5'-primer
gggtttcatatggcgattattattgtggtgccggcgattgcggcgccggcaaatattaccgttttctat

SEQ ID NO: 773 - DNA, 69 bp, Artificial Sequence
  Polynucleotide Sequence of aMTD896 5'-primer
gggtttcatatggcgattctgattgtggtggcgccgattgcggcgccggcaaatattaccgttttctat

SEQ ID NO: 774 - DNA, 69 bp, Artificial Sequence
  Polynucleotide Sequence of aMTD897 5'-primer
gggtttcatatggcggtgattgtgccggtggcgattattgcggcgccggcaaatattaccgttttctat

SEQ ID NO: 775 - DNA, 69 bp, Artificial Sequence
  Polynucleotide Sequence of aMTD899 5'-primer
gggtttcatatggcggtggtgattgcgctgccggcggtggtggcgccggcaaatattaccgttttctat

SEQ ID NO: 776 - DNA, 69 bp, Artificial Sequence
  Polynucleotide Sequence of aMTD900 5'-primer
gggtttcatatggcgctggtggcggtgattgcgccggtggtggcgccggcaaatattaccgttttctat

SEQ ID NO: 777 - DNA, 69 bp, Artificial Sequence
  Polynucleotide Sequence of aMTD901 5'-primer
gggtttcatatggcgctggtggcggtgctgccggcggtggcggtgccggcaaatattaccgttttctat

SEQ ID NO: 778 - DNA, 69 bp, Artificial Sequence
  Polynucleotide Sequence of aMTD902 5'-primer
gggtttcatatggcgctggtggcgccgctgctggcggtggcggtgccggcaaatattaccgttttctat

SEQ ID NO: 779 - DNA, 69 bp, Artificial Sequence
  Polynucleotide Sequence of aMTD904 5'-primer
gggtttcatatggcggtgctggcggtggtggcgccggtggtggcgccggcaaatattaccgttttctat

SEQ ID NO: 780 - DNA, 69 bp, Artificial Sequence
  Polynucleotide Sequence of aMTD905 5'-primer
gggtttcatatggcggtgattgcggtggcgccgctggtggtggcgccggcaaatattaccgttttctat

SEQ ID NO: 781 - DNA, 69 bp, Artificial Sequence
  Polynucleotide Sequence of aMTD906 5'-primer
gggtttcatatggcggtgattgcgctggcgccggtggtggtggcgccggcaaatattaccgttttctat

SEQ ID NO: 782 - DNA, 69 bp, Artificial Sequence
  Polynucleotide Sequence of aMTD907 5'-primer
gggtttcatatggtggcgattgcgctggcgccggtggtggtggcgccggcaaatattaccgttttctat

SEQ ID NO: 783 - DNA, 69 bp, Artificial Sequence
  Polynucleotide Sequence of aMTD908 5'-primer
gggtttcatatggtggcgctggcgctggcgccggtggtggtggcgccggcaaatattaccgttttctat

SEQ ID NO: 784 - DNA, 69 bp, Artificial Sequence
  Polynucleotide Sequence of aMTD910 5'-primer
gggtttcatatggtggcggcgctgctgccggcggtggtggtggcgccggcaaatattaccgttttctat

SEQ ID NO: 785 - DNA, 69 bp, Artificial Sequence
  Polynucleotide Sequence of aMTD911 5'-primer
gggtttcatatggtggcgctggcgctgccggcggtggtggtggcgccggcaaatattaccgttttctat

SEQ ID NO: 786 - DNA, 69 bp, Artificial Sequence
  Polynucleotide Sequence of aMTD912 5'-primer
gggtttcatatggtggcgctgctggcgccggcggtggtggtggcgccggcaaatattaccgttttctat

SEQ ID NO: 787 - DNA, 69 bp, Artificial Sequence
  Polynucleotide Sequence of aMTD921 5'-primer
gggtttcatatgatttggtggtttgtggtgctgccgctggtggtgccggcaaatattaccgttttctat

SEQ ID NO: 788 - DNA, 69 bp, Artificial Sequence
  Polynucleotide Sequence of aMTD922 5'-primer
gggtttcatatgtggtatgtgatttttgtgctgccgctggtggtgccggcaaatattaccgttttctat

SEQ ID NO: 789 - DNA, 69 bp, Artificial Sequence
  Polynucleotide Sequence of aMTD931 5'-primer
gggtttcatatggcggtgctgattgcgccggcgattctggcggcggcggcaaatattaccgttttctat

SEQ ID NO: 790 - DNA, 69 bp, Artificial Sequence
  Polynucleotide Sequence of aMTD934 5'-primer
gggtttcatatgctgattctggcgccggcggcggtggtggcggcggcggcaaatattaccgttttctat

SEQ ID NO: 791 - DNA, 69 bp, Artificial Sequence
  Polynucleotide Sequence of aMTD935 5'-primer
gggtttcatatggcgctgctgattctgccggcggcggcggtggcggcggcaaatattaccgttttctat

SEQ ID NO: 792 - DNA, 69 bp, Artificial Sequence
  Polynucleotide Sequence of aMTD936 5'-primer
gggtttcatatggcgctgctgattctggcggcggcggtggcggcgccggcaaatattaccgttttctat

SEQ ID NO: 793 - DNA, 69 bp, Artificial Sequence
  Polynucleotide Sequence of aMTD937 5'-primer
gggtttcatatggtgccggtgctggtgccgctgccggtgccggtggtggcaaatattaccgttttctat

SEQ ID NO: 794 - DNA, 69 bp, Artificial Sequence
  Polynucleotide Sequence of aMTD938 5'-primer
gggtttcatatggtgccggtgctgctgccggtggtggtgccggtgccggcaaatattaccgttttctat

SEQ ID NO: 795 - DNA, 69 bp, Artificial Sequence
  Polynucleotide Sequence of aMTD947 5'-primer
gggtttcatatgtgctattataatcagcagtccaataataataatcaggcaaatattaccgttttctat

SEQ ID NO: 796 - DNA, 69 bp, Artificial Sequence
  Polynucleotide Sequence of aMTD949 5'-primer
gggtttcatatgtccggcaattcctgccagcagtgcggcaattcctccgcaaatattaccgttttctat

SEQ ID NO: 797 - DNA, 39 bp, Artificial Sequence
  Polynucleotide Sequence of aMTD 3'-primer
cgcgtcgacttacctcggctgcaccggcacggagatgac

SEQ ID NO: 798 - protein, 16 aa, Artificial Sequence
  Amino acid Sequence of MTM
AAVALLPAVLLALLAP

SEQ ID NO: 799 - protein, 12 aa, Artificial Sequence
  Amino acid Sequence of MTS
AAVLLPVLLAAP

SEQ ID NO: 800 - protein, 16 aa, Artificial Sequence
  Amino acid Sequence of MTD10
LGGAVVAAPVAAAVAP

SEQ ID NO: 801 - protein, 11 aa, Artificial Sequence
  Amino acid Sequence of MTD13
LAAAALAVLPL

SEQ ID NO: 802 - protein, 10 aa, Artificial Sequence
  Amino acid Sequence of MTD47
AAAVPVLVAA

SEQ ID NO: 803 - protein, 9 aa, Artificial Sequence
  Amino acid Sequence of MTD56
VLLAAALIA

SEQ ID NO: 804 - protein, 7 aa, Artificial Sequence
  Amino acid Sequence of MTD73
PVLLLLA

SEQ ID NO: 805 - protein, 9 aa, Artificial Sequence
  Amino acid Sequence of MTD77
AVALLILAV

SEQ ID NO: 806 - protein, 11 aa, Artificial Sequence
  Amino acid Sequence of MTD84
AVALVAVVAVA

SEQ ID NO: 807 - protein, 11 aa, Artificial Sequence
  Amino acid Sequence of MTD85
LLAAAAALLLA

SEQ ID NO: 808 - protein, 11 aa, Artificial Sequence
  Amino acid Sequence of MTD86
LLAAAAALLLA

SEQ ID NO: 809 - protein, 9 aa, Artificial Sequence
  Amino acid Sequence of MTD103
LALPVLLLA

SEQ ID NO: 810 - protein, 12 aa, Artificial Sequence
  Amino acid Sequence of MTD132
AVVVPAIVLAAP

SEQ ID NO: 811 - protein, 9 aa, Artificial Sequence
  Amino acid Sequence of MTD151
AAAPVAAVP

SEQ ID NO: 812 - protein, 9 aa, Artificial Sequence
  Amino acid Sequence of MTD173
AVIPILAVP

SEQ ID NO: 813 - protein, 11 aa, Artificial Sequence
  Amino acid Sequence of MTD174
LILLLPAVALP

SEQ ID NO: 814 - protein, 9 aa, Artificial Sequence
  Amino acid Sequence of MTD181
AVLLLPAAA

SEQ ID NO: 815 - protein, 12 aa, Artificial Sequence
  Amino acid Sequence of rPeptide ID 931
AVLIAPAILAAA

SEQ ID NO: 816 - protein, 12 aa, Artificial Sequence
  Amino acid Sequence of rPeptide ID 936
ALLILAAAVAAP

SEQ ID NO: 817 - protein, 12 aa, Artificial Sequence
  Amino acid Sequence of rPeptide ID 152
LAAAVAAVAALL

SEQ ID NO: 818 - protein, 12 aa, Artificial Sequence
  Amino acid Sequence of rPeptide ID 27
LAIVAAAAALVA

SEQ ID NO: 819 - protein, 12 aa, Artificial Sequence
  Amino acid Sequence of rPeptide ID 935
ALLILPAAAVAA

SEQ ID NO: 820 - protein, 12 aa, Artificial Sequence
  Amino acid Sequence of rPeptide ID 670
ALLILAAAVAAL

SEQ ID NO: 821 - protein, 12 aa, Artificial Sequence
  Amino acid Sequence of rPeptide ID 934
LILAPAAVVAAA

SEQ ID NO: 822 - protein, 12 aa, Artificial Sequence
  Amino acid Sequence of rPeptide ID 37
TTCSQQQYCTNG

SEQ ID NO: 823 - protein, 12 aa, Artificial Sequence
  Amino acid Sequence of rPeptide ID 16
NNSCTTYTNGSQ

SEQ ID NO: 824 - protein, 12 aa, Artificial Sequence
  Amino acid Sequence of rPeptide ID 113
PVAVALLIAVPP

SEQ ID NO: 825 - protein, 12 aa, Artificial Sequence
  Amino acid Sequence of rPeptide ID 226
ALVAAIPALAIP

SEQ ID NO: 826 - protein, 12 aa, Artificial Sequence
  Amino acid Sequence of rPeptide ID 6
VIAMIPAAFWVA

SEQ ID NO: 827 - protein, 12 aa, Artificial Sequence
  Amino acid Sequence of rPeptide ID 750
LAIAAIAPLAIP

SEQ ID NO: 828 - protein, 12 aa, Artificial Sequence
  Amino acid Sequence of rPeptide ID 26
AAIALAAPLAIV

SEQ ID NO: 829 - protein, 12 aa, Artificial Sequence
  Amino acid Sequence of rPeptide ID 527
LVLAAVAPIAIP

SEQ ID NO: 830 - protein, 12 aa, Artificial Sequence
  Amino acid Sequence of rPeptide ID 466
IIAAAAPLAIIP

SEQ ID NO: 831 - protein, 12 aa, Artificial Sequence
  Amino acid Sequence of rPeptide ID 167
VAIAIPAALAIP

SEQ ID NO: 832 - protein, 12 aa, Artificial Sequence
  Amino acid Sequence of rPeptide ID 246
VVAVPLLVAFAA

SEQ ID NO: 833 - protein, 12 aa, Artificial Sequence
  Amino acid Sequence of rPeptide ID 426
AAALAIPLAIIP

SEQ ID NO: 834 - protein, 12 aa, Artificial Sequence
  Amino acid Sequence of rPeptide ID 606
AAAIAAIPIIIP

SEQ ID NO: 835 - protein, 12 aa, Artificial Sequence
  Amino acid Sequence of rPeptide ID 66
AGVLGGPIMGVP

SEQ ID NO: 836 - protein, 12 aa, Artificial Sequence
  Amino acid Sequence of rPeptide ID 248
VAAIVPIAALVP

SEQ ID NO: 837 - protein, 12 aa, Artificial Sequence
  Amino acid Sequence of rPeptide ID 227
LAAIVPIAAAVP

SEQ ID NO: 838 - protein, 12 aa, Artificial Sequence
  Amino acid Sequence of rPeptide ID 17
GGCSAPQTTCSN

SEQ ID NO: 839 - protein, 12 aa, Artificial Sequence
  Amino acid Sequence of rPeptide ID 67
LDAEVPLADDVP

SEQ ID NO: 840 - protein, 12 aa, Artificial Sequence
  Amino acid Sequence of rPeptide ID 692
PAPLPPVVILAV

SEQ ID NO: 841 - protein, 12 aa, Artificial Sequence
  Amino acid Sequence of rPeptide ID 69
PVAVLPPAALVP

SEQ ID NO: 842 - protein, 12 aa, Artificial Sequence
  Amino acid Sequence of rPeptide ID 390
VPLLVPVVPVVP

SEQ ID NO: 843 - protein, 12 aa, Artificial Sequence
  Amino acid Sequence of rPeptide ID 350
VPILVPVVPVVP

SEQ ID NO: 844 - protein, 12 aa, Artificial Sequence
  Amino acid Sequence of rPeptide ID 331
VPVLVPLVPVVP

SEQ ID NO: 845 - protein, 12 aa, Artificial Sequence
  Amino acid Sequence of rPeptide ID 9
VALVPAALILPP

SEQ ID NO: 846 - protein, 12 aa, Artificial Sequence
  Amino acid Sequence of rPeptide ID 68
VAPVLPAAPLVP

SEQ ID NO: 847 - protein, 12 aa, Artificial Sequence
  Amino acid Sequence of rPeptide ID 349
VPVLVPVVPVVP

SEQ ID NO: 848 - protein, 12 aa, Artificial Sequence
  Amino acid Sequence of rPeptide ID 937
VPVLVPLPVPVV

SEQ ID NO: 849 - protein, 12 aa, Artificial Sequence
  Amino acid Sequence of rPeptide ID 938
VPVLLPVVVPVP

SEQ ID NO: 850 - protein, 12 aa, Artificial Sequence
  Amino acid Sequence of rPeptide ID 329
LPVLVPVVPVVP

SEQ ID NO: 851 - protein, 12 aa, Artificial Sequence
  Amino acid Sequence of rPeptide ID 49
VVPAAPAVPVVP

SEQ ID NO: 852 - protein, 12 aa, Artificial Sequence
  Amino acid Sequence of rPeptide ID 772
LPVAPVIPIIVP

SEQ ID NO: 853 - protein, 12 aa, Artificial Sequence
  Amino acid Sequence of rPeptide ID 210
ALIALPALPALP

SEQ ID NO: 854 - protein, 12 aa, Artificial Sequence
  Amino acid Sequence of rPeptide ID 28
AVPLLPLVPAVP

SEQ ID NO: 855 - protein, 12 aa, Artificial Sequence
  Amino acid Sequence of rPeptide ID 693
AAPVLPVAVPIV

SEQ ID NO: 856 - protein, 12 aa, Artificial Sequence
  Amino acid Sequence of rPeptide ID 169
VALVAPALILAP

SEQ ID NO: 857 - protein, 12 aa, Artificial Sequence
  Amino acid Sequence of rPeptide ID 29
VLPPLPVLPVLP

SEQ ID NO: 858 - protein, 12 aa, Artificial Sequence
  Amino acid Sequence of rPeptide ID 190
AAILAPAVIAPP

SEQ ID NO: 859 - protein, 12 aa, Artificial Sequence
  Amino acid Sequence of rPeptide ID 30
WFFAGPIMLIWP

SEQ ID NO: 860 - protein, 12 aa, Artificial Sequence
  Amino acid Sequence of rPeptide ID 33
AAAILAPAFLAV

SEQ ID NO: 861 - protein, 12 aa, Artificial Sequence
  Amino acid Sequence of rPeptide ID 131
WIIAPVWLAWIA

SEQ ID NO: 862 - protein, 12 aa, Artificial Sequence
  Amino acid Sequence of rPeptide ID 922
WYVIFVLPLVVP

SEQ ID NO: 863 - protein, 12 aa, Artificial Sequence
  Amino acid Sequence of rPeptide ID 71
FMWMWFPFMWYP

SEQ ID NO: 864 - protein, 12 aa, Artificial Sequence
  Amino acid Sequence of rPeptide ID 921
IWWFVVLPLVVP

SEQ ID NO: 865 - protein, 12 aa, Artificial Sequence
  Amino acid Sequence of rPeptide ID 436
VVMLVVPAVMLP

SEQ ID NO: 866 - protein, 12 aa, Artificial Sequence
  Amino acid Sequence of rPeptide ID 138
PPAALLAILAVA

SEQ ID NO: 867 - protein, 12 aa, Artificial Sequence
  Amino acid Sequence of rPeptide ID 77
PVALVLVALVAP

SEQ ID NO: 868 - protein, 12 aa, Artificial Sequence
  Amino acid Sequence of rPeptide ID 577
MLMIALVPMIAV

SEQ ID NO: 869 - protein, 12 aa, Artificial Sequence
  Amino acid Sequence of rPeptide ID 97
ALLAAPPALLAL

SEQ ID NO: 870 - protein, 12 aa, Artificial Sequence
  Amino acid Sequence of rPeptide ID 214
ALIVAPALMALP

SEQ ID NO: 871 - protein, 12 aa, Artificial Sequence
  Amino acid Sequence of rPeptide ID 59
AVLAAPVVAALA

SEQ ID NO: 872 - protein, 12 aa, Artificial Sequence
  Amino acid Sequence of rPeptide ID 54
LAVAAPPVVALL

SEQ ID NO: 873 - protein, 12 aa, Artificial Sequence
  Amino acid Sequence of rPeptide ID 949
SGNSCQQCGNSS

SEQ ID NO: 874 - protein, 12 aa, Artificial Sequence
  Amino acid Sequence of rPeptide ID 39
CYNTSPCTGCCY

SEQ ID NO: 875 - protein, 12 aa, Artificial Sequence
  Amino acid Sequence of rPeptide ID 19
YVSCCTYTNGSQ

SEQ ID NO: 876 - protein, 12 aa, Artificial Sequence
  Amino acid Sequence of rPeptide ID 947
CYYNQQSNNNNQ

SEQ ID NO: 877 - protein, 12 aa, Artificial Sequence
  Amino acid Sequence of rPeptide ID 139
TGSTNSPTCTST

SEQ ID NO: 878 - protein, 12 aa, Artificial Sequence
  Amino acid Sequence of rPeptide ID 18
NYCCTPTTNGQS

SEQ ID NO: 879 - protein, 12 aa, Artificial Sequence
  Amino acid Sequence of rPeptide ID 20
NYCNTCPTYGQS

SEQ ID NO: 880 - protein, 12 aa, Artificial Sequence
  Amino acid Sequence of rPeptide ID 635
GSTGGSQQNNQY

SEQ ID NO: 881 - protein, 12 aa, Artificial Sequence
  Amino acid Sequence of rPeptide ID 40
TYNTSCTPGTCY

SEQ ID NO: 882 - protein, 12 aa, Artificial Sequence
  Amino acid Sequence of rPeptide ID 57
QNNCNTSSQGGG

SEQ ID NO: 883 - protein, 12 aa, Artificial Sequence
  Amino acid Sequence of rPeptide ID 159
CYSGSTSQNQPP

SEQ ID NO: 884 - protein, 12 aa, Artificial Sequence
  Amino acid Sequence of rPeptide ID 700
GTSNTCQSNQNS

SEQ ID NO: 885 - protein, 12 aa, Artificial Sequence
  Amino acid Sequence of rPeptide ID 38
YYNQSTCGGQCY

SEQ ID NO: 886 - protein, 22 aa, Artificial Sequence
  Amino acid Sequence of aMTD1 5'-primer
GFHMAAALAPVVLALPANITVF

SEQ ID NO: 887 - protein, 22 aa, Artificial Sequence
  Amino acid Sequence of aMTD2 5'-primer
GFHMAAAVPLLAVVVPANITVF

SEQ ID NO: 888 - protein, 22 aa, Artificial Sequence
  Amino acid Sequence of aMTD3 5'-primer
GFHMAALLVPAAVLAPANITVF

SEQ ID NO: 889 - protein, 22 aa, Artificial Sequence
  Amino acid Sequence of aMTD4 5'-primer
GFHMALALLPVAALAPANITVF

SEQ ID NO: 890 - protein, 22 aa, Artificial Sequence
  Amino acid Sequence of aMTD5 5'-primer
GFHMAAALLPVALVAPANITVF

SEQ ID NO: 891 - protein, 22 aa, Artificial Sequence
  Amino acid Sequence of aMTD6 5'-primer
GFHMVIAMIPAAFWVAANITVF

SEQ ID NO: 892 - protein, 22 aa, Artificial Sequence
  Amino acid Sequence of aMTD9 5'-primer
GFHMVALVPAALILPPANITVF

SEQ ID NO: 893 - protein, 22 aa, Artificial Sequence
  Amino acid Sequence of aMTD11 5'-primer
GFHMVVALAPALAALPANITVF

SEQ ID NO: 894 - protein, 22 aa, Artificial Sequence
  Amino acid Sequence of aMTD12 5'-primer
GFHMLLAAVPAVLLAPANITVF

SEQ ID NO: 895 - protein, 22 aa, Artificial Sequence
  Amino acid Sequence of aMTD13 5'-primer
GFHMAAALVPVVALLPANITVF

SEQ ID NO: 896 - protein, 22 aa, Artificial Sequence
  Amino acid Sequence of aMTD16 5'-primer
GFHMNNSCTTYTNGSQANITVF

SEQ ID NO: 897 - protein, 22 aa, Artificial Sequence
  Amino acid Sequence of aMTD17 5'-primer
GFHMGGCSAPQTTCSNANITVF

SEQ ID NO: 898 - protein, 22 aa, Artificial Sequence
  Amino acid Sequence of aMTD18 5'-primer
GFHMNYCCTPTTNGQSANITVF

SEQ ID NO: 899 - protein, 22 aa, Artificial Sequence
  Amino acid Sequence of aMTD19 5'-primer
GFHMYVSCCTYTNGSQANITVF

SEQ ID NO: 900 - protein, 22 aa, Artificial Sequence
  Amino acid Sequence of aMTD20 5'-primer
GFHMNYCNTCPTYGQSANITVF

SEQ ID NO: 901 - protein, 22 aa, Artificial Sequence
  Amino acid Sequence of aMTD21 5'-primer
GFHMAVALLPALLAVPANITVF

SEQ ID NO: 902 - protein, 22 aa, Artificial Sequence
  Amino acid Sequence of aMTD22 5'-primer
GFHMAVVLVPVLAAAPANITVF

SEQ ID NO: 903 - protein, 22 aa, Artificial Sequence
  Amino acid Sequence of aMTD23 5'-primer
GFHMVVLVLPAAAAVPANITVF

SEQ ID NO: 904 - protein, 22 aa, Artificial Sequence
  Amino acid Sequence of aMTD24 5'-primer
GFHMIALAAPALIVAPANITVF

SEQ ID NO: 905 - protein, 22 aa, Artificial Sequence
  Amino acid Sequence of aMTD25 5'-primer
GFHMIVAVAPALVALPANITVF

SEQ ID NO: 906 - protein, 22 aa, Artificial Sequence
  Amino acid Sequence of aMTD26 5'-primer
GFHMAAIALAAPLAIVANITVF

SEQ ID NO: 907 - protein, 22 aa, Artificial Sequence
  Amino acid Sequence of aMTD27 5'-primer
GFHMLAIVAAAAALVAANITVF

SEQ ID NO: 908 - protein, 22 aa, Artificial Sequence
  Amino acid Sequence of aMTD28 5'-primer
GFHMAVPLLPLVPAVPANITVF

SEQ ID NO: 909 - protein, 22 aa, Artificial Sequence
  Amino acid Sequence of aMTD29 5'-primer
GFHMVLPPLPVLPVLPANITVF

SEQ ID NO: 910 - protein, 22 aa, Artificial Sequence
  Amino acid Sequence of aMTD30 5'-primer
GFHMAMALLPAAVAVAANITVF

SEQ ID NO: 911 - protein, 22 aa, Artificial Sequence
  Amino acid Sequence of aMTD33 5'-primer
GFHMAAAILAPAFLAVANITVF

SEQ ID NO: 912 - protein, 22 aa, Artificial Sequence
  Amino acid Sequence of aMTD37 5'-primer
GFHMTTCSQQQYCTNGANITVF

SEQ ID NO: 913 - protein, 22 aa, Artificial Sequence
  Amino acid Sequence of aMTD38 5'-primer
GFHMYYNQSTCGGQCYANITVF

SEQ ID NO: 914 - protein, 22 aa, Artificial Sequence
  Amino acid Sequence of aMTD39 5'-primer
GFHMCYNTSPCTGCCYANITVF

SEQ ID NO: 915 - protein, 22 aa, Artificial Sequence
  Amino acid Sequence of aMTD40 5'-primer
GFHMTYNTSCTPGTCYANITVF

SEQ ID NO: 916 - protein, 22 aa, Artificial Sequence
  Amino acid Sequence of aMTD42 5'-primer
GFHMVAALPVVAVVAPANITVF

SEQ ID NO: 917 - protein, 22 aa, Artificial Sequence
  Amino acid Sequence of aMTD43 5'-primer
GFHMLLAAPLVVAAVPANITVF

SEQ ID NO: 918 - protein, 22 aa, Artificial Sequence
  Amino acid Sequence of aMTD44 5'-primer
GFHMALAVPVALLVAPANITVF

SEQ ID NO: 919 - protein, 22 aa, Artificial Sequence
  Amino acid Sequence of aMTD49 5'-primer
GFHMVVPAAPAVPVVPANITVF

SEQ ID NO: 920 - protein, 22 aa, Artificial Sequence
  Amino acid Sequence of aMTD54 5'-primer
GFHMLAVAAPPVVALLANITVF

SEQ ID NO: 921 - protein, 22 aa, Artificial Sequence
  Amino acid Sequence of aMTD57 5'-primer
GFHMQNNCNTSSQGGGANITVF

SEQ ID NO: 922 - protein, 22 aa, Artificial Sequence
  Amino acid Sequence of aMTD59 5'-primer
GFHMAVLAAPVVAALAANITVF

SEQ ID NO: 923 - protein, 22 aa, Artificial Sequence
  Amino acid Sequence of aMTD61 5'-primer
GFHMVAALPVLLAALPANITVF

SEQ ID NO: 924 - protein, 22 aa, Artificial Sequence
  Amino acid Sequence of aMTD62 5'-primer
GFHMVALLAPVALAVPANITVF

SEQ ID NO: 925 - protein, 22 aa, Artificial Sequence
  Amino acid Sequence of aMTD63 5'-primer
GFHMAALLVPALVAVPANITVF

SEQ ID NO: 926 - protein, 22 aa, Artificial Sequence
  Amino acid Sequence of aMTD64 5'-primer
GFHMAIVALPVAVLAPANITVF

SEQ ID NO: 927 - protein, 22 aa, Artificial Sequence
  Amino acid Sequence of aMTD65 5'-primer
GFHMIAIVAPVVALAPANITVF

SEQ ID NO: 928 - protein, 22 aa, Artificial Sequence
  Amino acid Sequence of aMTD66 5'-primer
GFHMAGVLGGPIMGVPANITVF

SEQ ID NO: 929 - protein, 22 aa, Artificial Sequence
  Amino acid Sequence of aMTD67 5'-primer
GFHMLDAEVPLADDVPANITVF

SEQ ID NO: 930 - protein, 22 aa, Artificial Sequence
  Amino acid Sequence of aMTD68 5'-primer
GFHMVAPVLPAAPLVPANITVF

SEQ ID NO: 931 - protein, 22 aa, Artificial Sequence
  Amino acid Sequence of aMTD69 5'-primer
GFHMPVAVLPPAALVPANITVF

SEQ ID NO: 932 - protein, 22 aa, Artificial Sequence
  Amino acid Sequence of aMTD71 5'-primer
GFHMFMWMWFPFMWYPANITVF

SEQ ID NO: 933 - protein, 22 aa, Artificial Sequence
  Amino acid Sequence of aMTD77 5'-primer
GFHMAMLLMPIVLIAPANITVF

SEQ ID NO: 934 - protein, 22 aa, Artificial Sequence
  Amino acid Sequence of aMTD81 5'-primer
GFHMAALLPALAALLPANITVF

SEQ ID NO: 935 - protein, 22 aa, Artificial Sequence
  Amino acid Sequence of aMTD82 5'-primer
GFHMAVVLAPVAAVLPANITVF

SEQ ID NO: 936 - protein, 22 aa, Artificial Sequence
  Amino acid Sequence of aMTD83 5'-primer
GFHMLAVAAPLALALPANITVF

SEQ ID NO: 937 - protein, 22 aa, Artificial Sequence
  Amino acid Sequence of aMTD84 5'-primer
GFHMAAVAAPLLLALPANITVF

SEQ ID NO: 938 - protein, 22 aa, Artificial Sequence
  Amino acid Sequence of aMTD85 5'-primer
GFHMLLVLPAAALAAPANITVF

SEQ ID NO: 939 - protein, 22 aa, Artificial Sequence
  Amino acid Sequence of aMTD97 5'-primer
GFHMALLAAPPALLALANITVF

SEQ ID NO: 940 - protein, 22 aa, Artificial Sequence
  Amino acid Sequence of aMTD101 5'-primer
GFHMLVALAPVAAVLPANITVF

SEQ ID NO: 941 - protein, 22 aa, Artificial Sequence
  Amino acid Sequence of aMTD102 5'-primer
GFHMLALAPAALALLPANITVF

SEQ ID NO: 942 - protein, 22 aa, Artificial Sequence
  Amino acid Sequence of aMTD103 5'-primer
GFHMALIAAPILALAPANITVF

SEQ ID NO: 943 - protein, 22 aa, Artificial Sequence
  Amino acid Sequence of aMTD104 5'-primer
GFHMAVVAAPLVLALPANITVF

SEQ ID NO: 944 - protein, 22 aa, Artificial Sequence
  Amino acid Sequence of aMTD105 5'-primer
GFHMLLALAPAALLAPANITVF

SEQ ID NO: 945 - protein, 22 aa, Artificial Sequence
  Amino acid Sequence of aMTD113 5'-primer
GFHMPVAVALLIAVPPANITVF

SEQ ID NO: 946 - protein, 22 aa, Artificial Sequence
  Amino acid Sequence of aMTD121 5'-primer
GFHMAIVALPALALAPANITVF

SEQ ID NO: 947 - protein, 22 aa, Artificial Sequence
  Amino acid Sequence of aMTD123 5'-primer
GFHMAAIIVPAALLAPANITVF

SEQ ID NO: 948 - protein, 22 aa, Artificial Sequence
  Amino acid Sequence of aMTD124 5'-primer
GFHMIAVALPALIAAPANITVF

SEQ ID NO: 949 - protein, 22 aa, Artificial Sequence
  Amino acid Sequence of aMTD131 5'-primer
GFHMWIIAPVWLAWIAANITVF

SEQ ID NO: 950 - protein, 22 aa, Artificial Sequence
  Amino acid Sequence of aMTD138 5'-primer
GFHMPPAALLAILAVAANITVF

SEQ ID NO: 951 - protein, 22 aa, Artificial Sequence
  Amino acid Sequence of aMTD139 5'-primer
GFHMTGSTNSPTCTSTANITVF

SEQ ID NO: 952 - protein, 22 aa, Artificial Sequence
  Amino acid Sequence of aMTD141 5'-primer
GFHMAVIVLPALAVAPANITVF

SEQ ID NO: 953 - protein, 22 aa, Artificial Sequence
  Amino acid Sequence of aMTD142 5'-primer
GFHMLLAAVPVALVAPANITVF

SEQ ID NO: 954 - protein, 22 aa, Artificial Sequence
  Amino acid Sequence of aMTD143 5'-primer
GFHMAVLAVPAVLVAPANITVF

SEQ ID NO: 955 - protein, 22 aa, Artificial Sequence
  Amino acid Sequence of aMTD144 5'-primer
GFHMVLAIVPAVALAPANITVF

SEQ ID NO: 956 - protein, 22 aa, Artificial Sequence
  Amino acid Sequence of aMTD145 5'-primer
GFHMLLAVVPAVALAPANITVF

SEQ ID NO: 957 - protein, 22 aa, Artificial Sequence
  Amino acid Sequence of aMTD152 5'-primer
GFHMLAAAVAAVAALLANITVF

SEQ ID NO: 958 - protein, 22 aa, Artificial Sequence
  Amino acid Sequence of aMTD159 5'-primer
GFHMCYSGSTSQNQPPANITVF

SEQ ID NO: 959 - protein, 22 aa, Artificial Sequence
  Amino acid Sequence of aMTD161 5'-primer
GFHMAVIALPALIAAPANITVF

SEQ ID NO: 960 - protein, 22 aa, Artificial Sequence
  Amino acid Sequence of aMTD162 5'-primer
GFHMAVVALPAALIVPANITVF

SEQ ID NO: 961 - protein, 22 aa, Artificial Sequence
  Amino acid Sequence of aMTD163 5'-primer
GFHMLALVLPAALAAPANITVF

SEQ ID NO: 962 - protein, 22 aa, Artificial Sequence
  Amino acid Sequence of aMTD164 5'-primer
GFHMLAAVLPALLAAPANITVF

SEQ ID NO: 963 - protein, 22 aa, Artificial Sequence
  Amino acid Sequence of aMTD165 5'-primer
GFHMALAVPVALAIVPANITVF

SEQ ID NO: 964 - protein, 22 aa, Artificial Sequence
  Amino acid Sequence of aMTD167 5'-primer
GFHMVAIAIPAALAIPANITVF

SEQ ID NO: 965 - protein, 22 aa, Artificial Sequence
  Amino acid Sequence of aMTD169 5'-primer
GFHMVALVAPALILAPANITVF

SEQ ID NO: 966 - protein, 22 aa, Artificial Sequence
  Amino acid Sequence of aMTD182 5'-primer
GFHMALIAPVVALVAPANITVF

SEQ ID NO: 967 - protein, 22 aa, Artificial Sequence
  Amino acid Sequence of aMTD183 5'-primer
GFHMLLAAPVVIALAPANITVF

SEQ ID NO: 968 - protein, 22 aa, Artificial Sequence
  Amino acid Sequence of aMTD184 5'-primer
GFHMLAAIVPAIIAVPANITVF

SEQ ID NO: 969 - protein, 22 aa, Artificial Sequence
  Amino acid Sequence of aMTD185 5'-primer
GFHMAALVLPLIIAAPANITVF

SEQ ID NO: 970 - protein, 22 aa, Artificial Sequence
  Amino acid Sequence of aMTD189 5'-primer
GFHMVILVAPAVIAPPANITVF

SEQ ID NO: 971 - protein, 22 aa, Artificial Sequence
  Amino acid Sequence of aMTD190 5'-primer
GFHMAAILAPAVIAPPANITVF

SEQ ID NO: 972 - protein, 22 aa, Artificial Sequence
  Amino acid Sequence of aMTD201 5'-primer
GFHMLALAVPALAALPANITVF

SEQ ID NO: 973 - protein, 22 aa, Artificial Sequence
  Amino acid Sequence of aMTD204 5'-primer
GFHMLIAALPAVAALPANITVF

SEQ ID NO: 974 - protein, 22 aa, Artificial Sequence
  Amino acid Sequence of aMTD205 5'-primer
GFHMALALVPAIAALPANITVF

SEQ ID NO: 975 - protein, 22 aa, Artificial Sequence
  Amino acid Sequence of aMTD210 5'-primer
GFHMALIALPALPALPANITVF

SEQ ID NO: 976 - protein, 22 aa, Artificial Sequence
  Amino acid Sequence of aMTD214 5'-primer
GFHMALIVAPALMALPANITVF

SEQ ID NO: 977 - protein, 22 aa, Artificial Sequence
  Amino acid Sequence of aMTD221 5'-primer
GFHMAAILAPIVALAPANITVF

SEQ ID NO: 978 - protein, 22 aa, Artificial Sequence
  Amino acid Sequence of aMTD222 5'-primer
GFHMALLIAPAAVIAPANITVF

SEQ ID NO: 979 - protein, 22 aa, Artificial Sequence
  Amino acid Sequence of aMTD223 5'-primer
GFHMAILAVPIAVVAPANITVF

SEQ ID NO: 980 - protein, 22 aa, Artificial Sequence
  Amino acid Sequence of aMTD224 5'-primer
GFHMILAAVPIALAAPANITVF

SEQ ID NO: 981 - protein, 22 aa, Artificial Sequence
  Amino acid Sequence of aMTD225 5'-primer
GFHMVAALLPAAAVLPANITVF

SEQ ID NO: 982 - protein, 22 aa, Artificial Sequence
  Amino acid Sequence of aMTD226 5'-primer
GFHMALVAAIPALAIPANITVF

SEQ ID NO: 983 - protein, 22 aa, Artificial Sequence
  Amino acid Sequence of aMTD227 5'-primer
GFHMLAAIVPIAAAVPANITVF

SEQ ID NO: 984 - protein, 22 aa, Artificial Sequence
  Amino acid Sequence of aMTD241 5'-primer
GFHMAAAVVPVLLVAPANITVF

SEQ ID NO: 985 - protein, 22 aa, Artificial Sequence
  Amino acid Sequence of aMTD242 5'-primer
GFHMAALLVPALVAAPANITVF

SEQ ID NO: 986 - protein, 22 aa, Artificial Sequence
  Amino acid Sequence of aMTD243 5'-primer
GFHMAAVLLPVALAAPANITVF

SEQ ID NO: 987 - protein, 22 aa, Artificial Sequence
  Amino acid Sequence of aMTD245 5'-primer
GFHMAAALAPVLALVPANITVF

SEQ ID NO: 988 - protein, 22 aa, Artificial Sequence
  Amino acid Sequence of aMTD246 5'-primer
GFHMVVAVPLLVAFAAANITVF

SEQ ID NO: 989 - protein, 22 aa, Artificial Sequence
  Amino acid Sequence of aMTD248 5'-primer
GFHMVAAIVPIAALVPANITVF

SEQ ID NO: 990 - protein, 22 aa, Artificial Sequence
  Amino acid Sequence of aMTD261 5'-primer
GFHMLVLVPLLAAAAPANITVF

SEQ ID NO: 991 - protein, 22 aa, Artificial Sequence
  Amino acid Sequence of aMTD262 5'-primer
GFHMALIAVPAIIVAPANITVF

SEQ ID NO: 992 - protein, 22 aa, Artificial Sequence
  Amino acid Sequence of aMTD263 5'-primer
GFHMALAVIPAAAILPANITVF

SEQ ID NO: 993 - protein, 22 aa, Artificial Sequence
  Amino acid Sequence of aMTD264 5'-primer
GFHMLAAAPVVIVIAPANITVF

SEQ ID NO: 994 - protein, 22 aa, Artificial Sequence
  Amino acid Sequence of aMTD265 5'-primer
GFHMVLAIAPLLAAVPANITVF

SEQ ID NO: 995 - protein, 22 aa, Artificial Sequence
  Amino acid Sequence of aMTD281 5'-primer
GFHMALIVLPAAVAVPANITVF

SEQ ID NO: 996 - protein, 22 aa, Artificial Sequence
  Amino acid Sequence of aMTD282 5'-primer
GFHMVLAVAPALIVAPANITVF

SEQ ID NO: 997 - protein, 22 aa, Artificial Sequence
  Amino acid Sequence of aMTD283 5'-primer
GFHMAALLAPALIVAPANITVF

SEQ ID NO: 998 - protein, 22 aa, Artificial Sequence
  Amino acid Sequence of aMTD284 5'-primer
GFHMALIAPAVALIVPANITVF

SEQ ID NO: 999 - protein, 22 aa, Artificial Sequence
  Amino acid Sequence of aMTD285 5'-primer
GFHMAIVLLPAAVVAPANITVF

SEQ ID NO: 1000 - protein, 22 aa, Artificial Sequence
  Amino acid Sequence of aMTD301 5'-primer
GFHMVIAAPVLAVLAPANITVF

SEQ ID NO: 1001 - protein, 22 aa, Artificial Sequence
  Amino acid Sequence of aMTD302 5'-primer
GFHMLALAPALALLAPANITVF

SEQ ID NO: 1002 - protein, 22 aa, Artificial Sequence
  Amino acid Sequence of aMTD304 5'-primer
GFHMAIILAPIAAIAPANITVF

SEQ ID NO: 1003 - protein, 22 aa, Artificial Sequence
  Amino acid Sequence of aMTD305 5'-primer
GFHMIALAAPILLAAPANITVF

SEQ ID NO: 1004 - protein, 22 aa, Artificial Sequence
  Amino acid Sequence of aMTD321 5'-primer
GFHMIVAVALPALAVPANITVF

SEQ ID NO: 1005 - protein, 22 aa, Artificial Sequence
  Amino acid Sequence of aMTD322 5'-primer
GFHMVVAIVLPALAAPANITVF

SEQ ID NO: 1006 - protein, 22 aa, Artificial Sequence
  Amino acid Sequence of aMTD323 5'-primer
GFHMIVAVALPVALAPANITVF

SEQ ID NO: 1007 - protein, 22 aa, Artificial Sequence
  Amino acid Sequence of aMTD324 5'-primer
GFHMIVAVALPAALVPANITVF

SEQ ID NO: 1008 - protein, 22 aa, Artificial Sequence
  Amino acid Sequence of aMTD325 5'-primer
GFHMIVAVALPAVALPANITVF

SEQ ID NO: 1009 - protein, 22 aa, Artificial Sequence
  Amino acid Sequence of aMTD329 5'-primer
GFHMLPVLVPVVPVVPANITVF

SEQ ID NO: 1010 - protein, 22 aa, Artificial Sequence
  Amino acid Sequence of aMTD331 5'-primer
GFHMVPVLVPLVPVVPANITVF

SEQ ID NO: 1011 - protein, 22 aa, Artificial Sequence
  Amino acid Sequence of aMTD341 5'-primer
GFHMIVAVALPAVLAPANITVF

SEQ ID NO: 1012 - protein, 22 aa, Artificial Sequence
  Amino acid Sequence of aMTD342 5'-primer
GFHMVIVALAPAVLAPANITVF

SEQ ID NO: 1013 - protein, 22 aa, Artificial Sequence
  Amino acid Sequence of aMTD343 5'-primer
GFHMIVAVALPALVAPANITVF

SEQ ID NO: 1014 - protein, 22 aa, Artificial Sequence
  Amino acid Sequence of aMTD345 5'-primer
GFHMALLIVAPVAVAPANITVF

SEQ ID NO: 1015 - protein, 22 aa, Artificial Sequence
  Amino acid Sequence of aMTD349 5'-primer
GFHMVPVLVPVVPVVPANITVF

SEQ ID NO: 1016 - protein, 22 aa, Artificial Sequence
  Amino acid Sequence of aMTD350 5'-primer
GFHMVPILVPVVPVVPANITVF

SEQ ID NO: 1017 - protein, 22 aa, Artificial Sequence
  Amino acid Sequence of aMTD361 5'-primer
GFHMAVVIVAPAVIAPANITVF

SEQ ID NO: 1018 - protein, 22 aa, Artificial Sequence
  Amino acid Sequence of aMTD363 5'-primer
GFHMAVLAVAPALIVPANITVF

SEQ ID NO: 1019 - protein, 22 aa, Artificial Sequence
  Amino acid Sequence of aMTD364 5'-primer
GFHMLVAAVAPALIVPANITVF

SEQ ID NO: 1020 - protein, 22 aa, Artificial Sequence
  Amino acid Sequence of aMTD365 5'-primer
GFHMAVIVVAPALLAPANITVF

SEQ ID NO: 1021 - protein, 22 aa, Artificial Sequence
  Amino acid Sequence of aMTD381 5'-primer
GFHMVVAIVLPAVAAPANITVF

SEQ ID NO: 1022 - protein, 22 aa, Artificial Sequence
  Amino acid Sequence of aMTD382 5'-primer
GFHMAAALVIPAILAPANITVF

SEQ ID NO: 1023 - protein, 22 aa, Artificial Sequence
  Amino acid Sequence of aMTD383 5'-primer
GFHMVIVALAPALLAPANITVF

SEQ ID NO: 1024 - protein, 22 aa, Artificial Sequence
  Amino acid Sequence of aMTD384 5'-primer
GFHMVIVAIAPALLAPANITVF

SEQ ID NO: 1025 - protein, 22 aa, Artificial Sequence
  Amino acid Sequence of aMTD385 5'-primer
GFHMIVAIAVPALVAPANITVF

SEQ ID NO: 1026 - protein, 22 aa, Artificial Sequence
  Amino acid Sequence of aMTD390 5'-primer
GFHMVPLLVPVVPVVPANITVF

SEQ ID NO: 1027 - protein, 22 aa, Artificial Sequence
  Amino acid Sequence of aMTD401 5'-primer
GFHMAALAVIPAAILPANITVF

SEQ ID NO: 1028 - protein, 22 aa, Artificial Sequence
  Amino acid Sequence of aMTD402 5'-primer
GFHMALAAVIPAAILPANITVF

SEQ ID NO: 1029 - protein, 22 aa, Artificial Sequence
  Amino acid Sequence of aMTD403 5'-primer
GFHMAAALVIPAAILPANITVF

SEQ ID NO: 1030 - protein, 22 aa, Artificial Sequence
  Amino acid Sequence of aMTD404 5'-primer
GFHMLAAAVIPAAILPANITVF

SEQ ID NO: 1031 - protein, 22 aa, Artificial Sequence
  Amino acid Sequence of aMTD405 5'-primer
GFHMLAAAVIPVAILPANITVF

SEQ ID NO: 1032 - protein, 22 aa, Artificial Sequence
  Amino acid Sequence of aMTD421 5'-primer
GFHMAAILAAPLIAVPANITVF

SEQ ID NO: 1033 - protein, 22 aa, Artificial Sequence
  Amino acid Sequence of aMTD422 5'-primer
GFHMVVAILAPLLAAPANITVF

SEQ ID NO: 1034 - protein, 22 aa, Artificial Sequence
  Amino acid Sequence of aMTD424 5'-primer
GFHMAVVVAAPVLALPANITVF

SEQ ID NO: 1035 - protein, 22 aa, Artificial Sequence
  Amino acid Sequence of aMTD425 5'-primer
GFHMAVVAIAPVLALPANITVF

SEQ ID NO: 1036 - protein, 22 aa, Artificial Sequence
  Amino acid Sequence of aMTD426 5'-primer
GFHMAAALAIPLAIIPANITVF

SEQ ID NO: 1037 - protein, 22 aa, Artificial Sequence
  Amino acid Sequence of aMTD436 5'-primer
GFHMAVVLVIMPAAIPANITVF

SEQ ID NO: 1038 - protein, 22 aa, Artificial Sequence
  Amino acid Sequence of aMTD442 5'-primer
GFHMALAALVPAVLVPANITVF

SEQ ID NO: 1039 - protein, 22 aa, Artificial Sequence
  Amino acid Sequence of aMTD443 5'-primer
GFHMALAALVPVALVPANITVF

SEQ ID NO: 1040 - protein, 22 aa, Artificial Sequence
  Amino acid Sequence of aMTD444 5'-primer
GFHMLAAALVPVALVPANITVF

SEQ ID NO: 1041 - protein, 22 aa, Artificial Sequence
  Amino acid Sequence of aMTD445 5'-primer
GFHMALAALVPALVVPANITVF

SEQ ID NO: 1042 - protein, 22 aa, Artificial Sequence
  Amino acid Sequence of aMTD461 5'-primer
GFHMIAAVIVPAVALPANITVF

SEQ ID NO: 1043 - protein, 22 aa, Artificial Sequence
  Amino acid Sequence of aMTD462 5'-primer
GFHMIAAVLVPAVALPANITVF

SEQ ID NO: 1044 - protein, 22 aa, Artificial Sequence
  Amino acid Sequence of aMTD463 5'-primer
GFHMAVAILVPLLAAPANITVF

SEQ ID NO: 1045 - protein, 22 aa, Artificial Sequence
  Amino acid Sequence of aMTD464 5'-primer
GFHMAVVILVPLAAAPANITVF

SEQ ID NO: 1046 - protein, 22 aa, Artificial Sequence
  Amino acid Sequence of aMTD465 5'-primer
GFHMIAAVIVPVAALPANITVF

SEQ ID NO: 1047 - protein, 22 aa, Artificial Sequence
  Amino acid Sequence of aMTD466 5'-primer
GFHMIIAAAAPLAIIPANITVF

SEQ ID NO: 1048 - protein, 22 aa, Artificial Sequence
  Amino acid Sequence of aMTD481 5'-primer
GFHMAIAIAIVPVALPANITVF

SEQ ID NO: 1049 - protein, 22 aa, Artificial Sequence
  Amino acid Sequence of aMTD482 5'-primer
GFHMILAVAAIPVAVPANITVF

SEQ ID NO: 1050 - protein, 22 aa, Artificial Sequence
  Amino acid Sequence of aMTD483 5'-primer
GFHMILAAAIIPAALPANITVF

SEQ ID NO: 1051 - protein, 22 aa, Artificial Sequence
  Amino acid Sequence of aMTD484 5'-primer
GFHMLAVVLAAPAIVPANITVF

SEQ ID NO: 1052 - protein, 22 aa, Artificial Sequence
  Amino acid Sequence of aMTD485 5'-primer
GFHMAILAAIVPLAVPANITVF

SEQ ID NO: 1053 - protein, 22 aa, Artificial Sequence
  Amino acid Sequence of aMTD501 5'-primer
GFHMVIVALAVPALAPANITVF

SEQ ID NO: 1054 - protein, 22 aa, Artificial Sequence
  Amino acid Sequence of aMTD502 5'-primer
GFHMAIVALAVPVLAPANITVF

SEQ ID NO: 1055 - protein, 22 aa, Artificial Sequence
  Amino acid Sequence of aMTD503 5'-primer
GFHMAAIIIVLPAALPANITVF

SEQ ID NO: 1056 - protein, 22 aa, Artificial Sequence
  Amino acid Sequence of aMTD504 5'-primer
GFHMLIVALAVPALAPANITVF

SEQ ID NO: 1057 - protein, 22 aa, Artificial Sequence
  Amino acid Sequence of aMTD505 5'-primer
GFHMAIIIVIAPAAAPANITVF

SEQ ID NO: 1058 - protein, 22 aa, Artificial Sequence
  Amino acid Sequence of aMTD521 5'-primer
GFHMLAALIVVPAVAPANITVF

SEQ ID NO: 1059 - protein, 22 aa, Artificial Sequence
  Amino acid Sequence of aMTD522 5'-primer
GFHMALLVIAVPAVAPANITVF

SEQ ID NO: 1060 - protein, 22 aa, Artificial Sequence
  Amino acid Sequence of aMTD524 5'-primer
GFHMAVALIVVPALAPANITVF

SEQ ID NO: 1061 - protein, 22 aa, Artificial Sequence
  Amino acid Sequence of aMTD525 5'-primer
GFHMALAIVVAPVAVPANITVF

SEQ ID NO: 1062 - protein, 22 aa, Artificial Sequence
  Amino acid Sequence of aMTD527 5'-primer
GFHMLVLAAVAPIAIPANITVF

SEQ ID NO: 1063 - protein, 22 aa, Artificial Sequence
  Amino acid Sequence of aMTD541 5'-primer
GFHMLLALIIAPAAAPANITVF

SEQ ID NO: 1064 - protein, 22 aa, Artificial Sequence
  Amino acid Sequence of aMTD542 5'-primer
GFHMALALIIVPAVAPANITVF

SEQ ID NO: 1065 - protein, 22 aa, Artificial Sequence
  Amino acid Sequence of aMTD543 5'-primer
GFHMLLAALIAPAALPANITVF

SEQ ID NO: 1066 - protein, 22 aa, Artificial Sequence
  Amino acid Sequence of aMTD544 5'-primer
GFHMIVALIVAPAAVPANITVF

SEQ ID NO: 1067 - protein, 22 aa, Artificial Sequence
  Amino acid Sequence of aMTD545 5'-primer
GFHMVVLVLAAPAAVPANITVF

SEQ ID NO: 1068 - protein, 22 aa, Artificial Sequence
  Amino acid Sequence of aMTD561 5'-primer
GFHMAAVAIVLPAVVPANITVF

SEQ ID NO: 1069 - protein, 22 aa, Artificial Sequence
  Amino acid Sequence of aMTD562 5'-primer
GFHMALIAAIVPALVPANITVF

SEQ ID NO: 1070 - protein, 22 aa, Artificial Sequence
  Amino acid Sequence of aMTD563 5'-primer
GFHMALAVIVVPALAPANITVF

SEQ ID NO: 1071 - protein, 22 aa, Artificial Sequence
  Amino acid Sequence of aMTD564 5'-primer
GFHMVAIALIVPALAPANITVF

SEQ ID NO: 1072 - protein, 22 aa, Artificial Sequence
  Amino acid Sequence of aMTD565 5'-primer
GFHMVAIVLVAPAVAPANITVF

SEQ ID NO: 1073 - protein, 22 aa, Artificial Sequence
  Amino acid Sequence of aMTD577 5'-primer
GFHMAAVLIVPIMVMPANITVF

SEQ ID NO: 1074 - protein, 22 aa, Artificial Sequence
  Amino acid Sequence of aMTD582 5'-primer
GFHMVAVALIVPALAPANITVF

SEQ ID NO: 1075 - protein, 22 aa, Artificial Sequence
  Amino acid Sequence of aMTD583 5'-primer
GFHMAVILALAPIVAPANITVF

SEQ ID NO: 1076 - protein, 22 aa, Artificial Sequence
  Amino acid Sequence of aMTD585 5'-primer
GFHMALIVAIAPALVPANITVF

SEQ ID NO: 1077 - protein, 22 aa, Artificial Sequence
  Amino acid Sequence of aMTD601 5'-primer
GFHMAAILIAVPIAAPANITVF

SEQ ID NO: 1078 - protein, 22 aa, Artificial Sequence
  Amino acid Sequence of aMTD602 5'-primer
GFHMVIVALAAPVLAPANITVF

SEQ ID NO: 1079 - protein, 22 aa, Artificial Sequence
  Amino acid Sequence of aMTD603 5'-primer
GFHMVLVALAAPVIAPANITVF

SEQ ID NO: 1080 - protein, 22 aa, Artificial Sequence
  Amino acid Sequence of aMTD604 5'-primer
GFHMVALIAVAPAVVPANITVF

SEQ ID NO: 1081 - protein, 22 aa, Artificial Sequence
  Amino acid Sequence of aMTD605 5'-primer
GFHMVIAAVLAPVAVPANITVF

SEQ ID NO: 1082 - protein, 22 aa, Artificial Sequence
  Amino acid Sequence of aMTD606 5'-primer
GFHMAAAIAAIPIIIPANITVF

SEQ ID NO: 1083 - protein, 22 aa, Artificial Sequence
  Amino acid Sequence of aMTD622 5'-primer
GFHMALIVLAAPVAVPANITVF

SEQ ID NO: 1084 - protein, 22 aa, Artificial Sequence
  Amino acid Sequence of aMTD623 5'-primer
GFHMVAAAIALPAIVPANITVF

SEQ ID NO: 1085 - protein, 22 aa, Artificial Sequence
  Amino acid Sequence of aMTD625 5'-primer
GFHMILAAAAAPLIVPANITVF

SEQ ID NO: 1086 - protein, 22 aa, Artificial Sequence
  Amino acid Sequence of aMTD635 5'-primer
GFHMGSTGGSQQNNQYANITVF

SEQ ID NO: 1087 - protein, 22 aa, Artificial Sequence
  Amino acid Sequence of aMTD643 5'-primer
GFHMLALVLAAPAIVPANITVF

SEQ ID NO: 1088 - protein, 22 aa, Artificial Sequence
  Amino acid Sequence of aMTD645 5'-primer
GFHMALAVVALPAIVPANITVF

SEQ ID NO: 1089 - protein, 22 aa, Artificial Sequence
  Amino acid Sequence of aMTD661 5'-primer
GFHMAAILAPIVAALPANITVF

SEQ ID NO: 1090 - protein, 22 aa, Artificial Sequence
  Amino acid Sequence of aMTD664 5'-primer
GFHMILIAIAIPAAAPANITVF

SEQ ID NO: 1091 - protein, 22 aa, Artificial Sequence
  Amino acid Sequence of aMTD665 5'-primer
GFHMLAIVLAAPVAVPANITVF

SEQ ID NO: 1092 - protein, 22 aa, Artificial Sequence
  Amino acid Sequence of aMTD666 5'-primer
GFHMAAIAIIAPAIVPANITVF

SEQ ID NO: 1093 - protein, 22 aa, Artificial Sequence
  Amino acid Sequence of aMTD667 5'-primer
GFHMLAVAIVAPALVPANITVF

SEQ ID NO: 1094 - protein, 22 aa, Artificial Sequence
  Amino acid Sequence of aMTD676 5'-primer
GFHMVPLLVPVPVVVPANITVF

SEQ ID NO: 1095 - protein, 22 aa, Artificial Sequence
  Amino acid Sequence of aMTD683 5'-primer
GFHMLAIVLAAPAVLPANITVF

SEQ ID NO: 1096 - protein, 22 aa, Artificial Sequence
  Amino acid Sequence of aMTD684 5'-primer
GFHMAAIVLALPAVLPANITVF

SEQ ID NO: 1097 - protein, 22 aa, Artificial Sequence
  Amino acid Sequence of aMTD685 5'-primer
GFHMALLVAVLPAALPANITVF

SEQ ID NO: 1098 - protein, 22 aa, Artificial Sequence
  Amino acid Sequence of aMTD686 5'-primer
GFHMAALVAVLPVALPANITVF

SEQ ID NO: 1099 - protein, 22 aa, Artificial Sequence
  Amino acid Sequence of aMTD687 5'-primer
GFHMAILAVALPLLAPANITVF

SEQ ID NO: 1100 - protein, 22 aa, Artificial Sequence
  Amino acid Sequence of aMTD692 5'-primer
GFHMPAPLPPVVILAVANITVF

SEQ ID NO: 1101 - protein, 22 aa, Artificial Sequence
  Amino acid Sequence of aMTD693 5'-primer
GFHMAAPVLPVAVPIVANITVF

SEQ ID NO: 1102 - protein, 22 aa, Artificial Sequence
  Amino acid Sequence of aMTD700 5'-primer
GFHMGTSNTCQSNQNSANITVF

SEQ ID NO: 1103 - protein, 22 aa, Artificial Sequence
  Amino acid Sequence of aMTD703 5'-primer
GFHMIVAVALVPALAPANITVF

SEQ ID NO: 1104 - protein, 22 aa, Artificial Sequence
  Amino acid Sequence of aMTD705 5'-primer
GFHMIVAVALLPALAPANITVF

SEQ ID NO: 1105 - protein, 22 aa, Artificial Sequence
  Amino acid Sequence of aMTD706 5'-primer
GFHMIVAVALLPAVAPANITVF

SEQ ID NO: 1106 - protein, 22 aa, Artificial Sequence
  Amino acid Sequence of aMTD707 5'-primer
GFHMIVALAVLPAVAPANITVF

SEQ ID NO: 1107 - protein, 22 aa, Artificial Sequence
  Amino acid Sequence of aMTD724 5'-primer
GFHMVAVLAVLPALAPANITVF

SEQ ID NO: 1108 - protein, 22 aa, Artificial Sequence
  Amino acid Sequence of aMTD725 5'-primer
GFHMIAVLAVAPAVLPANITVF

SEQ ID NO: 1109 - protein, 22 aa, Artificial Sequence
  Amino acid Sequence of aMTD726 5'-primer
GFHMLAVAIIAPAVAPANITVF

SEQ ID NO: 1110 - protein, 22 aa, Artificial Sequence
  Amino acid Sequence of aMTD727 5'-primer
GFHMVALAIALPAVLPANITVF

SEQ ID NO: 1111 - protein, 22 aa, Artificial Sequence
  Amino acid Sequence of aMTD743 5'-primer
GFHMAIAIALVPVALPANITVF

SEQ ID NO: 1112 - protein, 22 aa, Artificial Sequence
  Amino acid Sequence of aMTD744 5'-primer
GFHMAAVVIVAPVALPANITVF

SEQ ID NO: 1113 - protein, 22 aa, Artificial Sequence
  Amino acid Sequence of aMTD745 5'-primer
GFHMAAILAIVAPLAPANITVF

SEQ ID NO: 1114 - protein, 22 aa, Artificial Sequence
  Amino acid Sequence of aMTD746 5'-primer
GFHMVAIIVVAPALAPANITVF

SEQ ID NO: 1115 - protein, 22 aa, Artificial Sequence
  Amino acid Sequence of aMTD747 5'-primer
GFHMVALLAIAPALAPANITVF

SEQ ID NO: 1116 - protein, 22 aa, Artificial Sequence
  Amino acid Sequence of aMTD750 5'-primer
GFHMLAIAAIAPLAIPANITVF

SEQ ID NO: 1117 - protein, 22 aa, Artificial Sequence
  Amino acid Sequence of aMTD763 5'-primer
GFHMVAVLIAVPALAPANITVF

SEQ ID NO: 1118 - protein, 22 aa, Artificial Sequence
  Amino acid Sequence of aMTD764 5'-primer
GFHMAVALAVLPAVVPANITVF

SEQ ID NO: 1119 - protein, 22 aa, Artificial Sequence
  Amino acid Sequence of aMTD765 5'-primer
GFHMAVALAVVPAVLPANITVF

SEQ ID NO: 1120 - protein, 22 aa, Artificial Sequence
  Amino acid Sequence of aMTD766 5'-primer
GFHMIVVIAVAPAVAPANITVF

SEQ ID NO: 1121 - protein, 22 aa, Artificial Sequence
  Amino acid Sequence of aMTD767 5'-primer
GFHMIVVAAVVPALAPANITVF

SEQ ID NO: 1122 - protein, 22 aa, Artificial Sequence
  Amino acid Sequence of aMTD772 5'-primer
GFHMLPVAPVIPIIVPANITVF

SEQ ID NO: 1123 - protein, 22 aa, Artificial Sequence
  Amino acid Sequence of aMTD783 5'-primer
GFHMIVALVPAVAIAPANITVF

SEQ ID NO: 1124 - protein, 22 aa, Artificial Sequence
  Amino acid Sequence of aMTD784 5'-primer
GFHMVAALPAVALVVPANITVF

SEQ ID NO: 1125 - protein, 22 aa, Artificial Sequence
  Amino acid Sequence of aMTD786 5'-primer
GFHMLVAIAPLAVLAPANITVF

SEQ ID NO: 1126 - protein, 22 aa, Artificial Sequence
  Amino acid Sequence of aMTD787 5'-primer
GFHMAVALVPVIVAAPANITVF

SEQ ID NO: 1127 - protein, 22 aa, Artificial Sequence
  Amino acid Sequence of aMTD788 5'-primer
GFHMAIAVAIAPVALPANITVF

SEQ ID NO: 1128 - protein, 22 aa, Artificial Sequence
  Amino acid Sequence of aMTD803 5'-primer
GFHMAIALAVPVLALPANITVF

SEQ ID NO: 1129 - protein, 22 aa, Artificial Sequence
  Amino acid Sequence of aMTD805 5'-primer
GFHMLVLIAAAPIALPANITVF

SEQ ID NO: 1130 - protein, 22 aa, Artificial Sequence
  Amino acid Sequence of aMTD806 5'-primer
GFHMLVALAVPAAVLPANITVF

SEQ ID NO: 1131 - protein, 22 aa, Artificial Sequence
  Amino acid Sequence of aMTD807 5'-primer
GFHMAVALAVPALVLPANITVF

SEQ ID NO: 1132 - protein, 22 aa, Artificial Sequence
  Amino acid Sequence of aMTD808 5'-primer
GFHMLVVLAAAPLAVPANITVF

SEQ ID NO: 1133 - protein, 22 aa, Artificial Sequence
  Amino acid Sequence of aMTD809 5'-primer
GFHMLIVLAAPALAAPANITVF

SEQ ID NO: 1134 - protein, 22 aa, Artificial Sequence
  Amino acid Sequence of aMTD810 5'-primer
GFHMVIVLAAPALAAPANITVF

SEQ ID NO: 1135 - protein, 22 aa, Artificial Sequence
  Amino acid Sequence of aMTD811 5'-primer
GFHMAVVLAVPALAVPANITVF

SEQ ID NO: 1136 - protein, 22 aa, Artificial Sequence
  Amino acid Sequence of aMTD824 5'-primer
GFHMLIIVAAAPAVAPANITVF

SEQ ID NO: 1137 - protein, 22 aa, Artificial Sequence
  Amino acid Sequence of aMTD825 5'-primer
GFHMIVAVIVAPAVAPANITVF

SEQ ID NO: 1138 - protein, 22 aa, Artificial Sequence
  Amino acid Sequence of aMTD826 5'-primer
GFHMLVALAAPIIAVPANITVF

SEQ ID NO: 1139 - protein, 22 aa, Artificial Sequence
  Amino acid Sequence of aMTD827 5'-primer
GFHMIAAVLAAPALVPANITVF

SEQ ID NO: 1140 - protein, 22 aa, Artificial Sequence
  Amino acid Sequence of aMTD828 5'-primer
GFHMIALLAAPIIAVPANITVF

SEQ ID NO: 1141 - protein, 22 aa, Artificial Sequence
  Amino acid Sequence of aMTD829 5'-primer
GFHMAALALVAPVIVPANITVF

SEQ ID NO: 1142 - protein, 22 aa, Artificial Sequence
  Amino acid Sequence of aMTD830 5'-primer
GFHMIALVAAPVALVPANITVF

SEQ ID NO: 1143 - protein, 22 aa, Artificial Sequence
  Amino acid Sequence of aMTD831 5'-primer
GFHMIIVAVAPAAIVPANITVF

SEQ ID NO: 1144 - protein, 22 aa, Artificial Sequence
  Amino acid Sequence of aMTD832 5'-primer
GFHMAVAAIVPVIVAPANITVF

SEQ ID NO: 1145 - protein, 22 aa, Artificial Sequence
  Amino acid Sequence of aMTD843 5'-primer
GFHMAVLVLVAPAAAPANITVF

SEQ ID NO: 1146 - protein, 22 aa, Artificial Sequence
  Amino acid Sequence of aMTD844 5'-primer
GFHMVVALLAPLIAAPANITVF

SEQ ID NO: 1147 - protein, 22 aa, Artificial Sequence
  Amino acid Sequence of aMTD845 5'-primer
GFHMAAVVIAPLLAVPANITVF

SEQ ID NO: 1148 - protein, 22 aa, Artificial Sequence
  Amino acid Sequence of aMTD846 5'-primer
GFHMIAVAVAAPLLVPANITVF

SEQ ID NO: 1149 - protein, 22 aa, Artificial Sequence
  Amino acid Sequence of aMTD847 5'-primer
GFHMLVAIVVLPAVAPANITVF

SEQ ID NO: 1150 - protein, 22 aa, Artificial Sequence
  Amino acid Sequence of aMTD848 5'-primer
GFHMAVAIVVLPAVAPANITVF

SEQ ID NO: 1151 - protein, 22 aa, Artificial Sequence
  Amino acid Sequence of aMTD849 5'-primer
GFHMAVILLAPLIAAPANITVF

SEQ ID NO: 1152 - protein, 22 aa, Artificial Sequence
  Amino acid Sequence of aMTD850 5'-primer
GFHMLVIALAAPVALPANITVF

SEQ ID NO: 1153 - protein, 22 aa, Artificial Sequence
  Amino acid Sequence of aMTD851 5'-primer
GFHMVLAVVLPAVALPANITVF

SEQ ID NO: 1154 - protein, 22 aa, Artificial Sequence
  Amino acid Sequence of aMTD852 5'-primer
GFHMVLAVAAPAVLLPANITVF

SEQ ID NO: 1155 - protein, 22 aa, Artificial Sequence
  Amino acid Sequence of aMTD863 5'-primer
GFHMAAVVLLPIIAAPANITVF

SEQ ID NO: 1156 - protein, 22 aa, Artificial Sequence
  Amino acid Sequence of aMTD864 5'-primer
GFHMALLVIAPAIAVPANITVF

SEQ ID NO: 1157 - protein, 22 aa, Artificial Sequence
  Amino acid Sequence of aMTD865 5'-primer
GFHMAVLVIAVPAIAPANITVF

SEQ ID NO: 1158 - protein, 22 aa, Artificial Sequence
  Amino acid Sequence of aMTD867 5'-primer
GFHMALLVVIAPLAAPANITVF

SEQ ID NO: 1159 - protein, 22 aa, Artificial Sequence
  Amino acid Sequence of aMTD868 5'-primer
GFHMVLVAAILPAAIPANITVF

SEQ ID NO: 1160 - protein, 22 aa, Artificial Sequence
  Amino acid Sequence of aMTD870 5'-primer
GFHMVLVAAVLPIAAPANITVF

SEQ ID NO: 1161 - protein, 22 aa, Artificial Sequence
  Amino acid Sequence of aMTD872 5'-primer
GFHMVLAAAVLPLVVPANITVF

SEQ ID NO: 1162 - protein, 22 aa, Artificial Sequence
  Amino acid Sequence of aMTD875 5'-primer
GFHMAIAIVVPAVAVPANITVF

SEQ ID NO: 1163 - protein, 22 aa, Artificial Sequence
  Amino acid Sequence of aMTD877 5'-primer
GFHMVAIIAVPAVVAPANITVF

SEQ ID NO: 1164 - protein, 22 aa, Artificial Sequence
  Amino acid Sequence of aMTD878 5'-primer
GFHMIVALVAPAAVVPANITVF

SEQ ID NO: 1165 - protein, 22 aa, Artificial Sequence
  Amino acid Sequence of aMTD879 5'-primer
GFHMAAIVLLPAVVVPANITVF

SEQ ID NO: 1166 - protein, 22 aa, Artificial Sequence
  Amino acid Sequence of aMTD881 5'-primer
GFHMAALIVVPAVAVPANITVF

SEQ ID NO: 1167 - protein, 22 aa, Artificial Sequence
  Amino acid Sequence of aMTD882 5'-primer
GFHMAIALVVPAVAVPANITVF

SEQ ID NO: 1168 - protein, 22 aa, Artificial Sequence
  Amino acid Sequence of aMTD883 5'-primer
GFHMLAIVPAAIAALPANITVF

SEQ ID NO: 1169 - protein, 22 aa, Artificial Sequence
  Amino acid Sequence of aMTD884 5'-primer
GFHMVLIVPAAIAALPANITVF

SEQ ID NO: 1170 - protein, 22 aa, Artificial Sequence
  Amino acid Sequence of aMTD885 5'-primer
GFHMLVAIAPAVAVLPANITVF

SEQ ID NO: 1171 - protein, 22 aa, Artificial Sequence
  Amino acid Sequence of aMTD886 5'-primer
GFHMVLAVPAAIAALPANITVF

SEQ ID NO: 1172 - protein, 22 aa, Artificial Sequence
  Amino acid Sequence of aMTD887 5'-primer
GFHMVLAVAPAVAVLPANITVF

SEQ ID NO: 1173 - protein, 22 aa, Artificial Sequence
  Amino acid Sequence of aMTD888 5'-primer
GFHMILAVVAIPAAAPANITVF

SEQ ID NO: 1174 - protein, 22 aa, Artificial Sequence
  Amino acid Sequence of aMTD889 5'-primer
GFHMILVAAAPIAALPANITVF

SEQ ID NO: 1175 - protein, 22 aa, Artificial Sequence
  Amino acid Sequence of aMTD891 5'-primer
GFHMILAVAAIPAALPANITVF

SEQ ID NO: 1176 - protein, 22 aa, Artificial Sequence
  Amino acid Sequence of aMTD893 5'-primer
GFHMVIAIPAILAAAPANITVF

SEQ ID NO: 1177 - protein, 22 aa, Artificial Sequence
  Amino acid Sequence of aMTD895 5'-primer
GFHMAIIIVVPAIAAPANITVF

SEQ ID NO: 1178 - protein, 22 aa, Artificial Sequence
  Amino acid Sequence of aMTD896 5'-primer
GFHMAILIVVAPIAAPANITVF

SEQ ID NO: 1179 - protein, 22 aa, Artificial Sequence
  Amino acid Sequence of aMTD897 5'-primer
GFHMAVIVPVAIIAAPANITVF

SEQ ID NO: 1180 - protein, 22 aa, Artificial Sequence
  Amino acid Sequence of aMTD899 5'-primer
GFHMAVVIALPAVVAPANITVF

SEQ ID NO: 1181 - protein, 22 aa, Artificial Sequence
  Amino acid Sequence of aMTD900 5'-primer
GFHMALVAVIAPVVAPANITVF

SEQ ID NO: 1182 - protein, 22 aa, Artificial Sequence
  Amino acid Sequence of aMTD901 5'-primer
GFHMALVAVLPAVAVPANITVF

SEQ ID NO: 1183 - protein, 22 aa, Artificial Sequence
  Amino acid Sequence of aMTD902 5'-primer
GFHMALVAPLLAVAVPANITVF

SEQ ID NO: 1184 - protein, 22 aa, Artificial Sequence
  Amino acid Sequence of aMTD904 5'-primer
GFHMAVLAVVAPVVAPANITVF

SEQ ID NO: 1185 - protein, 22 aa, Artificial Sequence
  Amino acid Sequence of aMTD905 5'-primer
GFHMAVIAVAPLVVAPANITVF

SEQ ID NO: 1186 - protein, 22 aa, Artificial Sequence
  Amino acid Sequence of aMTD906 5'-primer
GFHMAVIALAPVVVAPANITVF

SEQ ID NO: 1187 - protein, 22 aa, Artificial Sequence
  Amino acid Sequence of aMTD907 5'-primer
GFHMVAIALAPVVVAPANITVF

SEQ ID NO: 1188 - protein, 22 aa, Artificial Sequence
  Amino acid Sequence of aMTD908 5'-primer
GFHMVALALAPVVVAPANITVF

SEQ ID NO: 1189 - protein, 22 aa, Artificial Sequence
  Amino acid Sequence of aMTD910 5'-primer
GFHMVAALLPAVVVAPANITVF

SEQ ID NO: 1190 - protein, 22 aa, Artificial Sequence
  Amino acid Sequence of aMTD911 5'-primer
GFHMVALALPAVVVAPANITVF

SEQ ID NO: 1191 - protein, 22 aa, Artificial Sequence
  Amino acid Sequence of aMTD912 5'-primer
GFHMVALLAPAVVVAPANITVF

SEQ ID NO: 1192 - protein, 22 aa, Artificial Sequence
  Amino acid Sequence of aMTD921 5'-primer
GFHMIWWFVVLPLVVPANITVF

SEQ ID NO: 1193 - protein, 22 aa, Artificial Sequence
  Amino acid Sequence of aMTD922 5'-primer
GFHMWYVIFVLPLVVPANITVF

SEQ ID NO: 1194 - protein, 22 aa, Artificial Sequence
  Amino acid Sequence of aMTD931 5'-primer
GFHMAVLIAPAILAAAANITVF

SEQ ID NO: 1195 - protein, 22 aa, Artificial Sequence
  Amino acid Sequence of aMTD934 5'-primer
GFHMLILAPAAVVAAAANITVF

SEQ ID NO: 1196 - protein, 22 aa, Artificial Sequence
  Amino acid Sequence of aMTD935 5'-primer
GFHMALLILPAAAVAAANITVF

SEQ ID NO: 1197 - protein, 22 aa, Artificial Sequence
  Amino acid Sequence of aMTD936 5'-primer
GFHMALLILAAAVAAPANITVF

SEQ ID NO: 1198 - protein, 22 aa, Artificial Sequence
  Amino acid Sequence of aMTD937 5'-primer
GFHMVPVLVPLPVPVVANITVF

SEQ ID NO: 1199 - protein, 22 aa, Artificial Sequence
  Amino acid Sequence of aMTD938 5'-primer
GFHMVPVLLPVVVPVPANITVF

SEQ ID NO: 1200 - protein, 22 aa, Artificial Sequence
  Amino acid Sequence of aMTD947 5'-primer
GFHMCYYNQQSNNNNQANITVF

SEQ ID NO: 1201 - protein, 22 aa, Artificial Sequence
  Amino acid Sequence of aMTD949 5'-primer
GFHMSGNSCQQCGNSSANITVF

SEQ ID NO: 1202 - protein, 13 aa, Artificial Sequence
  Amino acid Sequence of aMTD 3'-primer
RVDLPRLHRHGDD

SEQ ID NO: 1203 - protein, 184 aa, Artificial Sequence
  Amino acid Sequence of SDA
MANITVFYNEDFQGKQVDLPPGNYTRAQLAALGIENNTISSVKVPPGVKAILYQNDGFAGDQIEVVANAEELGPLNNNVSSIRVISVPVQPRMANITVFYNEDFQGKQVDLPPGNYTRAQLAALGIENNTISSVKVPPGVKAILYQNDGFAGDQIEVVANAEELGPLNNNVSSIRVISVPVQPR

SEQ ID NO: 1204 - protein, 99 aa, Artificial Sequence
  Amino acid Sequence of SDB
MAEQSDKDVKYYTLEEIQKHKDSKSTWVILHHKVYDLTKFLEEHPGGEEVLGEQAGGDATENFEDVGHSTDARELSKTYIIGELHPDDRSKIAKPSETL

SEQ ID NO: 1205 - protein, 109 aa, Artificial Sequence
  Amino acid Sequence of SDC
MSDKIIHLTDDSFDTDVLKADGAILVDFWAEWCGPCKMIAPILDEIADEYQGKLTVAKLNIDQNPGTAPKYGIRGIPTLLLFKNGEVAATKVGALSKGQLKEFLDANLA

SEQ ID NO: 1206 - protein, 208 aa, Artificial Sequence
  Amino acid Sequence of SDD
MKKIWLALAGLVLAFSASAAQYEDGKQYTTLEKPVAGAPQVLEFFSFFCPHCYQFEEVLHISDNVKKKLPEGVKMTKYHVNFMGGDLGKDLTQAWAVAMALGVEDKVTVPLFEGVQKTQTIRSASDIRDVFINAGIKGEEYDAAWNSFVVKSLVAQQEKAAADVQLRGVPAMFVNGKYQLNPQGMDTSNMDVFVQQYADTVKYLSEKK

SEQ ID NO: 1207 - protein, 100 aa, Artificial Sequence
  Amino acid Sequence of SDE
GSLQDSEVNQEAKPEVKPEVKPETHINLKVSDGSSEIFFKIKKTTPLRRLMEAFAKRQGKEMDSLTFLYDGIEIQADQTPEDLDMEDNDIIEAHREQIGG

SEQ ID NO: 1208 - protein, 297 aa, Artificial Sequence
  Amino acid Sequence of SDF
GSEIGTGFPFDPHYVEVLGERMHYVDVGPRDGTPVLFLHGNPTSSYVWRNIIPHVAPTHRCIAPDLIGMGKSDKPDLGYFFDDHVRFMDAFIEALGLEEVVLVIHDWGSALGFHWAKRNPERVKGIAFMEFIRPIPTWDEWPEFARETFQAFRTTDVGRKLIIDQNVFIEGTLPMGVVRPLTEVEMDHYREPFLNPVDREPLWRFPNELPIAGEPANIVALVEEYMDWLHQSPVPKLLFWGTPGVLIPPAEAARLAKSLPNCKAVDIGPGLNLLQEDNPDLIGSEIARWLSTLEISG

SEQ ID NO: 1209 - protein, 99 aa, Artificial Sequence
  Amino acid Sequence of SDB for deimunization
MAEQSDKDVKYYTLEEIQKHKDSKSTWLILHHKVYDLTKFLEEHPGGEEVLGEQAGGDATENFEDVGHSTDARELSKTYIIGELHPDDRSKIAKPSETL

SEQ ID NO: 1210 - DNA, 552 bp, Artificial Sequence
  Polynucleotide Sequence of SDA
atggcaaatattaccgttttctataacgaagacttccagggtaagcaggtcgatctgccgcctggcaactatacccgcgcccagttggcggcgctgggcatcgagaataataccatcagctcggtgaaggtgccgcctggcgtgaaggctatcctgtaccagaacgatggtttcgccggcgaccagatcgaagtggtggccaatgccgaggagttgggcccgctgaataataacgtctccagcatccgcgtcatctccgtgcccgtgcagccgcgcatggcaaatattaccgttttctataacgaagacttccagggtaagcaggtcgatctgccgcctggcaactatacccgcgcccagttggcggcgctgggcatcgagaataataccatcagctcggtgaaggtgccgcctggcgtgaaggctatcctctaccagaacgatggtttcgccggcgaccagatcgaagtggtggccaatgccgaggagctgggtccgctgaataataacgtctccagcatccgcgtcatctccgtgccggtgcagccgagg

SEQ ID NO: 1211 - DNA, 297 bp, Artificial Sequence
  Polynucleotide Sequence of SDB
atggcagaacaaagcgacaaggatgtgaagtactacactctggaggagattcagaagcacaaagacagcaagagcacctgggtgatcctacatcataaggtgtacgatctgaccaagtttctcgaagagcatcctggtggggaagaagtcctgggcgagcaagctgggggtgatgctactgagaactttgaggacgtcgggcactctacggatgcacgagaactgtccaaaacatacatcatcggggagctccatccagatgacagatcaaagatagccaagccttcggaaaccctt

SEQ ID NO: 1212 - DNA, 327 bp, Artificial Sequence
  Polynucleotide Sequence of SDC
atgagcgataaaattattcacctgactgacgacagttttgacacggatgtactcaaagcggacggggcgatcctcgtcgatttctgggcagagtggtgcggtccgtgcaaaatgatcgccccgattctggatgaaatcgctgacgaatatcagggcaaactgaccgttgcaaaactgaacatcgatcaaaaccctggcactgcgccgaaatatggcatccgtggtatcccgactctgctgctgttcaaaaacggtgaagtggcggcaaccaaagtgggtgcactgtctaaaggtcagttgaaagagttcctcgacgctaacctggcc

SEQ ID NO: 1213 - DNA, 624 bp, Artificial Sequence
  Polynucleotide Sequence of SDD
atgaaaaagatttggctggcgctggctggtttagttttagcgtttagcgcatcggcggcgcagtatgaagatggtaaacagtacactaccctggaaaaaccggtagctggcgcgccgcaagtgctggagtttttctctttcttctgcccgcactgctatcagtttgaagaagttctgcatatttctgataatgtgaagaaaaaactgccggaaggcgtgaagatgactaaataccacgtcaacttcatgggtggtgacctgggcaaagatctgactcaggcatgggctgtggcgatggcgctgggcgtggaagacaaagtgactgttccgctgtttgaaggcgtacagaaaacccagaccattcgttctgcttctgatatccgcgatgtatttatcaacgcaggtattaaaggtgaagagtacgacgcggcgtggaacagcttcgtggtgaaatctctggtcgctcagcaggaaaaagctgcagctgacgtgcaattgcgtggcgttccggcgatgtttgttaacggtaaatatcagctgaatccgcagggtatggataccagcaatatggatgtttttgttcagcagtatgctgatacagtgaaatatctgtccgagaaaaaa

SEQ ID NO: 1214 - DNA, 300 bp, Artificial Sequence
  Polynucleotide Sequence of SDE
gggtccctgcaggactcagaagtcaatcaagaagctaagccagaggtcaagccagaagtcaagcctgagactcacatcaatttaaaggtgtccgatggatcttcagagatcttcttcaagatcaaaaagaccactcctttaagaaggctgatggaagcgttcgctaaaagacagggtaaggaaatggactccttaacgttcttgtacgacggtattgaaattcaagctgatcagacccctgaagatttggacatggaggataacgatattattgaggctcaccgcgaacagattggaggt

SEQ ID NO: 1215 - DNA, 891 bp, Artificial Sequence
  Polynucleotide Sequence of SDF
ggatccgaaatcggtactggctttccattcgacccccattatgtggaagtcctgggcgagcgcatgcactacgtcgatgttggtccgcgcgatggcacccctgtgctgttcctgcacggtaacccgacctcctcctacgtgtggcgcaacatcatcccgcatgttgcaccgacccatcgctgcattgctccagacctgatcggtatgggcaaatccgacaaaccagacctgggttatttcttcgacgaccacgtccgcttcatggatgccttcatcgaagccctgggtctggaagaggtcgtcctggtcattcacgactggggctccgctctgggtttccactgggccaagcgcaatccagagcgcgtcaaaggtattgcatttatggagttcatccgccctatcccgacctgggacgaatggccagaatttgcccgcgagaccttccaggccttccgcaccaccgacgtcggccgcaagctgatcatcgatcagaacgtttttatcgagggtacgctgccgatgggtgtcgtccgcccgctgactgaagtcgagatggaccattaccgcgagccgttcctgaatcctgttgaccgcgagccactgtggcgcttcccaaacgagctgccaatcgccggtgagccagcgaacatcgtcgcgctggtcgaagaatacatggactggctgcaccagtcccctgtcccgaagctgctgttctggggcaccccaggcgttctgatcccaccggccgaagccgctcgcctggccaaaagcctgcctaactgcaaggctgtggacatcggcccgggtctgaatctgctgcaagaagacaacccggacctgatcggcagcgagatcgcgcgctggctgtctactctggagatttccggt

SEQ ID NO: 1216 - DNA, 297 bp, Artificial Sequence
  Polynucleotide Sequence of SDB for deimunization
atggcagaacaaagcgacaaggatgtgaagtactacactctggaggagattcagaagcacaaagacagcaagagcacctggctgatcctacatcataaggtgtacgatctgaccaagtttctcgaagagcatcctggtggggaagaagtcctgggcgagcaagctgggggtgatgctactgagaactttgaggacgtcgggcactctacggatgcacgagaactgtccaaaacatacatcatcggggagctccatccagatgacagatcaaagatagccaagccttcggaaaccctt

SEQ ID NO: 1217 - protein, 19 aa, Artificial Sequence
  Amino acid Sequence of Histidine Tag
MGSSHHHHHHSSGLVPRGS

SEQ ID NO: 1218 - DNA, 57 bp, Artificial Sequence
  Polynucleotide Sequence of Histidine Tag
atgggcagcagccatcatcatcatcatcacagcagcggcctggtgccgcgcggcagc

SEQ ID NO: 1219 - protein, 7 aa, Artificial Sequence
  Amino acid Sequence of NLS
PKKKRKV

SEQ ID NO: 1220 - DNA, 21 bp, Artificial Sequence
  Polynucleotide Sequence of NLS
ccgaaaaagaaacgtaaagtg

SEQ ID NO: 1221 - protein, 1368 aa, Artificial Sequence [sequence omitted]

SEQ ID NO: 1222 - DNA, 4104 bp, Artificial Sequence
  Polynucleotide Sequence of Cas9
atggacaaaaagtatagcattggcctggacattggcaccaacagcgtgggctgggcggttatcaccgatgagtacaaggttccgagcaagaaatttaaggtgctgggtaacaccgatcgtcacagcatcaagaaaaacctgattggtgcgctgctgtttgacagcggtgaaaccgcggaagcgacccgtctgaaacgtaccgcgcgtcgtcgttacacccgtcgtaagaaccgtatctgctacctgcaggagattttcagcaacgaaatggcgaaggtggacgatagcttctttcaccgtctggaggagagcttcctggttgaggaagataagaaacacgagcgtcacccgatctttggcaacattgtggacgaggttgcgtatcacgaaaaatacccgaccatctatcacctgcgtaagaaactggtggacagcaccgataaagcggacctgcgtctgatctatctggcgctggcgcacatgattaagttccgtggtcactttctgatcgaaggcgatctgaacccggacaacagcgatgtggacaaactgttcatccagctggttcaaacctacaaccagctgtttgaggaaaacccgattaacgcgagcggtgttgacgcgaaagcgatcctgagcgcgcgtctgagcaagagccgtcgtctggagaacctgatcgcgcaactgccgggtgaaaagaaaaacggtctgtttggcaacctgattgcgctgagcctgggcctgaccccgaacttcaagagcaactttgatctggcggaggacgcgaaactgcagctgagcaaggacacctatgacgatgacctggataacctgctggcgcaaatcggcgatcagtacgcggacctgttcctggcggcgaaaaacctgagcgacgcgatcctgctgagcgatattctgcgtgtgaacaccgagattaccaaagcgccgctgagcgcgagcatgatcaagcgttatgacgaacaccaccaagatctgaccctgctgaaggcgctggttcgtcagcaactgccggagaagtacaaggaaatcttctttgatcaaagcaagaacggttacgcgggctatattgacggtggcgcgagccaggaagagttctacaagtttatcaaaccgattctggagaagatggacggtaccgaggaactgctggtgaaactgaaccgtgaagacctgctgcgtaagcaacgtacctttgataacggtagcatcccgcaccagattcatctgggtgaactgcatgcgatcctgcgtcgtcaggaagacttctacccgtttctgaaagataaccgtgagaagatcgaaaaaattctgaccttccgtattccgtactatgttggtccgctggcgcgtggcaacagccgttttgcgtggatgacccgtaaaagcgaggaaaccatcaccccgtggaacttcgaggaagtggttgataagggtgcgagcgcgcagagcttcattgagcgtatgaccaactttgacaaaaacctgccgaacgaaaaagtgctgccgaagcacagcctgctgtacgagtatttcaccgtttataacgaactgaccaaggtgaaatacgttaccgagggtatgcgtaagccggcgttcctgagcggcgaacaaaagaaagcgatcgtggacctgctgtttaaaaccaaccgtaaggtgaccgttaagcagctgaaagaggactacttcaagaaaattgaatgcttcgatagcgtggagatcagcggtgttgaagaccgttttaacgcgagcctgggcacctaccacgatctgctgaagatcattaaggataaagacttcctggacaacgaggaaaacgaggatatcctggaagacattgtgctgaccctgaccctgtttgaggatcgtgaaatgatcgaggaacgtctgaaaacctatgcgcacctgttcgatgacaaggttatgaaacagctgaagcgtcgtcgttacaccggttggggccgtctgagccgtaagcttatcaacggtattcgtgacaaacaaagcggcaagaccatcctggactttctgaaaagcgatggtttcgcgaaccgtaactttatgcagctgattcacgatgacagcctgaccttcaaagaggatatccagaaggcgcaagttagcggtcaaggcgacagcctgcacgaacatattgcgaacctggcgggtagcccggcgatcaagaaaggcattctgcagaccgtgaaagtggttgacgagctggtgaaagttatgggtcgtcacaagccggaaaacatcgttattgagatggcgcgtgaaaaccagaccacccaaaaaggccagaagaacagccgtgagcgtatgaaacgtatcgaggaaggtattaaggaactgggcagccagatcctgaaagagcacccggtggaaaacacccagctgcaaaacgagaagctgtatctgtactatctgcaaaacggtcgtgatatgtacgttgaccaggaactggatattaaccgtctgagcgattacgacgtggatcacatcgttccgcagagcttcctgaaagatgacagcattgacaacaaggtgctgacccgtagcgacaaaaaccgtggcaagagcgataacgttccgagcgaggaagtggttaagaaaatgaagaactactggcgtcaactgctgaacgcgaaactgatcacccagcgtaagtttgataacctgaccaaagcggagcgtggtggcctgagcgaactggacaaagcgggtttcattaagcgtcaactggtggagacccgtcagatcaccaaacacgttgcgcagattctggatagccgtatgaacaccaagtacgatgagaacgacaaactgatccgtgaagtgaaggttattaccctgaagagcaaactggttagcgacttccgtaaggatttccaattctacaaggttcgtgaaatcaacaactatcaccacgcgcacgacgcgtacctgaacgcggtggttggtaccgcgctgattaagaaatacccgaaactggagagcgaattcgtttacggcgactataaggtgtacgatgttcgtaaaatgatcgcgaagagcgagcaggaaattggtaaagcgaccgcgaagtatttcttttacagcaacatcatgaacttctttaagaccgagatcaccctggcgaacggtgaaatccgtaagcgtccgctgattgagaccaacggcgagaccggcgaaatcgtgtgggacaaaggccgtgattttgcgaccgtgcgtaaggttctgagcatgccgcaagtgaacattgttaagaaaaccgaggttcagaccggtggcttcagcaaggaaagcattctgccgaaacgtaacagcgataagctgatcgcgcgtaagaaagactgggacccgaagaagtatggtggcttcgacagcccgaccgtggcgtacagcgttctggtggttgcgaaggtggagaagggtaaaagcaagaaactgaaaagcgttaaggaactgctgggcatcaccattatggagcgtagcagcttcgagaagaacccgatcgattttctggaggcgaaaggttataaggaagtgaagaaagacctgatcattaaactgccgaagtacagcctgtttgagctggaaaacggccgtaaacgtatgctggcgagcgcgggcgagctgcagaaaggcaacgaactggcgctgccgagcaagtacgtgaacttcctgtatctggcgagccactacgagaagctgaaaggtagcccggaggataacgaacagaaacaactgtttgttgagcaacacaagcactatctggacgagatcattgaacagattagcgaattcagcaaacgtgtgatcctggcggacgcgaacctggataaggttctgagcgcgtacaacaaacaccgtgataagccgatccgtgagcaggcggaaaacatcattcacctgttcaccctgaccaacctgggtgcgccggcggcgttcaagtattttgacaccaccatcgatcgtaaacgttacaccagcaccaaagaggtgctggacgcgaccctgattcaccaaagcattaccggcctgtatgaaacccgtattgacctgagccaactgggcggcgat

SEQ ID NO: 1223 - DNA, 36 bp, Artificial Sequence
  polynucleotide Sequence of HC9 5'-primer
cccaagcttatcaacggtattcgtgacaaacaaagc

SEQ ID NO: 1224 - DNA, 133 bp, Artificial Sequence
  polynucleotide Sequence of HNM563C9 or HNM563C9SB 5'-primer
cccaagcttatcaacggtattcgtgacaaacaaagcggaattccatatgcccaagaagaagaggaaggtggcgctggcggtgattgtggtgccggcgctggcgccgatggacaaaaagtatagcattggcctg

SEQ ID NO: 1225 - DNA, 39 bp, Artificial Sequence
  polynucleotide Sequence of HNM563C9SB 5'-primer
cccggatccatggcagaacaaagcgacaaggatgtgaag

SEQ ID NO: 1226 - DNA, 36 bp, Artificial Sequence
  polynucleotide Sequence of HC9 3'-primer
cccaagcttacggctcagacggccccaaccggtgta

SEQ ID NO: 1227 - DNA, 36 bp, Artificial Sequence
  polynucleotide Sequence of HNM563C9 3'-primer
cgcggattcatcgccgcccagttggctcaggtcaat

SEQ ID NO: 1228 - DNA, 39 bp, Artificial Sequence
  polynucleotide Sequence of HNM563C9SB 3'-primer
cgcggattcttaatcgccgcccagttggctcaggtcaat

SEQ ID NO: 1229 - DNA, 39 bp, Artificial Sequence
  polynucleotide Sequence of HNM563C9SB 3'-primer
cgcgtcgacttaaagggtttccgaaggcttggctatctt

SEQ ID NO: 1230 - protein, 1509 aa, Artificial Sequence
  Amino acid Sequence of of HNM563C9SB
MGSSHHHHHHSSGLVPRGSHMPKKKRKVALAVIVVPALAPMDKKYSIGLDIGTNSVGWAVITDEYKVPSKKFKVLGNTDRHSIKKNLIGALLFDSGETAEATRLKRTARRRYTRRKNRICYLQEIFSNEMAKVDDSFFHRLEESFLVEEDKKHERHPIFGNIVDEVAYHEKYPTIYHLRKKLVDSTDKADLRLIYLALAHMIKFRGHFLIEGDLNPDNSDVDKLFIQLVQTYNQLFEENPINASGVDAKAILSARLSKSRRLENLIAQLPGEKKNGLFGNLIALSLGLTPNFKSNFDLAEDAKLQLSKDTYDDDLDNLLAQIGDQYADLFLAAKNLSDAILLSDILRVNTEITKAPLSASMIKRYDEHHQDLTLLKALVRQQLPEKYKEIFFDQSKNGYAGYIDGGASQEEFYKFIKPILEKMDGTEELLVKLNREDLLRKQRTFDNGSIPHQIHLGELHAILRRQEDFYPFLKDNREKIEKILTFRIPYYVGPLARGNSRFAWMTRKSEETITPWNFEEVVDKGASAQSFIERMTNFDKNLPNEKVLPKHSLLYEYFTVYNELTKVKYVTEGMRKPAFLSGEQKKAIVDLLFKTNRKVTVKQLKEDYFKKIECFDSVEISGVEDRFNASLGTYHDLLKIIKDKDFLDNEENEDILEDIVLTLTLFEDREMIEERLKTYAHLFDDKVMKQLKRRRYTGWGRLSRKLINGIRDKQSGKTILDFLKSDGFANRNFMQLIHDDSLTFKEDIQKAQVSGQGDSLHEHIANLAGSPAIKKGILQTVKVVDELVKVMGRHKPENIVIEMARENQTTQKGQKNSRERMKRIEEGIKELGSQILKEHPVENTQLQNEKLYLYYLQNGRDMYVDQELDINRLSDYDVDHIVPQSFLKDDSIDNKVLTRSDKNRGKSDNVPSEEVVKKMKNYWRQLLNAKLITQRKFDNLTKAERGGLSELDKAGFIKRQLVETRQITKHVAQILDSRMNTKYDENDKLIREVKVITLKSKLVSDFRKDFQFYKVREINNYHHAHDAYLNAVVGTALIKKYPKLESEFVYGDYKVYDVRKMIAKSEQEIGKATAKYFFYSNIMNFFKTEITLANGEIRKRPLIETNGETGEIVWDKGRDFATVRKVLSMPQVNIVKKTEVQTGGFSKESILPKRNSDKLIARKKDWDPKKYGGFDSPTVAYSVLVVAKVEKGKSKKLKSVKELLGITIMERSSFEKNPIDFLEAKGYKEVKKDLIIKLPKYSLFELENGRKRMLASAGELQKGNELALPSKYVNFLYLASHYEKLKGSPEDNEQKQLFVEQHKHYLDEIIEQISEFSKRVILADANLDKVLSAYNKHRDKPIREQAENIIHLFTLTNLGAPAAFKYFDTTIDRKRYTSTKEVLDATLIHQSITGLYETRIDLSQLGGDGSMAEQSDKDVKYYTLEEIQKHKDSKSTWVILHHKVYDLTKFLEEHPGGEEVLGEQAGGDATENFEDVGHSTDARELSKTYIIGELHPDDRSKIAKPSETL

SEQ ID NO: 1231 - DNA, 4527 bp, Artificial Sequence
  Polynucleotide Sequence of HNM563C9SB
atgggcagcagccatcatcatcatcatcacagcagcggcctggtgccgcgcggcagccatatgcccaagaagaagaggaaggtggcgctggcggtgattgtggtgccggcgctggcgccgatggacaaaaagtatagcattggcctggacattggcaccaacagcgtgggctgggcggttatcaccgatgagtacaaggttccgagcaagaaatttaaggtgctgggtaacaccgatcgtcacagcatcaagaaaaacctgattggtgcgctgctgtttgacagcggtgaaaccgcggaagcgacccgtctgaaacgtaccgcgcgtcgtcgttacacccgtcgtaagaaccgtatctgctacctgcaggagattttcagcaacgaaatggcgaaggtggacgatagcttctttcaccgtctggaggagagcttcctggttgaggaagataagaaacacgagcgtcacccgatctttggcaacattgtggacgaggttgcgtatcacgaaaaatacccgaccatctatcacctgcgtaagaaactggtggacagcaccgataaagcggacctgcgtctgatctatctggcgctggcgcacatgattaagttccgtggtcactttctgatcgaaggcgatctgaacccggacaacagcgatgtggacaaactgttcatccagctggttcaaacctacaaccagctgtttgaggaaaacccgattaacgcgagcggtgttgacgcgaaagcgatcctgagcgcgcgtctgagcaagagccgtcgtctggagaacctgatcgcgcaactgccgggtgaaaagaaaaacggtctgtttggcaacctgattgcgctgagcctgggcctgaccccgaacttcaagagcaactttgatctggcggaggacgcgaaactgcagctgagcaaggacacctatgacgatgacctggataacctgctggcgcaaatcggcgatcagtacgcggacctgttcctggcggcgaaaaacctgagcgacgcgatcctgctgagcgatattctgcgtgtgaacaccgagattaccaaagcgccgctgagcgcgagcatgatcaagcgttatgacgaacaccaccaagatctgaccctgctgaaggcgctggttcgtcagcaactgccggagaagtacaaggaaatcttctttgatcaaagcaagaacggttacgcgggctatattgacggtggcgcgagccaggaagagttctacaagtttatcaaaccgattctggagaagatggacggtaccgaggaactgctggtgaaactgaaccgtgaagacctgctgcgtaagcaacgtacctttgataacggtagcatcccgcaccagattcatctgggtgaactgcatgcgatcctgcgtcgtcaggaagacttctacccgtttctgaaagataaccgtgagaagatcgaaaaaattctgaccttccgtattccgtactatgttggtccgctggcgcgtggcaacagccgttttgcgtggatgacccgtaaaagcgaggaaaccatcaccccgtggaacttcgaggaagtggttgataagggtgcgagcgcgcagagcttcattgagcgtatgaccaactttgacaaaaacctgccgaacgaaaaagtgctgccgaagcacagcctgctgtacgagtatttcaccgtttataacgaactgaccaaggtgaaatacgttaccgagggtatgcgtaagccggcgttcctgagcggcgaacaaaagaaagcgatcgtggacctgctgtttaaaaccaaccgtaaggtgaccgttaagcagctgaaagaggactacttcaagaaaattgaatgcttcgatagcgtggagatcagcggtgttgaagaccgttttaacgcgagcctgggcacctaccacgatctgctgaagatcattaaggataaagacttcctggacaacgaggaaaacgaggatatcctggaagacattgtgctgaccctgaccctgtttgaggatcgtgaaatgatcgaggaacgtctgaaaacctatgcgcacctgttcgatgacaaggttatgaaacagctgaagcgtcgtcgttacaccggttggggccgtctgagccgtaagcttatcaacggtattcgtgacaaacaaagcggcaagaccatcctggactttctgaaaagcgatggtttcgcgaaccgtaactttatgcagctgattcacgatgacagcctgaccttcaaagaggatatccagaaggcgcaagttagcggtcaaggcgacagcctgcacgaacatattgcgaacctggcgggtagcccggcgatcaagaaaggcattctgcagaccgtgaaagtggttgacgagctggtgaaagttatgggtcgtcacaagccggaaaacatcgttattgagatggcgcgtgaaaaccagaccacccaaaaaggccagaagaacagccgtgagcgtatgaaacgtatcgaggaaggtattaaggaactgggcagccagatcctgaaagagcacccggtggaaaacacccagctgcaaaacgagaagctgtatctgtactatctgcaaaacggtcgtgatatgtacgttgaccaggaactggatattaaccgtctgagcgattacgacgtggatcacatcgttccgcagagcttcctgaaagatgacagcattgacaacaaggtgctgacccgtagcgacaaaaaccgtggcaagagcgataacgttccgagcgaggaagtggttaagaaaatgaagaactactggcgtcaactgctgaacgcgaaactgatcacccagcgtaagtttgataacctgaccaaagcggagcgtggtggcctgagcgaactggacaaagcgggtttcattaagcgtcaactggtggagacccgtcagatcaccaaacacgttgcgcagattctggatagccgtatgaacaccaagtacgatgagaacgacaaactgatccgtgaagtgaaggttattaccctgaagagcaaactggttagcgacttccgtaaggatttccaattctacaaggttcgtgaaatcaacaactatcaccacgcgcacgacgcgtacctgaacgcggtggttggtaccgcgctgattaagaaatacccgaaactggagagcgaattcgtttacggcgactataaggtgtacgatgttcgtaaaatgatcgcgaagagcgagcaggaaattggtaaagcgaccgcgaagtatttcttttacagcaacatcatgaacttctttaagaccgagatcaccctggcgaacggtgaaatccgtaagcgtccgctgattgagaccaacggcgagaccggcgaaatcgtgtgggacaaaggccgtgattttgcgaccgtgcgtaaggttctgagcatgccgcaagtgaacattgttaagaaaaccgaggttcagaccggtggcttcagcaaggaaagcattctgccgaaacgtaacagcgataagctgatcgcgcgtaagaaagactgggacccgaagaagtatggtggcttcgacagcccgaccgtggcgtacagcgttctggtggttgcgaaggtggagaagggtaaaagcaagaaactgaaaagcgttaaggaactgctgggcatcaccattatggagcgtagcagcttcgagaagaacccgatcgattttctggaggcgaaaggttataaggaagtgaagaaagacctgatcattaaactgccgaagtacagcctgtttgagctggaaaacggccgtaaacgtatgctggcgagcgcgggcgagctgcagaaaggcaacgaactggcgctgccgagcaagtacgtgaacttcctgtatctggcgagccactacgagaagctgaaaggtagcccggaggataacgaacagaaacaactgtttgttgagcaacacaagcactatctggacgagatcattgaacagattagcgaattcagcaaacgtgtgatcctggcggacgcgaacctggataaggttctgagcgcgtacaacaaacaccgtgataagccgatccgtgagcaggcggaaaacatcattcacctgttcaccctgaccaacctgggtgcgccggcggcgttcaagtattttgacaccaccatcgatcgtaaacgttacaccagcaccaaagaggtgctggacgcgaccctgattcaccaaagcattaccggcctgtatgaaacccgtattgacctgagccaactgggcggcgatggatccatggcagaacaaagcgacaaggatgtgaagtactacactctggaggagattcagaagcacaaagacagcaagagcacctgggtgatcctacatcataaggtgtacgatctgaccaagtttctcgaagagcatcctggtggggaagaagtcctgggcgagcaagctgggggtgatgctactgagaactttgaggacgtcgggcactctacggatgcacgagaactgtccaaaacatacatcatcggggagctccatccagatgacagatcaaagatagccaagccttcggaaaccctt

SEQ ID NO: 1232 - protein, 1408 aa, Artificial Sequence
  Amino acid Sequence of of HNM563C9
MGSSHHHHHHSSGLVPRGSHMPKKKRKVALAVIVVPALAPMDKKYSIGLDIGTNSVGWAVITDEYKVPSKKFKVLGNTDRHSIKKNLIGALLFDSGETAEATRLKRTARRRYTRRKNRICYLQEIFSNEMAKVDDSFFHRLEESFLVEEDKKHERHPIFGNIVDEVAYHEKYPTIYHLRKKLVDSTDKADLRLIYLALAHMIKFRGHFLIEGDLNPDNSDVDKLFIQLVQTYNQLFEENPINASGVDAKAILSARLSKSRRLENLIAQLPGEKKNGLFGNLIALSLGLTPNFKSNFDLAEDAKLQLSKDTYDDDLDNLLAQIGDQYADLFLAAKNLSDAILLSDILRVNTEITKAPLSASMIKRYDEHHQDLTLLKALVRQQLPEKYKEIFFDQSKNGYAGYIDGGASQEEFYKFIKPILEKMDGTEELLVKLNREDLLRKQRTFDNGSIPHQIHLGELHAILRRQEDFYPFLKDNREKIEKILTFRIPYYVGPLARGNSRFAWMTRKSEETITPWNFEEVVDKGASAQSFIERMTNFDKNLPNEKVLPKHSLLYEYFTVYNELTKVKYVTEGMRKPAFLSGEQKKAIVDLLFKTNRKVTVKQLKEDYFKKIECFDSVEISGVEDRFNASLGTYHDLLKIIKDKDFLDNEENEDILEDIVLTLTLFEDREMIEERLKTYAHLFDDKVMKQLKRRRYTGWGRLSRKLINGIRDKQSGKTILDFLKSDGFANRNFMQLIHDDSLTFKEDIQKAQVSGQGDSLHEHIANLAGSPAIKKGILQTVKVVDELVKVMGRHKPENIVIEMARENQTTQKGQKNSRERMKRIEEGIKELGSQILKEHPVENTQLQNEKLYLYYLQNGRDMYVDQELDINRLSDYDVDHIVPQSFLKDDSIDNKVLTRSDKNRGKSDNVPSEEVVKKMKNYWRQLLNAKLITQRKFDNLTKAERGGLSELDKAGFIKRQLVETRQITKHVAQILDSRMNTKYDENDKLIREVKVITLKSKLVSDFRKDFQFYKVREINNYHHAHDAYLNAVVGTALIKKYPKLESEFVYGDYKVYDVRKMIAKSEQEIGKATAKYFFYSNIMNFFKTEITLANGEIRKRPLIETNGETGEIVWDKGRDFATVRKVLSMPQVNIVKKTEVQTGGFSKESILPKRNSDKLIARKKDWDPKKYGGFDSPTVAYSVLVVAKVEKGKSKKLKSVKELLGITIMERSSFEKNPIDFLEAKGYKEVKKDLIIKLPKYSLFELENGRKRMLASAGELQKGNELALPSKYVNFLYLASHYEKLKGSPEDNEQKQLFVEQHKHYLDEIIEQISEFSKRVILADANLDKVLSAYNKHRDKPIREQAENIIHLFTLTNLGAPAAFKYFDTTIDRKRYTSTKEVLDATLIHQSITGLYETRIDLSQLGGD

SEQ ID NO: 1233 - DNA, 4224 bp, Artificial Sequence
  Polynucleotide Sequence of HNM563C9
atgggcagcagccatcatcatcatcatcacagcagcggcctggtgccgcgcggcagccatatgcccaagaagaagaggaaggtggcgctggcggtgattgtggtgccggcgctggcgccgatggacaaaaagtatagcattggcctggacattggcaccaacagcgtgggctgggcggttatcaccgatgagtacaaggttccgagcaagaaatttaaggtgctgggtaacaccgatcgtcacagcatcaagaaaaacctgattggtgcgctgctgtttgacagcggtgaaaccgcggaagcgacccgtctgaaacgtaccgcgcgtcgtcgttacacccgtcgtaagaaccgtatctgctacctgcaggagattttcagcaacgaaatggcgaaggtggacgatagcttctttcaccgtctggaggagagcttcctggttgaggaagataagaaacacgagcgtcacccgatctttggcaacattgtggacgaggttgcgtatcacgaaaaatacccgaccatctatcacctgcgtaagaaactggtggacagcaccgataaagcggacctgcgtctgatctatctggcgctggcgcacatgattaagttccgtggtcactttctgatcgaaggcgatctgaacccggacaacagcgatgtggacaaactgttcatccagctggttcaaacctacaaccagctgtttgaggaaaacccgattaacgcgagcggtgttgacgcgaaagcgatcctgagcgcgcgtctgagcaagagccgtcgtctggagaacctgatcgcgcaactgccgggtgaaaagaaaaacggtctgtttggcaacctgattgcgctgagcctgggcctgaccccgaacttcaagagcaactttgatctggcggaggacgcgaaactgcagctgagcaaggacacctatgacgatgacctggataacctgctggcgcaaatcggcgatcagtacgcggacctgttcctggcggcgaaaaacctgagcgacgcgatcctgctgagcgatattctgcgtgtgaacaccgagattaccaaagcgccgctgagcgcgagcatgatcaagcgttatgacgaacaccaccaagatctgaccctgctgaaggcgctggttcgtcagcaactgccggagaagtacaaggaaatcttctttgatcaaagcaagaacggttacgcgggctatattgacggtggcgcgagccaggaagagttctacaagtttatcaaaccgattctggagaagatggacggtaccgaggaactgctggtgaaactgaaccgtgaagacctgctgcgtaagcaacgtacctttgataacggtagcatcccgcaccagattcatctgggtgaactgcatgcgatcctgcgtcgtcaggaagacttctacccgtttctgaaagataaccgtgagaagatcgaaaaaattctgaccttccgtattccgtactatgttggtccgctggcgcgtggcaacagccgttttgcgtggatgacccgtaaaagcgaggaaaccatcaccccgtggaacttcgaggaagtggttgataagggtgcgagcgcgcagagcttcattgagcgtatgaccaactttgacaaaaacctgccgaacgaaaaagtgctgccgaagcacagcctgctgtacgagtatttcaccgtttataacgaactgaccaaggtgaaatacgttaccgagggtatgcgtaagccggcgttcctgagcggcgaacaaaagaaagcgatcgtggacctgctgtttaaaaccaaccgtaaggtgaccgttaagcagctgaaagaggactacttcaagaaaattgaatgcttcgatagcgtggagatcagcggtgttgaagaccgttttaacgcgagcctgggcacctaccacgatctgctgaagatcattaaggataaagacttcctggacaacgaggaaaacgaggatatcctggaagacattgtgctgaccctgaccctgtttgaggatcgtgaaatgatcgaggaacgtctgaaaacctatgcgcacctgttcgatgacaaggttatgaaacagctgaagcgtcgtcgttacaccggttggggccgtctgagccgtaagcttatcaacggtattcgtgacaaacaaagcggcaagaccatcctggactttctgaaaagcgatggtttcgcgaaccgtaactttatgcagctgattcacgatgacagcctgaccttcaaagaggatatccagaaggcgcaagttagcggtcaaggcgacagcctgcacgaacatattgcgaacctggcgggtagcccggcgatcaagaaaggcattctgcagaccgtgaaagtggttgacgagctggtgaaagttatgggtcgtcacaagccggaaaacatcgttattgagatggcgcgtgaaaaccagaccacccaaaaaggccagaagaacagccgtgagcgtatgaaacgtatcgaggaaggtattaaggaactgggcagccagatcctgaaagagcacccggtggaaaacacccagctgcaaaacgagaagctgtatctgtactatctgcaaaacggtcgtgatatgtacgttgaccaggaactggatattaaccgtctgagcgattacgacgtggatcacatcgttccgcagagcttcctgaaagatgacagcattgacaacaaggtgctgacccgtagcgacaaaaaccgtggcaagagcgataacgttccgagcgaggaagtggttaagaaaatgaagaactactggcgtcaactgctgaacgcgaaactgatcacccagcgtaagtttgataacctgaccaaagcggagcgtggtggcctgagcgaactggacaaagcgggtttcattaagcgtcaactggtggagacccgtcagatcaccaaacacgttgcgcagattctggatagccgtatgaacaccaagtacgatgagaacgacaaactgatccgtgaagtgaaggttattaccctgaagagcaaactggttagcgacttccgtaaggatttccaattctacaaggttcgtgaaatcaacaactatcaccacgcgcacgacgcgtacctgaacgcggtggttggtaccgcgctgattaagaaatacccgaaactggagagcgaattcgtttacggcgactataaggtgtacgatgttcgtaaaatgatcgcgaagagcgagcaggaaattggtaaagcgaccgcgaagtatttcttttacagcaacatcatgaacttctttaagaccgagatcaccctggcgaacggtgaaatccgtaagcgtccgctgattgagaccaacggcgagaccggcgaaatcgtgtgggacaaaggccgtgattttgcgaccgtgcgtaaggttctgagcatgccgcaagtgaacattgttaagaaaaccgaggttcagaccggtggcttcagcaaggaaagcattctgccgaaacgtaacagcgataagctgatcgcgcgtaagaaagactgggacccgaagaagtatggtggcttcgacagcccgaccgtggcgtacagcgttctggtggttgcgaaggtggagaagggtaaaagcaagaaactgaaaagcgttaaggaactgctgggcatcaccattatggagcgtagcagcttcgagaagaacccgatcgattttctggaggcgaaaggttataaggaagtgaagaaagacctgatcattaaactgccgaagtacagcctgtttgagctggaaaacggccgtaaacgtatgctggcgagcgcgggcgagctgcagaaaggcaacgaactggcgctgccgagcaagtacgtgaacttcctgtatctggcgagccactacgagaagctgaaaggtagcccggaggataacgaacagaaacaactgtttgttgagcaacacaagcactatctggacgagatcattgaacagattagcgaattcagcaaacgtgtgatcctggcggacgcgaacctggataaggttctgagcgcgtacaacaaacaccgtgataagccgatccgtgagcaggcggaaaacatcattcacctgttcaccctgaccaacctgggtgcgccggcggcgttcaagtattttgacaccaccatcgatcgtaaacgttacaccagcaccaaagaggtgctggacgcgaccctgattcaccaaagcattaccggcctgtatgaaacccgtattgacctgagccaactgggcggcgat

SEQ ID NO: 1234 - DNA, 97 bp, Artificial Sequence
  Polynucleotide Sequence of HNM161C9SB 5'-primer
ggaattccatatgcccaagaagaagaggaaggtggcgctggcggtgattgtggtgccggcgctggcgccgatggacaaaaagtatagcattggcctg

SEQ ID NO: 1235 - DNA, 97 bp, Artificial Sequence
  Polynucleotide Sequence of HNM165C9SB 5'-primer
ggaattccatatgcccaagaagaagaggaaggtggcgctggcggtgccggtggcgctggcgattgtgccgatggacaaaaagtatagcattggcctg

SEQ ID NO: 1236 - DNA, 97 bp, Artificial Sequence
  Polynucleotide Sequence of HNM264C9SB 5'-primer
ggaattccatatgcccaagaagaagaggaaggtgctggcggcggcgccggtggtgattgtgattgcgccgatggacaaaaagtatagcattggcctg

SEQ ID NO: 1237 - DNA, 97 bp, Artificial Sequence
  Polynucleotide Sequence of HNM442C9SB 5'-primer
ggaattccatatgcccaagaagaagaggaaggtggcgctggcggcgctggttccggcggttctggttccgatggacaaaaagtatagcattggcctg

SEQ ID NO: 1238 - DNA, 97 bp, Artificial Sequence
  Polynucleotide Sequence of HNM552C9SB 5'-primer
ggaattccatatgcccaagaagaagaggaaggtggcgctgctggtgattgcggttccggcggtggcgccgatggacaaaaagtatagcattggcctg

SEQ ID NO: 1239 - DNA, 97 bp, Artificial Sequence; identical to SEQ ID NO: 1234
  Polynucleotide Sequence of HNM563C9SB 5'-primer

SEQ ID NO: 1240 - DNA, 97 bp, Artificial Sequence
  Polynucleotide Sequence of HNM661C9SB 5'-primer
ggaattccatatgcccaagaagaagaggaaggtggcggcgattctggcgccgattgtggcggcgctgccgatggacaaaaagtatagcattggcctg

SEQ ID NO: 1241 - DNA, 97 bp, Artificial Sequence
  Polynucleotide Sequence of HNM889C9SB 5'-primer
ggaattccatatgcccaagaagaagaggaaggtgattctggtggcggcggcgccgattgcggcgctgccgatggacaaaaagtatagcattggcctg

SEQ ID NO: 1242 - DNA, 97 bp, Artificial Sequence
  Polynucleotide Sequence of HNM899C9SB 5'-primer
ggaattccatatgcccaagaagaagaggaaggtggcggtggtgattgcgctgccggcggtggtggcgccgatggacaaaaagtatagcattggcctg

SEQ ID NO: 1243 - DNA, 39 bp, Artificial Sequence; identical to SEQ ID NO: 1228
  Polynucleotide Sequence of Cas9 3'-primer